European Patent Application EP 4 722 352 A1, published April 8, 2026. Title: African Swine Fever Virus ASFV-KOR.INJE.MEC-01.2022 attenuated by cell adaptation and uses thereof. Applicant: National Institute of Wildlife Disease Control and Prevention(NIWDC). Application KR. The sequence listing filed with the application follows.

SEQUENCE LISTING (3 sequences)

SEQ ID NO: 1 - DNA, 25 bp, synthetic construct
  source 1..25: mol_type = other DNA
ctgctcatggtatcaatcttatcga

SEQ ID NO: 2 - DNA, 19 bp, synthetic construct
  source 1..19: mol_type = other DNA
gataccacaagawsgccgt

SEQ ID NO: 3 - DNA, 177622 bp, African swine fever virus
  source 1..177622: mol_type = genomic DNA
actgctgtaggcgtcaaagattaaaattattactactgctgtaggcgttaaacattaaaattattactactgctgtaggcgttaaagattaaaaatattagtactgctgcaggcgttaaagattaaaaatattagtactgctgcaggcgttaaacattaaaattattgtactgctgtaggcgttaaacattaaaattattactactgctgtaggcgtcaaagattaaaattattactactgctgtaggcgttaaacattaaaattattactactgctgtaggcgttaaagattaaaaatattagtactgctgcaggcgttaaagattaaaattattactactgctgtaggcgtaaaagattaaaattattactgtaggcgttcatttcacaagatgcggaattatttcgcaaagattattttttgaaacgccgcggccggaaatatttttttttgcggttgtaattgatttttttttgcggctgggcggcgggccagacaaaattgaccataactggtgttacgccgccggtaataaaccctaccgtaaatacttttttttggggcggccagagagacattatcgccgtaggtatcaattactgctgtaggtatcaattattatactacaggcgttaaacattattagtacacaggcgtcaaagaagctaaaacttaatgttttttcgtcaaaaatcgccatgaatatctatcttgtgtggtttctctacatactattggggaacctgatattagcagtaatatattgcgtcatagatgaggtggtgtgtgacaatatccatataaaaaaaaatgttgccgcccctgagatgccgcggcggttctaaattttaatgtttttttcggcgaacatttttcacatatgcgatattggcgctaaagcgagcgtattaccgcttgtaacaacattttttttcgatcggcaatagataagtagaatataccatattattgctattgccatcaatgagaatgccacgtaggcataggtcatcctatggccggaccaatccatggctgcacttaaaaatatcaaaaaaagtttaagttttgggccggcgttaaaatttaaaccttttctggttgatctttagccatgtatagctgcgatgtttggtgccttatctacatgctattggcattcctgatattcgcactaaagtgctatgttacaaccgtcttatgcgtgatttttatccaccttattggccgaagggccgccttgtatttcctgttaggtggtttggccgtattctactggtggcaagcagctatcaataaaatttaatggctctcacttaagatccttgctgtaagcgggcgtttacatactttgatcaagaaaaaaaattatttttggacccccccccatgttttatacaaaaatcatataataaagtggcgacaatcaacatattaatcaaccacagcattttatgatgtgttaatcaacatataccatattaatcaaccacagcattttatgatgcgtcaatcaacatattattacggagagcgtcaatcaatataatattgagaacagcgacttgataccgtgtatggtggtggcggcggcatgttgtttgtaacagcatttttcatcattcgaagcttacaaaagatatgtataagatagcatattaatgttattaacagtaatatcaataaggcgtagctatagatcttcactttggtagaccaataatccatggttgcgcttaaaaataccaaaaaaaacattaagttttggagggtaagattggtttttcaccattggtaaagattattattctaaatgtttaccccatagatgtgaaacaatgattcttcatatattaacatattttttgacttatacttttcttcatctagtaaggcgttaattttttccggatctgtcgtttttattgataaaagagaagagtctggactgtaatttttaaataataagatatttattaatatccaattattcgtttggctcgctatttccatgctctcttcgaaagcatcagctcctaaatctatacaaaggaataagttaccttcacaaaaattcattaccgaggtaatcattgcccgattaatgtcagcccccaacataaaacaataatatatagttgtataattacaatcatacatacaggccaactgcatcatttcatcaatgtctatatttgtcttctctttgttataaatttcatgaaggtcaaagacgttgttataagcaaccccacatattaaccgccaatctttaaaatgactatatcgttgataaaaatattggatggcttcagtaagcttatatggtatcgccatactataccaatacctagttagcatttcgttgaatgaaatattatccaatgtaaagttaattgataatgtatctagttcaccaaaaattcttaatttcagttgagcattatttaggaaaaggggattatcagataataattcatggcatagaataatattactgctagttttaacatactgtacattataaaatatttctaaaattttattttcactcaaagctttcctcgcacctaacttttggcataggtcctggtgcactccatattgacagtaaccaacccaaagctgatgtctgcaccccattcggtaaacagctctattaaaccatgattgttttcctgtacagccttcattaatgcaacatttaatgttaaaccatgtttaaaacttgctgtttttattaatatttgttcatctatacaagtatgataaatcgtaattggggcttcatgccaccacaaaccacaacgctctaaaatacaataatcatcttttaacacaggctgtgtagctagtacttttttagtaagtgcttgtaaagtagatggcatcttctatctgcaaaataattatttccgaaaaaaaaatcaaattaaaatactaaattctatttttttttttaataaagcctgtaaattatataataaatctcgcccaccgtattatttccggacacaactttttatacctcattatatttttagatctatagttttttaacaaggcattaattttttctggatctgtcgtttttaaagataaaagagagacgtttgaactataataatctttaaatgataatatttctactaatatatcatgattcttttgttttgctaattctaagctctcttcgaaagcattagctcctaaatctatacaaaagaacaagttattcatataaaagttttttaccgaggtaaccattgcccgattgatgtcagcccccaatacaaaacaatagtaaatggttaaaaaattgctatctctcatacaggccagatatatcatttcatcaatattcatatcaaccttttttatatgatacatttcatgaagatcagacacgttattaaaagaaagcccacatattagccgccaatctttaaaatgactatatcgttgataaaaatattggatggcttcagtaagcttacatagtatcgctatactataccaatatctagttagcatttcgttgaatgttatttcattcaatataaagttgatcgatatcttctctagaaaacaacaaattattacttttaattcctctatattctggaaaaggggattattagataacaatttatggcataaaataatattactactagttttaatacgatgtattttataaaatatttgtacaatatccatttcattcaaaatttttgcgcctaactcccggcagaaattccaagtatgctccgtattgacagtgactaagctagagttgatgtctgcaccccattcagtaaacaactctattagatcatagttgttttcctgcacagttttcattaatgcgagatttaactctaaaccatctttaaaaattgctgattttatcatcaattgattatcctcattagtagaaagcataattggagctccatgccaccacaaaccacaatatttcaaaataaagtagtgttctttagatatgtgctgtgtggccagtatttttttagcaagagcctgcagagaaattggagtagacatatttttttttgcaaaatggtttaagtttttcaagaatacagattggataaattaggttgttgacttagttacaggaggtattaaatattatgtagacataaaaatgagatcctccaaaaaaataaacaacaaaaaaaaatatgtttaatattaaaatgacaatttctacattgcttattgctcttattatactacttattattattttagtagtgtttttatactataagaaacaacaaccaccgaaaaaggtctgtaaagtagataaagattgtggtagtggagagcattgtgttcgtggatcatgtagctcattgagctgcttagatgccgtaaaaatggacaaacgaaatattaagatagattctaagatttcctcatgcgaattcactcccaatttttaccgttttacggatactgctgctgatgagcagcaagaatttggaaaaacacggcatcctataaaaataactccatctccaagtgaatcccatagcccccaagaggtgtgtgaaaaatattgttcatggggaaccgatgactgtacaggttgggaatatgttggtgatgaaaaggagggaacatgttatgtatataataatccacatcacccggttcttaaatatggtaaggatcacatcatagccttacctagaaatcataaacatgcataaataaatacattaggctcatcgtatctttttaaaatccataaatattcgtttgatatatgctgaaatttttataaaaaaaaataactatttcctataaatcatctagaaatagtcctcgttttgatcggtttatatcttataatattgtgcatcgatgcacaactgctttttttggtccttctggaacatcattatattttctttcattaatataccattcagatgtaaacgttgaataatttttatggcaacaatctaccattgaattatatttagtaacatctaatacatcgtttgttttatcaggctcagctctataatcttgataatttttgttatcagcttctaaagctccatcattatttttcaaagaagtatccataattatgtttggtaaaaatactttaagttttaatgtgatatttaaaatggttgttatataaatttaccgcttacaggtaatctttattcagtgtcataaactatacttttgatgattcagtattttgtgaatcagtacatttattatcattaatatttttaggctgtttttccaatgttttattgttgcaatgagcctgctcctcctttgacgaggaagtgtctgttggagtcatctgtttaggaagagtatcatccatatctattatgaagaaaatatataaatattgatatacaatcaaaaatatttttgatcacgtctttgttatctatcgatattgttgataacgtcttgaataacctacatcatttttttacataaaaaaatagatataatttttattatatctcaattattttaaagataattatcaatacagcaaatatcataagctaacatatttttcgaataatagttttttagtaaagtattaatcttttcaggattggtttcttttgataataagataggattcgctttataaatttttaaagataatatattcacaatgatagaataaccgtatatatctgctaatgtcttactgtgttcaataacattagcccctaaatccatacaaaagaacatattttcaatacaaaagttttttaccgagattaacattgctcgattagcgttggctcccaatgcaaaacagtagtaaatggtcaaaaaattattatcgcgcatacaggccagctccatcattttattaatactcatatgaattttcgttgtgttacatatttcatgaaggtcaaacacattgttgaaagaaagtgcacaaattaatcgccattcatcaaaatgcctgtattcttgacaaaaatattgaatagcttctttaagattatattttaccgctatgccataccaatatttggttagcatctcactaaatgagatctcatttaacatagaatttgttgttaaatccttcaactcccaataaatgatcatccttaaatccaccatgtttacattttgtaaaaaagggttattagaaaataattcatgacacaaaatgacattactacttgttattttacactttgtttcaaagaaaaatcgtaaaatttcacttgtctcaagctcttctttagctcccaattttcggcataggtttcgagtatgctcgttattaataaaaagtaacccataattaatatttgcaccccattcagtaaacaacatgattagatcatcattgttttccttaactgccaataccaatgcagtattaagccttataccctctttaaagcataatgtccttatcattatttgattatcatcatctatatacattgagataggagcttcatgccaccataaaccataacgctctaaaatataataatcatctttagatacgtgttgcgtggccaatgcccttttagcaagtgcttgtaaagtcgatggctgcatgtttattctgttaaaaaaaaatcaaattatcgggtaaacataaggatcaacccgtagttaatatttgcagtagtattttttaacaatgaattataataaaaaaataattcattactatctattataaaacccatctttaactttaaagaagaactagatcatctttttttttgttgtgtcagaacttcttcaatttattacccacattttatctaaaaaaaataaaaactacatcatatcttgtttcttcatcaaattatcataccatttatagggtgtaggttgggaacattccatcatgtggtaatcagggtatttatatattttttgatagtaacatctatttggcagatgtattgtccaacaatcatgtctaataaaatcattttcacctatgggggaatcatcttaaaaaccttattcctacagattccattttgacagtcctagcaaaagtcacaatattttccatgagtacaccaatgttcaagctctctttcgggaggaatgctgccaattttatgttttttagcttctaactctctgtacaacatcagttgggaaagcagaaagaagattaccaggagaaccattaaatatataatagtctgcaaactacgtttgcgaatgtaatttgcaactaaaacacaacccacaaggtaaaatccataagttaataacttttgccattttcgtatgacagcctcgtgccattcatggttgtgttgtgggcattctgttcggtaaacttcatgaggctttatagaagttacatagtaggtacagaattcattgtgacgaaaaacactgcagttagctatgtagtcattttcaagaatgggagaatggttttcaaagaccttattcttacagatgccatcttgacagtcccaacagaacctacaatgatttgcataggtgcaccagtattcaagctccttttcaggaggggttcttgttagatccaggagctctagctcatatgtataaagaagagttggaatggatagtaaagtaaatatttgcagaccaagcatggctacttgtgaacaagtggctgctcgtcaacaaatagctgtttatcagcaaatagctgtttatcagcaacaactaattatcagcaaatgctgcttgtgggtaagccaataaataggccatacccttgaaaggagaattcagtttgataaaaaaaataacgagttttctaataacccggtcaagcatttaataaatgaatagcatcacacgtctgcatcgtgcattctgcctggaaaatgggcccatctctaatatatttacactgacggtgaatcatacagtgttccatgggatagctatgctcctgtacaggaggcatatcttttagaactttattcttacaaagaccatcttgacaagcccagcaaaaccgacaatttttcacatattgacaccagtatctaagctcctcttccaggggattgtcggtcgaaaacccctgtagactagctaggccagctagcagcaagccgaggtaactaaagaacctcattgtagtgttatattacgaaaaaacatgttaaaatttggaaaaaaaagccctttttatagatctggaaaaaaattttcacaaatctaattaaaagccttacagatcatccttttcataaattttcattaacaattggtgggggcggttgtgaggtactggatcagaacaatccataacatggtaatgtccatttccttcaccatatgtacactggttataccagcgagaaacctcacaagatgtcaaataactgttctcaacaatcaatggcatgctcttattcaccttgttcttgcaaattccatgtgcacattcccagcaaaacttgcagttttccatgtaagtacaccagtatccaagttcttcttgtggaggattatccgttgaacgaagatgccctcctgcctgagtaggtagtcctaagacctgattggccagcaggccaagaatttccaagaagatcaccaacattgctacggctggctgaacagctggcagatagctagctaattagcaaaccaagtgactcgccctctctactcttaatatgagaatttaagattcggtccggcttttttcccatgttttacagggaaaaggtatttttagcctatgaatgtacatggttccgcacattaaaaaaaaataaaagaaattatttaatattggctgttattttctttcaactagcaacaagccaggtaactaaagaacttcattgtagttttatattacggaaaaggttaaattttggacaaaaaaaatcatatctaattaaaaatcctcacagatctttcttttcataaattttcattaacaattggtaggggcggttgtgaggtactggatcagaacaatccataacatggtaatgcccatttccttcaccatatgtacactggttataccagcgagaaacctcacatgttgtcaagtagctgttttcaataatcaatggcatgctattattcaccttgttcttgcaaattccatgtgcacattcccagcaaaacttgcacctttccatgtaagtgcaccagtatccaagttcttcttgtggaggattatccgttgaacgaagatgccctcctgcctgagtaggtagtcctacgacctgattggccagcaggccaagaattcccaagaagactaccaacattgctacggctggctgaacagctggcagatagctagctaattagcaaaccaagtgactcaccctctctactcttaatatgagaatttaagatccggtccgacatttttccgatattttacaagaaaaagatatttttagctacaaatacacttcatatatccctaaaaaaaacaaaaatttatttaattttaactattattttctttccactctctctttaagattttgtaaggattccagggctttggttcagaacaggccattacatggtgaatcccctgtcctagatcatacatacatttatttagccagcgggaaactatacatgattgcacatactcattttcaagaattgttgtattctccaatttgccctcacaaaggccattttgacaattccagcaaaacttgcagttttctgtataagtgcaccagtattcaagttcttcttgtggaggattatccgttggatgaagttgtccagctggttgattaggtagccctaagacctggttgcaattcatggtatggtagatacccttatctaaatcatacatacatttatccagccaacgggaaaccagacatgatttcacatactcattcttgtaaattactgacccatctattttgtttatacaagtgccgtcttggcagtcccagcaaaattggcaactttccatgtaggcacaccagtattcgagttcttcctctggaggctcctctgttggacgaagttgtccaacgagctgacttgaaacctggctggccagaaggccaagaattcccaagaagatcaccaacattgctacggctggctgaacagctgactgaatagctagccaattagcaatccactgtacttttcataagatcatttaagattcggtcggcattttttcaatagtttgctaggaaaaaatttttaattttatagattcacactacttcattctcatgcttaggaaaaaaacaaactaaatcttacaatgtatctggatctaatgagaagctagaattcatcttttttcaaatcctttctgggatgttcattctttttccactccttccttgcaattttataaggattccagggctttgggtcagaacagttcatgctatggtaaatgtgctcctccacatcatatctacataggtcaccccagcgggaaacctcacaatattttacatagtcattctcaataatacttgtggagttgtttccccaaaccctgctggtacaaatcccatcttcacaatcccagcagaaccgacagctttccacataagtgcaccagtatccaagttcattctctgggggttcaaatgttagaggaagatgtccacctacccgagtagaagtggaggatgaaaccaggttgctactggccagcaggccaataattcccaggataatcaccagcattgtgctcaaccagcaacggctagcaacgactagcaactgactagcaatagctagaaatggctagcaatcagtagtagctaacgctctactctttataagaaaatttaaaattcgatcagatttttttagaattgagaatgagtaaaacgcttatattctttttctagctagaaaaaataagctagtttaagataggatttcccttactaacggtttaatttttagcaaaggtataggtaaaatacacttgtacttagctgcaaaaaaataagcttatggcgtataagccgccataagtttatttaattaaaatgttaaactctgtgataagactggaatcttaggcaggtttgatgtggagaacagcatgaaatacaagagtgcctgttacacgaataagttctctcaaaccggggatggtcatactcacatctatgaaatcctggtctaggagattcatttgatgcatgatggccgcacccacacttatgagacactgaagaactaaagggtttaattttgatctgaatggtactatataggatgatggcaatccatatcaagattagagcaatcaaaatcacctcctcaagaagcatgatgtagccttaaatcttagactgctttaaaccttaggccctcactatctttaatgaaggagtttaaattttgatccctttttcaagacccatttagaagaaaaaaataaagtttatatcaatctaattcataagtcatctctttcataaatcttcatgtattctctatgtggataagtatgggatgttggatttgcgcaatcaaaaactttaactctcgatgaatctcttcccccatttcctgtacatttagagcttccaacataggatttttatcaaatatttcatgacataaaataatgttattgctcgttttatgacgcattaaaccggtgaaaatttccttattatttaaactatctttagctcctaactttcgacacagctcctgagtttgttccgtcctagcacaggtcagcccataataaatgtttgctccccactcggtgaacagccttattacgtcatagttattttcttttatggccatgattaatgccacatcaagatgaagaagttcccccttaaagggggttgagcttaaaataacgtaattacagtagtgacataagctaatgggcttgttttgccaccataagccacaatattttaaaatataatgatactcctcaggcacgctctgtttggccacagcctttttggccagggtttgcaaggagagcatgataacttcttgaaaaaaaaactcaaattaagttcctacttttttaaaatattagtatggacagatctaccatcatatgaaggaattctttcatcgttaaacactgaagagataatactttcatcgtatagagaatatcatgtcaatccatatattgaatgttatatatcattaaacccatcattaatatagtgtttatgtgctatggacaggttttttgaatgataatcttttaacatacgttttataacttcgggatcagtttcttttaaagataaagaatcattcatgttataacaatttaatgataacatgctggcaatgaacgagttgtctttttgatgcgctagagtctttccctcctcaaaggcattggcgcctaagtctatacaaaagaatatgtttccgatattatagaactgaatagaatgaaacatggcctgattgatatcagcccctaagacgacgcaacagtaataaatcgttaaatagttatagttcttgcgacaggcccactttagcatttcattcatgtctatgcgaatcctctccttttcgtacacttcgtgaagttcaaacacattattgtaaaaaagggcgcacataagccgccaccgatgtagatgagcatatctctgataaaaatagcaaatcgcctccttaaggttacattctattgccatcgcgtaccaatatttagtaaacatctcgcttaatatatcggtttctaccattaatccctccagttgttcataaatcattccctttacttcaaaacgatttatggtatctaaaatgggattattagaaaatacctcatggcagaaaatgatgttactgctagttagatcacgtttcaatgtgtaaaaaaatcgtaaaatttcctggtcatttaactgttctttggcacctagctgcctgcacaggtctcgggtgtgctccgtgttgacagaaagcaaaccgtagttgatgtttgcaccccactcggtgaacaattctattagatcgtgattgttttcctccacagctttcaccaaggccgcgttaagatttgtgccgttcttaaaatacggcgtccatattttcttttgatgatacatgatagggccattatgccaccatagaccgcagcacttcaaaaaatgaggatggcatttggccggatactggctggccagcacctttttggtgagagtctgcagagagaggaccatatttcttttttttgaaaaaatcaaattaaaaaaatcatgcttgtttagcatacatgtaatattgttataattacgttataattacgttataattacgttataactatattataacaatggtataacaatggtataacaatgttataacaatgttataacgatgtatcattgatgtcatcattcaactaggccaacatactttttaatttatagttttttaatagatgatatattttgctaggatctgcttcttttaacgttaatagcgaggagtctgcactataaatgtctaatgataaatgatgagatatcaaatagtaattccgttgctctgctagggcctttgcctcttcaaaggcgtcggctcccagatctatacaaaagaacaagttatccatattataaaatcgtacgcaggcaagcatagctgaattaatattagctcctaagagaaaacaataatatatggttaaaaaattgttatcttttgtgcaggccatccgcatcatttcatccacgtccatgcggatcttttccttttcatacaaattatgtaggtcaaacagcttattaaaacaaagagcacagattaaccaccacgtatttagatacttaaaatgttggtaaacataagaaatggcctccctaagattatcctgcaatgccactataaaacagtatatcgttaacatatcaccatccgacatattacttaatatgtcggtgtcttctactaaccttttcaacttccaatatatggatgaccttatttcccttataatgacataggctggaaagggattatcattaaaaagtttaagacataagataatattactgctagtagtgccagggtgtattaatttaaagaacatgtgcataatcttctttttatccacgcggtacttggctcctaattcccagcaaaattctcgaacaggcggcgtattggcgcaaattaacccatagttgatgtctgcgccccattctgtaaacagttttattaactgatagttgctttcctttgtagccaacattagtgccgtattaaggtccaagccgtctgcaaagcttggcagctttatcagcatatgtttgcaatcaagggaaattggggccttataccaccatagtccgcagcgttctaagataacatggtactcaatagatacttgctgtctggctagtacctttttggcgaaggattgtaaggaaggaaacatcctgtttcttttttttttaaaaatcaattatctttgttcataatcaagaaaaatccccatatttattgagtgataattttttaacatgcaatttattttttcagggtccgtaacgatcgacaacagagaaataaccggattgtaatgctttaatgataaggcatgggctatcagataattttccttttgttctgccaaagctttgccctcctcaaaggcatcggcacccaggtctatacaaaagaacaggtttccaagattatagttttgtatggaaacaagcatggcttgattgatgttggctcccatgataaaacagtagtaaatggccgaatagctataatcttggatgcaggctatgtgcatcatttcatcaatatccatgcggaccctttctatttcgtacagctcgtgaaggtcgaacacgttgttgtaaaaaagggcgcacatgagccgccacctatgtagacgcgggtatttctggtaaaagtagcggatagcatctttgaggtcatagtccaccgctatcgcgtaccagtatttggttaaaacagtgctaaagctatcatcatggtccagcatgaaggttatctccatgagccctcttaactcccacatgatttcccccctcagatccagattatctataatccttaaattggggttattggaaaacacctcgtggcaaaagataatattgctactggttttatcgcgcgttgtatcaaagaaaatttttaaaatatactctctttctaaatattctttggctcccagctctttgcacagatcacgggtattttccgtgagagcacaaatcattccatagttaatatctgcaccccattcagtaaacagctttatcaagtcatgattattctccttcacggctttcatcagtcctatgtttaactcgataccttgactaaaacaggttgaccttataaataatttattgcgtcgaatatgaagcataatggggccattatgccaccacaggccacaacacttcaggacatgatattgatctaccggtatacactgcccggccagtactttcttcgtgagggattgcagggaaggcaacatgcctttccatcctttgacggaaatcaaattatctactaataactatcagtgtttatattaagtatttagatattatcccgggctggatacgtagtatcgctattcacatgtacttccaactctagccggagcctgcagggtcatttatttttaatattgattcttttttgtatttaatcatttagagaaggtcatcataggagccagatgttctctctccagaacttatgtcgaaaaacattacctaaccgtaaacttcctgaattttttgacgaatatatattacaactgctgggattatactgggaaaaccatggaactattcaacgagcaggaaacaactgtgtgcttatacagcaacataccctcattcccgtaaatgaagccctgagaacagcagcatctgaagaaaattatgagatcgtgagccttttattagcgtgggaggggaacctttactatgctattataggggctctagagggcaaccgccacgacttaattcgtaaatatgatgaccaaatcaaggaccatcatgaaattctgccattcattgacgatccagtcatatttcacaaatgccatatcatgcggcaatgcttttttgattgtattttatatcaagctgtaaaatatagtaagtttcgcgttcttctttactttaaacatagattagaggatgatttgcccttcactcatttacttattgaaaaggcatgtaaagatcataattatgaagttattaaatggatatatgaaaacctacatatctacaatatgatagatacctttgaatgtgctattgcccataaggatctacatctatattgtttggggtatagatttatatataacagaatcgtacccgataagtatcatcatttagatattcgcatgctttcaagcctacaactcctacataaggtggcagccaaaggatacttagattttatcctagaaaccttaaagtatgatcataataaagataatataaatattattctaacacaagctgcaacctataaccatagaaaaattttaatctatttcattcctcaatcaacccacgcacagatagaacaatgtttactagtggcgataaaagcaaaatcttccaggaaaaccttgaacttactactgtctcacctaaacctttccatcaacctcatcaaaaaaataagccattatgttgccacttacaattcaacaaatataataggcattctgagtatgcggcggaaaaagaagatatatttagatatcatattgacaaaatttgtaaaaaaagctatttttaataagtttgtcgttcgatgtatggatacattttctataaacccggaaagaatccttaaaatagccgcgcgaataaataggatgatgttagtgaaaaaaatatctgaacatgtttggaaaaatcatgcggttagacttaaataccttaaacatgcggtacacacgatgaagcataaagatgggaaaaatagactcatgaactttatctatgatcgctgttattaccatatgcaaggggaagaaatctttagcctcgcaagattttatgcaatccatcatgcaccaaagttgtttgacgttttttatgattgttgtatcctagatacgatacgattcaaaagccttcttttagattgttcacatatcataggtaaaaacgctcatgatgctaccaatatcaacatcgtgaacaagtatatcggcaacctgtttgttatgggagttcttagcaaaaaagaaatcttacaggactatccatccatttattctaaacaatacatgccttagtttattttttttgcggccgaaacattattcttaccctagaaaacgcttatagtcatcttaaatcataggtaaggaagatcatcatattttttgaaacgtaattttttaacgcatgatctatgatttcagggtccgtgcttttaggcaacggggtggtggccggactataaatctttagggataaaatgttctttataagctcatacccttcccctaaagctgtagtaccctcttcgaaaacatcagcccccagatctatacaaaagaacatgttttctatattatagtactgtattgagctaagcatggcttgattgatgttggcgcccaggacatagcagtagtacatggttgaaaggttgtggtctttgatgcaggcgatccgcatcatctcttctatgtccatatggatcttgtccttttcatacgcctcatgaaggtcaaacacattattaaaacaaagagcacatgttaaccgccacgtattcaggtgtgtatatttttggtaaaaatactgtatggcctctttcaggttatagcgtatggctatagcgtaccagtatttgagtagtaatgtactgagcgaaaactcattatttagcagatcggtttttactattaactcccttaactcccagaaaatttctatcctcatttttatattatttactttttgtaatatcggattgttggaaaacacctcatggcataaaataatgttactactagttttatgaaactttagatctataaaaatttgtaaaatttcttcttcattcaaggtttccttggcacctagctctcgacagaggtcccaggtgtgctccgtgttgacagataccagcccgtagttgatgtccgccccccactctgcaaacagttttataaggttgtagttgttttcccttacagccttcactaacgccgtatttaggtttaagccctctttaatacctgctgattttatgagccttaggttatgatcaaacgtgatcggagcatcatgccaccataggtcataacactttaaaagataatgttggttcgtgggcacgcattgtccagccaacacctttttggtcagagattgcagggaaggcaacatgtctcttcatcttttaaaaaaaaatcaaattaattagccgaataaatttttctttcgagggctttttaaaagagctctttaagagctctttaagagctttttaagagattaaaaaattattcttgctggcattctgccaagtatgcggcattcctatcatctatagtatattatgagaatattcccaaatgatggataagttttttgatttataatcttttaataaactgcttatttcttcggggtcctttaagtttagtggcaaggaagcatctgagctgtaaatatccaaagccaaactatggctcagaaaattataacctttttgttccgctatggcacgaccctcttcaaaggcattaccacccaaatctatacagaaaaatatattaccgatgttataatattgtactgaagtaagcatagcttggttgatgttgccccccagcgcgtaacagtaatatattgttaatggattgttatccttggtagaagccagacatatcatgtcatggacgtctatttggatgttttccttgtggtacatctcatgaagctcatatattttgttataatacaggagacattttaatcgccattcattaagatccgtatatttctcatctagaaaacaaatggcgtccttacaatcgtattgtactgctttggcgtaccaatacttcactagtaaaccatttaactcgtccgtttcttttatttctatgagcccccatagtcttttataaattaagccccttaattgtataacaaatttgttttctaaaataggattattcataaaaatttcatggcacaaaataatactgccgctggttttattgtgcattatcctggtaaaaatacggaaaatatcgttgtcctctagagtttctttggcgcctagctgtctacacaactctcggatgtgcttcgtattgatagaaagcaaaccatagttgatatttgcgccccactctgtaaagagctttatcagactatagttgttttccttaacagctattattaatgccacacgaaggtctatatcttctcctaaaaatcctgattttatttgtattcggccacgatccatacaaagcttgagaggagcatcatgccaccataggccacaatatttcaaaatgcagtgttcatctattgacaaacactggctggctatcgtctttttgacgagggtctgcagagagagcggcaacgacatgtttctttttcaccaaaaaaaaatcaaatgttctcgtctttaaaggttaattcatgttcttaaaatgttcatttcatgatagtgattaataatatggtttaataacgctagaaggcttgtttataagacagtcataagcagtctataagacagtctataagcagtctataagacagtctatgacttagtctataactataatttctggatgggctgtaagatactcttcggctcgtttcagattttttgaagtatatgtctttagcatatcatatatttcctggggttcggttacatctaataccaaggtcacatcacggctgaaaagctgctttactaagaaaatgttgctcaagttatacatataagctttgtgcgcaatgagttgtgccctatcaaaatcggcagcccccaaatcaatacagaaaaacatgtttaaagtattattgttatagatagaaagattcatgccataatcgagactagcccccaacctatgacagtaataaatggccgcgtaatttttttcccgcaagcaagcaaatttcatcatcagattagggctgatgcaaatctctttttcacgacacaactcgtgtatgtcaaaaatgttattaaaataaaggctacaagctacccgccaatagaggtgatttttatgccttttatagaaatagtgaatagcctttgtaaaattatgtcgtaatgccagggcaaaccaaaactttgttaataggtggtgcgccgtatcccccgtcaacggaatgtttgaacaggtgtacgtaactgtgtctaaagtggttctagttacggtttccaagagtggattatgacaaaacatgtcataacccagcagaactcctgcacaggattttagcctggccacttcttttaaaatttccagaagacggggttcggatacaggcgttaagcctcccagttccgcacacagccgctttagatacacggcaggaacacgtataagcccatattcaggatttgcgccccaatccacaaataaacgtataagttcaagattatcgctcttcacggcctttactagcgccgcttcgagacaaagatcatcctcagaaaaacactgtaaatgtttatacgaaaaaacttgcttacaattgttacataggtgaataggacctaaatcccaccacaaaccaaaacgctgcaacgtataatcatagtcacttgaaagataattgcatgccacaacttttttggccaacgtttgtaaagacaacatactaagtttaaaacatcttaaatctaagctagctaactttcaagaaaaccctctatccctaagaatatatcttataactagacttatagcagtaaaaatcaactttggttattctttttaatataaaacgtctaattacttgcaaaggactataaagcccattttcctcagctagaatttttattttttaatgaagtagggggatatgttttcccttcaagacctttgccgaaagcatctttttattcttcccgatgtttttggcgagcatgtactacaacgattaggactgtattggagatgtcacggctcccttcaacgcataggagacgaccacatactcatacgacgggatctcatcctttccaccaacgaggccttaagaatggcgggagaggaaggaaacaatgaagtagtaaagctcttgttactgtggaagggaaatcttcattacgccgtcataggagccttgcagggtgatcaatatgacctgatccataagtatgaaaaccaaatcggcgactttcattttatcttaccattgattcaagacgcgaatacgtttgaaaaatgccacgctttagaacgtttttgtggtgtttcatgtctgctaaaacatgctacaaaatacaacatgctccctattctccaaaaataccaagaagagctgtctatgagagcgtatcttcacgaaaccctatttgaactagcatgcctatggcagaggtatgatgtccttaaatggatagagcaaaccatacatgtttacgacctaaagattatgtttaatattgccatctccaagagggatctgactatgtactccttaggatatattttcctttttgatagagggaacaccgaagctacgttgctaacgcaacatctcaagaagacagcggccaaagggctcctccactttgtgctagaaacgttaaaatacggcggcaacatagataccgtcctgacccaagccgtaaagtacaatcatagaaaacttttagattattttctgcgtcaactacctcgtaaacatattgaaaaacttttgttgctggccgtgcaggaaaaggcttctaaaaaaacattgaacttactgttgtcacatttaaactactccgtgaaacgcatcaaaaaactaccgcgctatgtgatagagtacgagtccaccttggtgataaagattttattaaaaaaaagagtgaacctgatagatgccatgttggaaaagatggtaagatatttttctgcgacgaaagtgaggacgatcatggatgagctttcgattagtccggaaagagtcattaagatggctatacagaaaatgagaacggatatcgtaatccatacttcttatgtttgggaggatgatctagaacgtcttactcgtcttaaaaatatggtatacaccataaagtacgaacatgggaaaaaaatgttaattaaagtcatgcacggcatatacaaaaacttattatacggcgaaagggaaaaagtcatgttttatttagccaagctctatgttgctcaaaacgcggccacccaattcagagacatttgtaaggactgttacaaactggatgtggcacggtttaaaccgcggtttaagcaactaatattagactgtttagaaattattactaaaaaatcttgctatagtatcctggaaatcttagaaaaacatattatttccctgtttactatgaaagttatgactgaagaagaaaaaaacctatgtttagaaatattatataaagtaattcattataaaacaatacaatgttaaaattcaatagatatccatcattaatattgattatattttcgaatattatcttctatggtgcaagataatcatctagcgcgtgaaacatgtcctcttctcttcaggaactttgtcgaaaaaagctgcctgactgcatacttccagagttttttgacgactatgtattgcaactgttaggactgcactggcaagatcatggttcccttcagcgtatcgagaagaaccagatacttgttcaacaggaacccatccatatcaatgaagcactcaaagtagcagcatcggaagggaactatgaaatcgtagagctgttgttgtcatgggaggcagatccccgctacgccgtcgtaggagccctagaaagcaaatactatgacctggtttacaaatactatgaccaagttaaagactgccatgatatcttgccgctgattcaaaatccggaaacattcgaaagatgtcatgagttaaacagcacctgttcactgaaatgcttattcaagcatgctgtgataaatgacatgctgccgattcttcaaaaatatacagactatctggataggtgggagtattgcagccagatgctgttcgaactggcatgtagtaaaaaaaaatatgagatggttgtgtggatagagggagttctaggcgtcggcaaagttacatctcttttcaccattgcgattagcaacagagacctacagctgtattctctgggctactcaattatccttgagaatttgtactcctgtggacaggaccccaagtttttactaaatcatttcctgcgagacgtttcaataaaagggcttctaccctttgtaatcaaaaccatagaatatggtggaagcaaggagatagccataactctggctaaaaaatatcagcataaacatattttgaaatacttcgaaacctgggaaagctaggttcagtatggtgtactcactattgtagtgaatcgtatcctgtaaattttgtaaaaaagcttaaacttttgaccacatcatattgttttagaaatctcaaaccagtgaacaacagtcttatcatacattaaaattccagtaaaatttatattttttttggtaaacaaatgttttctcttcaagacatctgtcggaaacatctttttcaacttcctgacgcttttgatgaatatatattacaagcgctaggactatactgggaaaaacacggatctcttcaacgaataagaaaggacgctgtgtttgtacagcgaaacatcgtcctttctaccaatgaggccctgagaatcgcagcctcagagggaaacgaaagggtaataaaacttctgttatcatgggagggaaattttcattatgtgatcataggagctctagagggtgaccaatatgacctaattcataagtatgatagtcaaattaaagactaccacatgattttatcattgatccaaaatgcaaatacctttgaaaagtgtcatcagttatccaatagtaatatgtggtgtcttatacagaatgctataaaatataatatgctccctattctccaaaaacacagaaatattctgacacatgagggagagaatcaggaattgtttgagatggcatgtgaggaacagaaatatgacatagttttatggataggacaaaccctaatgttaaatgagccggagtttatttttgatatcgccttcgaacggatagatttttctttattaacaatgggttatagccttctttttgataacaagatgagtagtatagacattcatgatgaagaagatcttacttcattaccaacagaacacctcgaaaaagcagccactaagggatgtttcttctttatgctagaaactttaaaacatggtggaaatgtaaatatggcagtcttatctaaagctgttgagtataatcatagaaaaattttagaccattttattcggcggcaaaaatgtttatcacgtgaagagattgaaaacctattattaaccgccataaccaattgtgcatccataaaaacgttaaacttactcttgtcttacctaaactattccgtaaaaaatatcattggaaaaatagtacaacatgtcataaaagatggtgattataccatcatattacttttaaaaaaaaagaaaataaacctagtggaacctgttttaacaggttttatagattattactatagctattgttttataaaacattttatccaagagtttgctattcgtccggaaaaactgattaaaatggccgcgcgaaaaggtaaactaaatatgattatcgaattccttaacgaaaaatatgttcataaagatgatcttggaactatatttaaatatctcaaaaccctagtatgtaccatgaaacataaaaaaggaaaagagacattaattgttcttattcataaaatatatcaagatattcatctggagactaaagaaaaatttaaattattaagattttatgtcatgcatgatgcaactatccaatttctatctatgtgcaaagactgttttaatttagccggttttaaaccatttgttttagaatgtttggatattgctattaaaaaaaattaccctgatatgatacaatatatagaaattctatcgaaatctgagtaaaatttatttttttgatcagagtaagaaaatgttctccctccaggagatctgtcgaaagaacatctactttctacctgactggctcggtgagcatgtgattcagcgactaggtctgtactgggaaaaacatggttctcttcagcgaatcggagacaactatgtacttatacaacaggacctcatcatccccatcaatgaagccctaagaatggcaggggaggaggggaatgatgaggtggtacaactcctattactatgggagggaaacattcattatgccatcataggagctttggagagtgaccattatagcctaatacgtaagctctatgaccaaatcgaagactgtcacgacatccttcccttgattcaagacccaaaactctttgaaaaatgccatgaattagataaatcttgtaacattttatgtctcgtattacacgccgtaaaaaacgatatgctttgcattcttcaagagtataaaatgcatctaagtggagaggatattcaagtggtgtttgaaacagcatgccgttcacaaaaaaacgatattgtgtcatggatgggacaaaatattgcaatatacaaccccgaagttatttttgatattgcctttgataagatgaatgtgtccttattatctatagggtatacgcttcttttcaatcatcatataaataatacgaacgaaaatattaattctttattgacacaacatcttgaatgggctgccggcatgggccttcttcattttatgctggaaactttaaagtatggcggggatgtaacgataatagtcttgtctgaggccgtaaaatatgaccacagaaagattttagattattttctccgtcgaaaaaacttgtaccaagaagatcttgaagaactattattgttggcgatacgtgcagattgttctaaaaagaccttaaacttgttattatcttacttaaactattccataaacaatatccgtaaaaaaatattacaatgtgtaaaagaatatgaaacgaccgttattataaaaattttacggaaaagaaagataaatctgatagagcccattttggcagactttataggatatcatagctatacctatatggtagattttatgcgtgagttttccatccatccggaaaaaatgatcaaaatggctgcacgagaatcgagggaggacttgatcataaaattttccaaaaaagtttgcaaagagcctaaagatagacttcactatctcaaaagcttagtgtatactatgcgacataaagaaggcaaacaactgttaatttatacaatccataacttatacaaagcttgtcatctagagagtaaagaaatgtttaatttggcacgattttatgcacggcataatgcagtgatccagttcaaatcgatttgccacgatctctccaagctcaatattaatatcaaaaacttgttgttagaatgtttaggtattgctattaaaaaaaattactttcaacttatcaaaacaatagaaacggatatgcgttatgagtaacatttttagatgagggaagattctaccaaactaactaagacctttcgctagaatgtatcttattgttaatatagatgagatatgtcattgtgaaaaaatagattaggtaggttgtgaaaaacagattaaacttaaaattatgtgtattatgtaaaattttagaaataaaaatttatttttttttattgagggtacggaaaatgttctccctacaggacctctgtcggaagaacattttcttccttccaaatgattttagcaagcataccctacaatggctgggattatattggaaagagcatggatccgtccatcgagcagaaaaagacagcataatgatacagaatgaattggttctttctatcaatgatgctttacagcttgcaggagaggagggggacacagatgtagtacagctcttgttattatgggagggaaatctgcattatgccatcataggagccttgaagactgaaaaatataacctaatatgtgagtatcatagccaaattcaggactggcatattctcctacccatgattcaagatccagaaacattcgaaaaatgtcatgatttaagccttggatgtgactttatttgccttctccaacatgctgtaaaatacaacatgctttctattcttgtcaaatataaggaggatctactaaatgcaaggattaggcatcgtatccaatccctgtttgttttggcatgcgaaaatcggagaattgaaattattgattggataggccaaaatctgccaattcctgaacctgatgccatttttagcattgctgttgctacaagagatttagaactgttttccttagggtacaagattatttttgattacatgcaaagacagggaatcattcaattaaccaatggagttcgcatggttgtgctaaatcgtcacattagcatggcaatagataatggtcttttaccttttgttctggaaactttaaaacatggtgggaatatacatagagccttatcttatgcagtaacacacaatagaagaaaaattctggattatcttattcgccagaaaaatatagcccctaatacaattgaaagacttttatatctggccgtgaaaaatcaatcttccaggaaaactttgaacttgttgctatcttacataaattacaaggtgaaaaatgttaaaaagctggtagagcatgtagtaaatgagaaatccactcttgtgttaaaaattttattagaaaaaaaggaaaatctagtggatgctgttttaacaagacttgtaaaacattctacatatttccaggtgagagaatttatccaggagttttccatcagcccagaaaaattcattaaaatagctgtgcgggaaaagaaaaatgtgttaatcgaggctatttctgaagatatttgggaaaatcccacagaaagaattacttatctcaaacagatagtgcacaccataaaatatgaaagtggaaggcgatttttggtagacatcattcacagcatttaccaaagttactcactaaaacacgaagatattcttaaactggcaacattttatgtcaaacacaatgcaatcacccattttaaagacctctgcaaatatctttggctgaacagaggaacagaaagtaagaaactgtttttagagtgtttagaaattgctgatgagaaggagtttcctgatattaaaagtattgtgagtgaatatattaactacttgtttactgcaggagctattaccaaggaagaaatcatgcaagcctatgatgctttagagtagccatgtattaacattctgaaagtagaataaaatatactatatactaaaaaccaaattagccatttttaactatcttcttcttaaaaactctggataaaaatttatttttttttaatttgggtagggaaaatgttctcccttcaggacctctgtcggaagaacaccttcttccttccaagtgattttagcaagcataccctgcatttgctggggttatactggaaggggcatggatctatccaaaggataaagaatgatggtgtgcttatagagcatgatcttactctttccatcaatgaagccttaattcttgcaggagaagagggaaacaatgaagtagtaaagctcttgttactatgggaaggaaatcttcattatgccatcataggagctttgaggactgagaactataacctagtatgtgagtaccatagtcaaattcaggactggcatgttctcctccctttgattcaagatccagaaacattcgaaaaatgtcatgatttaagccttgaatgtgatctttcatgccttctccaacatgctgtaaaatataacatgctttcgattcttgttaaatataaagaggatctactaaatgtactatttaggcaacaaattcaaggactatttattttagcatgtgaaaatcggaagcttgagattcttacgtggatgggtcaaaatctgccaattcctgatcctgagcctatttttagcattgctgttgtcacaaaagatttagaaatgttttccttagggtacaagattgtttttgaatacatggaaaaccaaggacttcatttaacccaggtagttcgtatggttatgctaaatcatcactttggcatggtaataaataaaggacttttaccctttgtgctggaaattttaaattatggtgggaatgtaaatagagccttatcttatgctgtcacacaaaataaaagaaagattttagaccatgttgttcgccaaaagaatataccccataaaaccattgaaagaatgttgcatctggctgtaaaaaagcatgctcccaggaaaactctgaacttgttactatcttacataaattacaaggtgaaaaatgttaaaaagttgttagaacatgtagtgaaatacaactctactcttgtgataagactcttgttagaaaaaaagaaaaacctgctggatgctactttgacaagatatgtcaaagattctacatactttcaggtgaaagaatttatgcaagacttctccatcagcccagaaaaattcattaaaatagctgtgcgggaaaagagaaatgtgttgatcaagggtatttctgaagatatttgggaaaatcccgcggaaagaatcaggaatcttaagcagatagtgtgtaccataaaatatgaaagtggaagacaattcctgataaatatcattcacaccatttaccagagttattctttgaaacctgaagaaattcttaaattggcaacattttatgtcaaacacaatgcaaccacccattttaaagatctctgcaaatatctttggctgaacagaagaacagaaagtaagaaactgtttttagagtgcttggaaattgctgataagaaggagtttcctgatattaaaagtattgtgagtgaatacattaactatttgtttactgcaggagctattaccaaggaagaaatcatgcaagcctatgctttggagtatgccatgtattaaatttctgaatcagtaagcaatagatagattttagaatatgctgtattaagttagtttctgaataagtaattaatagatagattttagtttatgtaaaaatgttaacatttgttcataagttttagataccattttagagttacttttttagatattactattttagccattattatcttaaataatcactattttagataggtccccgtattaaaaaccaaattaaccattatctatgtttttaataatactttttaaaaaccctccataaaaatttatttttttttcataaaagtagagaaaatgttctccctacaggatctctgtcggaagaacctttttcttccacttgagcccttaggcaagcatgtggttcaacggctgggattatactgggaaggccatggttcagttaaacgagtgggtgattgctttatatgtgtagaccagatttggatgctatcaatccataaggctatacaaattgcagcctcggaaggaaatgagaacattgtcaagcttttcttactatggaaggggagtctacaatatgccatcataggagccttagagggcaggcaatatgatctgattcaaaaatattacaaccaaattggggactgccatcagattctaccactgattcaagatccagaaatttacgaaagatgtcatgaattaaatgttacatgtacctttcaatgcttatttcaacatgctataagagataacatgctgcccattttccaaaaatatggagaagatctgaatggaaacaggagaatggttcaacttctgtatgagatggcatgccgattacaaaattatgatatcatcaaatggataggatctaacctgcatgtttataacttggaagccatttttagcattgcttttgttagaaaggatttaactttgtattctttaggctacatgcttcttctgggtagaatgagtactgaagatagaaactttatctcaatcataacacgccatcttgaatacgcatcaaaaaagggactttttgactttgtactagaatctttgaaatatggaggtcaagtggatacagtgttgtttcaggctgtaaaatacaaccataggaaaattttggcccattttattcatgaaattccccgtgaaacggttgaaaagctgatactccatgctgtggagtcacgggcctccagaaaaacattcaacctgcttttatcttccataaactactgtgtgaacccttttgtcaaaaaactactgcacgctgtggtggaacacaagtacatgcttatcataaagcttttgctcgagcggcccaaaaagaagataaacctggtagatgctgctctattcaaacttgtaaaatactctacttatacagaaatagtaaaatacatgggtgagttttctgtggacccaaaaagggtggtcaaaatggcagcacgactcatgagagtggacctgattaaaaagatttctaatgatgcatgggaagataaactagagagaatcaagcaccttaaacagatggtaaataccatgaaccacagaaatggaaaaaatctattgatgtacaatattcacaatattactggatatacctatctgaacaccaaagaagcatttaacttaacaagattttatgctgtccacaatgcaacatgtttgtttaaagaaatgtgtaaaagctgttttgtacatgataaaatacagctcagagaattgcttgaagattgtttacatattgctaataggcatgattatatccagattgcagaaaccgcagatgaatgtatcaaatatatagatcttattacatttaagtaaaccatgtatatatcaagtaaatccagattaaatcaggctaattgtaaatagttgtagataccatataatgaatgttttattaggatagtagttcagttaagatagtagtttagttaagatagtagtttagttaagatagtagttatgttaagatagtagttctgttaagataatagtttagttaaaactagttcatgttaagttaatagttttgttaagacaatagttcatttaagtcaatagttcagttaagtcaatagttttgttaagtcaatagtttagttaagtcaatagtttagttaagtcaatagtttagttaagtcaatagttatattaagacattagttctgctaatacattagttttgttaagataataaaaatttatttttttttcatcagggtagagaaaatgttctccctacaggagctctgccggaagaacatttacattcttccttaccccttggctaagcatgtacttcaacaactagggctgtactggaagggacatggatctcttcaacgaatcggagatgaccatgtactcttacagcaggacctgatcttttccatcaacgaggccttaagaatggcaggagaggaaggaaacaatgaagtagtaaagctcttgttactatgggagggaaaccttcattatgccatcataggagctttagagggcgaccgatatgaccttatccataaatattatgatcaaattggggactgccacaagattcttcctttaatccaagacccgcaaatctttgaaaaatgccatgaattgagtaactcctgtaatattcgatgccttttagaacatgcagtaaaacacgacatgctttctattcttcaaaaacacaaggagcaaataagattacacatggcattaacccaaatactatttgaattggcgtgtcatgaacgtaaaaatgacatcattagatggatcggttattccctgcacatacaccatctagagactatttttgatgttgcattcgcccataaaaatttatccttatacgttttagggtatgaacttctcatgcacaaagtaaatacagaggctgcatatatagaattacccaatttgctatcatatcaccttcgaactgcggcggcaggaggtcttcttaactttatgttagaaacaataaagcatggtggatatctggataaaacggttttatccgcggctatcaggtacaagcataggaaaattgtggctcattttattcatcaggttccccgtaaaaccgttaaaaaactgttactctatgctgtgcaggctcgggcccccaaaaaaacactgaacctacttttatcttccttaaactactccgtgcacaccatcaccaaacaactcgtacacaatgtcgtcatctacagttccacgcttatcgtaaagcttttactcatgcggcgaaaaaacaagttaaacctagtagatgccgttttagccagacttgtaaaatattccacctatacagacattgtacaattcatgggtgagttttctgtgagcccagaaagggtgatcaaaatggctgcacgggaatccaggacctttctgattgaaatgatctccaaagctgcttggggaaatcacccacagacgttgattcatcatctcaaacaactaaccaataccatgaagcctcaatctggaaaagaccacatcatatataccatccactatatttatctaaactctaatatgctggtagcggaggaggaaaaaaatatttttaaattagcaaaattttatgcgaatcataatgcggtaaacaggtttaaacaaatttgtgaagactattatatattagatgcacgatttaaaacacttattttagaatgttttgaaattgccgtccagaaaaactatcctagaattgcaaatattgtggatgactatattcgattccttttttacaggggaaatataaccgaggaagaaattcgtgaagcctattctttaaaagatgctgaggtttatgtagatttaaaatggttacaacaaggagaaatggtttaaaccaaatccggtttaaactaaatccaatttaaactacatttggtttatcattagtcattgaaaccatcgaaaaaaaagctatttgtttatccccataaactcatcttttttttgtctcaaagtttgacactaaaattcagtgttttatagtgtttataattaagtgttttgcatgcattgcagaaattttcatcttttttaattggttcaataccacatgtcatacaatatgttgtttgattatcaagattaactttatgaaaggaaagtaagtgagccgcaaatttaaaagtaaaatatctttcatttaaaatgatcttatgaatgtattttcgataaggaggaatgaaagcatttgccaaaataaatcgcataaaaggcttggaaaaacccatatcttctaatcttttgtgggtataaaccctattttggtgttttacaaaaacttcattgttataatagtcgttatagctatcaatcatttttttaagtcctataatgcccaaggttgcacgcataaagccacagtttctgctccaaaaagcatgcacctgtaaagggtgcttttcatataaccaattacaaaatttcattccgcaacagtagcatgttatttcagtgggggatgtatagaataatccggcattcgaaaatttttcataattttttatgtcatggattgcgaagctttgatttcgtgcatctatggagctatagcctacatatttaggttttacttcaaataatcgcaaagagatgtatggatctatcgtatttattttaggaaacatttcataattttaaattcttatatataatataaaaaaaattacaaacatttgtaatgatcatcctcaattgaaggctgagttgtaggctttatttttctaattatacgaagaaggtaggttctcataaagccttcaagatgactattgatgtttccaatacattttctcaatgagttcataaacccagacattttgctaatggcttggcaaagtgccaacaagttgtccacaaagtactggtagattgccactagctatagctagctatagtgagccaacctctctgtatgtattttatatatttcattttttaatagatttaatatttttataaaaaaatatttagttttttatacaagaatgtcgacaaaaaaaaagcccacaattaccaagcaagagctttactccttagtagcggcagatacccagttaaataaagcattgattgaaagaatctttacaagtcagcaaaaaataatacaaaatgctttaaagcacaatcaagaagttattataccacccggaatcaagttcaccgtcgttacggtgaaagctaaacctgctcgccagggccataatcccgccacaggagagcctattcaaattaaagctaaacctgaacataaagccgtaaagatacgagcattgaaacctgtccatgatatgttaaactaaactataaagtcatattcttctttatcgttattatcttcaatatatttttgccaatcgaaatcgaataaattcagatcctggacatttaaatacttatcatcgtacattttaatataatttaaacatgagttgttgtcaaaaacttttagcgtttttgttaaaattatcatatgaataatttccttattaagagttgccggaataatacaaaacctatttttaggtacatcatccatgataatagtaaaattagtaaaaattgtttcttgtttttcttttgtttcaaataaacgttgtaaggttaaaggtttctcgttcaatggtttctttgaagataaaaagaatgtataatctggtttaaaggtatttttggtttcaatcgtgattccatctgcttgagcatatactaaaccagaccaaatataacggtccactattacaatataatttagcttaagtagcactgcaatttctgcgataaattcactacgatgttttgtaaataatttatgtaattgttccgatgacatttctatggttttatttaacacctgcaatataagatcaccggtggtcgtgtctggattaggaaaatgtatacatatagcattataatccatgcattccaatgtttcttttaatttcattgcctgtgtgctttttcccacaccattgattccctcgatggcaatgagtattccacgcatgattaataaaaggaaaaaaagaattcagtttttaacatttcttacaaatctttttttatacaacattgtacaacactgcattagcggtatatgatgttatagcttcattaaatatttgcttttatataatctttaccaacctatatttggtagatcactgcagatggtcataaataggccataactaagataaaaattatttcagacgctactacggtagtattattaaaatcatgtgtggcaatgtatgacgtcttaatagataaaacatttaaggaaaacaaatttgaataaaaaaaataattgttatgatggcgttgttacacaaagaaaagcttatagagtgcatctatcatgagctagaaaatggcgggacaatattgcttctaacaaaaaatattgttgtgtcagaaatttcatacattggcaatacttataaatattttacctttaatgacaatcatgatctgataagcaaagaagatcttaaaggagcaacatccaaaaacattgctaaaatgatttataattggattataaaaaatcctcaaaataataagatttggagtggtgagccgcgtactcaaatttattttgaaaatgatttatatcatacaaattacaatcataaatgtataaaagatttttggaatgtttcaacttcagtcggtcctcatatctttaatgatcgtagcatttggtgtactaaatgcacatccttttacccatttaccaacattatgtcgcccaatatattccaataaattagatatctttgctattaaaatagttaaaaaccttataggataattaggtactttattacgataaattatgatattttataattagttactttattataattaatctctttattaatgaattatcataagataactaattatttttttccatatatcagataataaatctgatatgggctaaaagtatgtttcaaactatttacaatagaatttctgttaagaaaacatacataatttgaataaaatttttttaaatatcaccgaaacaatcaacatggtgttaatagagtttttaacaggtttcttctatttatatggaaagagactgttttccattagtaaagtcatggacatgatatgtctagactattataccattattcctgctcctctggcgatgatgttagcggcaagactaaaaaactatgacctcatgaaacgactgcacgaatgggaaatctctattgactacgctctacttgtagtagatgatgtgccgtctattgactattgcttaagtcttggcgctagatccccgactagagcacaaaaaagagaactgctgagggacaacacgtttaatcccgtgtataagtatcttatgaactgttccggcttcccaacaaagagagaaaaaaacattccttgtgatgttcaatgcgaaagactgcaaaaaaacattataaaagaactggtatttaactgctctgtactgcttgaaatggtactgcacacagaaagagaatatgcatacgccctacactgtgctgcaaaacataaccaattgcccatcctcatgtattgttggcaacaatccacagacgcggaatctattttgttgaaaacctgctgttctgataagaacatcaattgttttaactattgtattctatatggcggcgcccaaaatttggatgctgcaatggtggaagcggcaaagcacgatgcccggatgctgataaactactgtgtcatgcttggtggaagatccttaaacgaagcaaaagaaacggctgccatgtttggacacattgaatgcgcacaacactgttttaaactgcagtcttacgtcgtggacacatcgaatacagacgacactgattaaagcgacaatcttacgtcatgaacgactgtcttttgagtatctatacttacattatatttttttatgaaaaaaatataaaggttgtatacaaacctttgtatacaagaaatttggatcattaaacaataattaatttggacacaggaaacgatctagatcgatcaaaaagctattttttttgcacacagaacatttagataattgagagattactttccatacttgttaagcttttttacacacaggaactttggattctgttcaggaagtttttcatagacattatgtttacagccagtaataataattttgggctttttcttaaaccaccggtggaaaacatccagcttgtaaagagggaaatgcatgtagagaggttttggtagtcatggttaagagatttgactaactccatgtttcctgtaaagactgcccagtcccaagcagtaaaacctctatgatagtctttttgagtcggatctgctccaaattttatgagagaaagcatatttaaagaacggccccgtattgcggccttcatcacaggagtcatcccattaaaattcggtaaacaaattctggtcccattttttccgaaatagcccaacaccccttccaggattaaatgattttttttctcagctaaataatgtaaagcagagtttccatctttatccctcctatgagggttaattatttctccaggataagattcttgttcaaaaagaaattttaaaaagtctatacgtccgtagatgcatatccacatgaataccgaggatccatttttatcgcatctattgacaatccacggatctgttttaaaaaattcctcaaatagtgtaagattcccatttctaatatgttttttaatccatttaacaaacaagttttctatctccctttctggaaacatgtgttccattttgaatgtcgcccctactccactatatgattttactcctttaatttttaatgtccttttttttcggacttctttggataagctgtttattaccatctttaaatgccttatagcggggaggagccaggcccttttcccatatgtgcggtaattcttggtgtttatgcttgcctttggcataaccaggccagtatttttcgatatattcagggtttgtttttacgtattctttaaaggtccgataggcttcttgaatacaggtaggctcaccggtataatttccatgttcatcttcctttaaaaagccattaaccctgtcctttctccacttaagattgtgctttccaaaaatgcgatcaagatcttgcgcctgctggggtggaatcataaatccctttttaggtcgaagctttttattttttccatagcttcggccatcgcgttgcgaaacagtggttaggacgcctgatagtctttccatgggcgtcgcatctaatcctatccatccaccctgatgaatatcaatggcaacaagctctcctttattttgggcaagccaagtttccaagaatgccatgctttcttcccagggataaggcccgccaacaccacgggttgtccaatcttgcaaggactccaggtccgacacctggtaaggctctaaagaagacggttccttgtttttgtactgcaaataagatttaatgacccatttataccatgtgtcgaaccgcagcgtggcgcctccaaagtgaaagccgtcgttgattttaggatatctgcaacatatttcaaccgtacgtttgagttctgcaaaagcggccttccaaggaagtctttcgctgcgggtaagacggtctattttgccctgcgtgccatagcgtatggcatgtcgtgccaattgcaacaattctgacaccgatccgtgggccccgatccagtttatcggataggcaacctccgaagggtttaaaagatgctcgtaaaagcgtggatcttcagatgccaaggcgtctgcaaaggggataatgctagaaaacctgtctagacatacgttttctgtgtttacttctaaaggtagaaaaatggttgcgtgaggcttttgaacctgcttgttcagcggtctgcatatgctttgaataatgtctctaggactatgtcgcggcgctgcaaaaaataccgcgtttagttctggaacctctacgccctcttgaaagagtcgacagtttaataaaataacgggttcctttgaggaacaaaattctgtaaatgttttgaggataacctgtcgcggcagggttgagtgagctatcagggcatagaccccttggtctaccaacgccgcgtatagctccttggcctgtttaatatcacgggtaaataccagcattttaggagccggtatattggtttttaaataggctaaggccattataatttgctttactatgatctgtttcgtggtctcctctttggtactcggttggtgggccaatttaggcgcggctaccatctgcaattcaaaatcatttacatagccggcctctatgccttctcgcagatagtagcgaaaggcaacgccgccaaaaagttcacgatttttcatggaaagcggggtgtcgtacctgggcgttgccgttaaaaaaagtcggtgcccttttttaaagttgagcaacacgtgggtaaagggccgtgtctcccattcgccgcaaatccggtgacattcatcgctaataataagatcgaaatcatccaccagtagcgtggaggattggtaggtggcaatcacaagaagagaaggggcctcccgtatccgttttgcaataaagacaggattggtggtcatttctatattgtcgtgatttagcacaatgcgggtctggtcagaccccacaagcaaaacgttcttcaaagaaattccatactgatagagtttttccagagtctgccgtagtagggacaggcccggcaccaggtacaaaacttttccttgaagataattggagaggataagataggcgacgcgagttttgccgcatcggcaggccatctgcagaatggccctcccacttcgccgcagctcctgatagcccatattggccgcctccttctgataaagtcgatcctcgattgcagtccgtgtctcatctgtagaaaaaaataatacgtcatctgcgaaatgttcatcttccacaggagttatcaccaggtgtctcagtttctccttgcttatcagcggatcagagggcaaagatggctcaaccactatcgtggaatcattcatctcataggcgggagaatcacacaaagtatagcttatgtccagacagtttgcaacatcctcagccaattgttttattttttcgggtaaaagacatacgagttctttgtttttgacgcgaaaaaactgtgcacaatataacacccctgcttcaattttttgcgcatccttctttgtagatgtttccaatgtgaaacaatacttccattcatccgtaaaacaggttgtataagatccatcatgaagcctagcggccaagtttcctgtgtgcccaactttatgtaaggattgggcctccagccagggatgaaccgccacgtaaaatcctgcgcacatgctatatcaaattgcagtttcttaataactgtacacaggatctgaaaaacatgtgattacaaaatttagataagaaatatttaatattaaaaatcacagaatacatgtcactgtgtagagagaaagccaaaaactcctcttgaccgccgtgggaaatcatccagggtagtaggttgtgtttcataaagttgtatgccgtagtgatcaccgtggactccagatggttattggcatctttgcaatactttgccatcttggcagaaaagacgataaatccacaaattctaccccagttgataagatccttaaacagctcagtcacaaccccagtaaactgggttttaatttcttgaacactcgtaagagaaaaggtaattgtaacctgtttgttcaaacactcatcataataggttaaaattttttttatttgttgttgatatgggctaagctcatgctctgaaatatcattaatgtaatatttaatatatcccactagtatttcattaatgatattatgatatattaactcttctccctccatagcggcaccctatatttttttatttaggtttcaatgttatcacaattgcgatacaattgtgatacaattgtgacacaactgtgttgtatacaacaaatgttaggccacgtatagcaacctatatgttaagaaatatttttatcccaacattagttggaaacgagcagccgcaaagaagtcatttaaaataagccatttaaagatttagaatttatatgtatacaactgtacaatggaagcagttcttaccaaactcgaccaggaggaaaaaaaggctctccaaaattttcatcgttgtgcttgggaagaaactaaaaatattataaacgattttcttgaaatccctgaggaacgatgcacctataaattcaactcatacacaaaaaaaatggagcttttatttacccctgaattccacaccgcctggcatgaagttcctgagtgcagagagttcatattaaactttttgagactcatttcgggacatcgagtggtattaaaaggccctacatttgtttttacaaaagagatcaagaatctgggcattcctagtaccatcaatgttgactttcaggccaacattgaaaatatggatgatctacagaagggaaatctcatcggcaagatgaatatcaaagaaggctaaataaaacaactaacatcaaaaaacattaaaggctatgttgtggacgatgcctttgtctcaatagtttcgaggtcatccaataactcatgtaacgtaaaaaagttggtccatttttttgaaaacattaaaagacgttcgtcttcataaataaaaaagtcattcgaaggaaaaatgatatactcaataccatagtcttgtaatattttttttaggtctctcagggtccagggatttaccaggcttctacgcgaagtgagcatcataaaaatatctaatattttttgcgccataagccagcgcggattctcattggcccacaaatcaacaataattctcttatcaaccgtgagcattcctacttgattcgaagaaatgattagatgcccagcagtccaccccatgagtagataacgcagcgttgtagaaatgtcacatatggaaggcattcctccacaacatgaacccaaattaggatgcgtgtgaaacacaaacatagcaggcttgttggccaccctgctataaatatcagcaggcatcatagcctcgctgccaaaataaatgttctctcctgccctataggggcttggaatgatttccactatctcgggtacaccgtttatcatattaatgcggccgcaccattcacggtcatcgtccaaaaattttttgatggcaccccgaacattgtcccagttaagcaacagagtattcacaatctcattacgctccgcccagtattccttaaaacttcttttagacttgctgagctgttcccaggattcgaactcagtccaatgttttttttcttttggggaagacttcccttttgaaacattttttgcggctccaccatctacactatgattttccaaaataatctccttcatcgtttgagttatatgggcattgctaagcaccttagtggtaacctgtttacctatgtgatttagcagaaaaccaagtttgtccatttgtgtctcaaccatttattcttaacaaaacaaaaaaaaattaaaaatcatcgtcgtttaaaaagagtttgaaggcaaacgcatcatccttaacacagttctgatactgcgtaggtcttaactcgaaaaagttggttttttctacttcattaagaaagaatttagtcatctgaggaaaagggtttcccaccttataaatgcttttgcactgcatcatgaagcacaaattatctgtaaagtagcgtatatattgaaatagcatttcttttgaaaaaccgggaactcttcctcttgccttgtcaaaggcatagttaataaactcatccaccaactccacagcctccttcaaaattttgtgaatgatcttttcctcgggaatgttatacacgtaatttgagataagaaaacacgcaaaactacagtgcatcccttcatcacgtgagataaactcattatagcttacaagccccggcataatattctgttccttaagaaactggatcgccacaaagtggttttgaaataaaatgccttctacggcggcgaagcccaccagccgctcacctagagtgttcctgtcggggtccatccactgccgcacccactgcgccattttttttatgatagggtgtttttcaatgccgctaaagatgcgctgttgttccttctcatccgggatcagcgtttttacctgtattgagtaggcttcgctatgaacgcactcttgggcagcctgcattgtataaaagtataacacttcctttactttaatttcgcgcataaaattggttaaaaggttttcgataacaatttcgtcggcaacaacaaagaaggctaaaatttgtttataaaattcgcgctgtggctttggcatggcttcccaatcatcaatgtccttacacatgtccacctcctgcgccgtccacgtcaaactttctaattttttataccagttccaacattcggggtgctgaataggaaaaatagtgaaacgttgggaattttcaattagtaattcctccatatttgaaataaatattaacatcttcaaatttattggctgccatggagacgttttttattgagacgttggcatctgatgtgtatggaaaggcgttaaatgttgatttagatagactatcgcaggcgcaggttaaatatacccttcaagagcttatttcctactgcagcgctctaaccattttacattatgactattcaacccttgcggcgcgtctttcggtgtaccagctgcaccagtcaacggcctcctccttctcaaaggcggtgaggctgcaggccgcacaatcctgctcacgcctgtccccccagtttgtggacgtcgtttacaagtacaaagccatttttgacagctacattgactatagcagagattacaagctgtccctcctggggatagaaaccatgaaaaattcttatttgttaaaaaataaagatggggtcatcatggaacgcccgcaggatgcttatatgcgggttgccatcatgatctatgggatgggaagagtggtcaatatgaaaatgattctgctaacctatgacctgctttcccagcacgtcatcacacacgcgtcgcccaccatgttcaatgcaggcaccaaaaagccacaactctccagctgtttcctgctaaatgtaaatgataatttagaaaatttatatgatatggtcaaaacggccggcatcatttcaggcggcggcggtggaatagggctgtgcttgtcaggaatacgggcaaagaatagttttatttctggtagtggtcttaaaagtaacggcatacagaattatattgtgctgcaaaatgcttcacaatgctacgcgaaccagggaggcctacgtcccggagcctacgccgtctacttagagctgtggcaccaagacatctttacatttttacaaatgcctcgcctaaaaggacaaatggctgaacaacggcttaatgcccctaatctcaagtacggcctatgggtccccgacctattcatggaaatacttgaagaccaaatacacaacagaggcgacggcaaatggtacctcttttcgccggatcaggcccccaatctacataaggtctttgatttggaacggtcgcagcacgaaaacgcacaccgcgaatttaaaaagctttactatcagtatgttgctgaaaaaaggtacaccggcgtcacaacggccaaagagattatcaaagagtggttcaaaacagttgttcaagtagggaatccctatatcgggtttaaagatgccataaatcgtaaaagtaatctttcacatgtaggcactatcacgaactccaatctttgtattgaagtcacaatcccctgctgggagggtgataaggctgaacaaggtgtttgtaatctggccgcagtaaatctagccgcctttatacgtgaaaatggctacgactaccgtgggctcatagaagcatcaggcaatgtcacagaaaatttagataatattatagataatggctactaccccacagaagccacgcggagaagcaatatgcgtcaccgacctattggcatcggggtctttggcctagccgacgtgtttgcgtctttaaaaatgaaatttggttcacccgaggccattgccatggatgaggccatccatgcggccctatactacggggccatgcgacgatccatagaacttgcaaaagaaaaaggaagtcatcccagctttccggggtctgcggcctcaaagggtctactgcagcccgacctatgggttcgctgtggtgatttagtttcctcctgggaagaacgcgtggcacagacgacgcagggtgtgttgacgccgaaaaggtggtcgcagctacgcctggcggctatgcagggacttcgaaatggatatgtcacagctcttatgcccaccgcaacctcctcaaattctacaggaaaaaacgaatgttttgagccctttacatccaatctatatacacgtagaacgttaagcggggagtttattgttttaaataagtatttaatagacgatttaaaagaaattaatctttggacagaagccattcaacagcagctactaaatgcgggaggtagcattcagcacattttggatataccggccgagatccgcgatcggtataaaacctccagggaaatgaatcaaaaaattttaacaaaacacgcggccgcacgaaacccctttgtatcccaaagtatgtccttgaactattacttttatgaacctgaactaagccaggtacttacagtgctcgtcctaggctggaaaaaaggtttaactaccggttcctattactgtcattttagccctggagcgggtacccaaaaaaagattataagaaactctgagaaagcgtgtaatgcggactgcgaggcgtgtcttctgtaggtgtctcgcggtaaaagagcagcggggaccatatggtaaaccccaacaagaggataatgaataaaaaaagtaaacaggcatccattagttccatattaaatttttttttcttctatataatggaatattttgttgcggtagacaatgaaacctccttgggggtttttacttctatagagcaatgtgaagaaacgatgaaacaataccccggcctccattatgtcgtttttaagtatatgtgtccggcggatgcagaaaatacagatgttgtatatttaataccctcgttaaccttgcatacccccatgtttgtagaccactgtccaaatcgtaccaaacaagcacgacacgtattgaaaaaaataaacttagtgttcgaggaagagtctattgaaaattggaaggtttcagtaaatactgtgttcccccatgttcacaacagattatctgcgccgaaactttccatcgacgaggctaatgaagccgtagaaaagtttttgatacaagcaggacgactcatgtctctgtaaatgtctcttcctttatgggtgacgtctcttcctttgccgaggaagtctctgttatgggcaagaggtttgaaacaacgcaaggactctgcttaatctgctgtctcacaaagggaatcaaactacctgctttcgtatttttaatgtagtaattacccttgttgtgatgaattttaagaccatagcgtagtcccagtactttattaatgaattttaaaattgtttgagggtccgttttattgggctttttaagcttaaactcaaagctgatcgcgcttaaatcatactgaacaaattcatcaacgagtttcgtcattaattgttcattggtcaatatattagggtcctgaacgcatttaaagccgcacttagttaatagcataatagcgtacatatgagattgaaaactataattaaattgtagatcatgatgctctgcgtgttgcatggcccattgatgaaagtttaattcctgagtttgtaacatagtgagcgactcgtatactgtctttccgcggcttatttggacacggccagtatagttctgttttgtcataaaactattgtattgttcaacaaatttgggagtaattttatgaccgtgccatgcataaaattcgagtagtttatacttttcatacgcaaataggtcttgctggtctactgtgatgccttcctttaagttttgtttaatttgtaaagctttattggcatcaatggtttcagccgaggcaatgtttacatagtcctggtgtttaatttccattttaatgcttgtatattgtttgactgtctccagcttttcacccgtcagtataaacaccttagcgccggtgtcggcgatctggttaataaatcgggttataaagtgattttttgatagatgttgtatccgcattgtttcgagccatagatggtagtatggagttttataatatatcggcctacctgtttccttactatacgtgaaggaaagctggtgattgcttatggtctgaaaaagggtgtcacgtttttgtaacgtaaacatttcaatgtcttcgatggtttctggatagtaattttgtttcccctgtaagcagattttataacacttactttttaattcacgcacgcggcccaacatttggcaacatgtttctacgtcacacgacatattgttaaaaaagccgtataaaacatcaaatctcttatcttcgtatgaaacacccgctgaaatcgtgggcgtatagataaggatatcaacgagcccccaataatacgatacattattaaaatgggattcccgttcatgagcagtgcttttagaactataaaacccaatttttttttccggaaactttttttggataaatgattgcaacagccgggcctccattaatgaatttgtagggataacaatttttttgtcttctagcaaatcctttaaaaggttatttaaccaagtttctcgtgaagaggtaaaataatacgtgtcatgctgggcccttttatattgattccagtgaaagaagatagggacatccccgcgaaaacgctgtagaatattatacgttcgatttcctaggtttgcgtccaagcatataacataatttgccgtttcgagcatccacatgaaaatggcaaaagagggagcaaagtatttgtgcaggccgctattgaattgattaaaaatcgattctacctcatccaaaataagtaggtctacaggctcggctgtggaggttagccggaaaagtgattctacctgaatgatgactctttcgtagctgtccaaatctccagttacttcgctgtacaatgtgaaattcggtagccgggattgtatattttttgagaagatctgtcgaaacgtcacaaaccgtatggtttgttgttttgaaatagaattattgccgtagtatttttgcaaatagttgcgcagttggacggttttacctattttcatttgagcctttacaacaagcgtagggactcgttcatattctcgcatactactttcatcatagatgtgtttttgagtatcaggcagttcttcaaagagaatggactcatgaacctctatgctctttgtcatcacttggtccacatatgtttccacaaaattatttgtgccggaaaggctgcccatgagaaggctatgtttattgtcatggcgacagtgttgatacactttgtttcccgtgactcttaaaattagggtattgtccttatcatgcatacgcttacatatttcgcagtaacttggacttgtacgtttaaacaatactaaatttttatgaacacggaggaagcaatgatttttacatagtgttcctgcaaattttaatacctcttcaagttcactttgttggatagtatcgcaggaactcggtgttgtttcttttacatttgtgaagatacaaggtaaacacgtcgtttcaaagggggttgctataagggtatcactctttttcgtggttgtactggtctcaaacacctctgcaagctcctcattaaacattttaacacgcatgctaccttttttatgagaccctatgatgcgaaaattttgaatacttttgttgacctgggggtcaacaaaaggataaacgtgtttgggaagattttctaacactttggatgtaaagactttggcctcattattgtttaatactgagtatgtataaagtatgatatgaaaggagtatttaagttctcgctttttatttaatccgatagaatctgttagcaaaatttgttcacgcgttagattgatgttataaggtaaagaatatgtctcgtaaaatacatccatgatgacgttaattatcatgtcaaggatgtcatagacattgtcttcgacattatcattgtcatcaacattgtcatcagagtatgacttatttaccggaaagtcgatgtcaaattttaagcgctgaggcaaaaacccaaataccacttcgtggaaacacttctgctcaaagggctgagccgcctcccactcccaaaagtcatcacgacttgaaaaaactctaaaaagattattatattcatctcgcaccacgaagtgattctttaaggtttcgagagaatatttatcctctacggcttctccttgggagttacagcgaagaaacttgaatgtttcttgcattttgatatttaaaattaaatcaattatgatgcggccgctaatgcggcggttgacgcggccgcgccgctgacgcagccatcatacataaagcggcatggccgttttataacgactagtcggccgttatatgacgaactatataaaaatgaattcttttaattagagttaagtattgttgattgtataatccatcatggttgagccacgcgaacagttttttcaagatctgctttcagcagtggatcaacaaatggacactgtaaaaaatgacataaaagacattatgaaagaaaaaacgtcttttatggtatcattcgaaaactttatagaacgttacgataccatggaaaaaaatattcaagaccttcagaataagtacgaagaaatggcggccaaccttatgaccgtcatgacggatacaaaaattcagcttggagccattatcgcccaacttgagattctaatgataaatggcactccacttccggcaaaaaagacaacaattaaggaggctatgcccttaccttcatcaaacacgaataatgaacaaacgagtcctcccgcctcaggcaaaacaagtgaaacacctaaaaaaaatcccacgaatgcgatgttcttcacgcgtagcgaatgggcatcctcgaatacttttcgagaaaagtttttaacaccagaaattcaagccatattggatgagcagtttgcaaacaagaccgggatcgaaagattgcatgccgagggtctttacatgtggagaacccaattctctgacgaacagaagaaaatggtcaaagagatgatgaagaagtaatatttttggtaaaaatatttttatcaaaatttttttaccaaataataaaaaatattttttacttttttttcttcataatatacatagaatgcctacaaaagctggcacaaaaagtaccgcaaataaaaaaacaacgaagggctcctccaaatctggttcttccagaggccacaccggcaaaacccatgcttcttcgtccatgcattccgggatgctctataaagatatggtaaatattgctagatctagaggcattccgatttaccagaatggatcgcgtcttactaaaagtgaattggagaaaaaaattaaacggtcaaaatgaatataatcaggaaacttaagcctggaacaattagccttgtgctgggacccatgtttgccggcaaaactacgtttcttattcattgcatttacatgctcgaacgtttggaaaaaaaagtagtcttcataaaatctaccaaaaacacccgagacaaaactattaaaacacactccggtatacagctacgacccaaacaatgtaaaatcatagaaagcacacagttatctgacgtgggttctctcaccgatatccatgcagttgtcgtagatgaagcgcatttttttgacgatttaatcacatgccgcacttgggcagaggaagaaaaaattattattcttgcgggactcaatgcttccttcgagcagaaaatgtttccgcccatcgttcgtatttttccttactgcagctgggttaagtatattggccgcacctgtatgaaatgtaaccaacataatgcatgctttaatgtgcgtaagaacgcagacaagacgcttatccttgcgggaggaagtgaactgtacgtaacatgttgtaacaactgtctaaaaaatacatttattaagcagttgcaacctattaaatattaaaaatcttatacaataatggatcattatcttaaaaaattacaagatatttatacgaagctcgagggtcatccctttctttttagcccgtcgaaaaccaatgaaaaagagtttattactctgctaaaccaggccttggcctcaacgcagctttaccgcagcatacaacagctgtttttaacgatgtataagctagatcccattgggtttattaactatattaaaacgagtaaacaagagtatttatgcctgttaattaatcctaaactcgttactaagtttttaaaaataacgagctttaaaatttacattaatttcaggctgaaaactttttatataagtcctaataagtataataatttttacaccgctccctctgaagaaaagactaaccatcttctaaaagaagaaaaaacttgggcaaagattgttgaagaaggaggagaagaatcctaagtcgcttacatttttttttgctatttttatagaatgtacacgcatgttgatgttgtcggaatagctgaagcctcagcggccctctacgtgcaaaaagatagggatcgctacttagacgtgctaacaaccattgaaaactttatttaccaacacaaatgcatcataacaggggaaagcgcccacctactctttttaaaaaaaaatatttatctttacgaattttactccaacaatgtggcggagcacagcaaggctttggcgaccctgctttataaacttgatccggaatacctcactcgttacacagtactcattaccaaaattcccaaccattggtatgtgattaacgtagatcagcgagaatttgtgcgcctatatgccatcccggcagttaaacaacacttaccgattcccattttacccttctattgcaccagcgcactcacccagcaagaattgttttgtttaggacctgaactgcagttaatacaaatatattccaagctctgtaaccccaactttgtcgaggaatggcctacgttgctcgactacgaaaaaagcatgcggatgttatttttagaacagtttccgcaaagattggaaatgacgggcgggaagaaggaggagaaggaaaagcatgaaagtatcattaaaaaaataatactagaaatggtctctacccgtcagcgaatcgttgttgggggttacatacaaaaaaacctgtacaaccatgtactcaagaatagaaatcgtttacagcttattacgagcttaaatatttatgaagaaaaagatatcatccagcaattttgtgattcaaatggactgaagatcaaaatacgtatcaacaatccgctcttgcctacaaatccggaattacggcgtttgactatttattttaatcataataatgatgatgatcagtcatatctaatagtagatatgtacaacacgggaagctatgagctagtgcctacaaatcagataaacacgcttgatggcagctttttaataggaacacccttcgtgcaagcgcgatttttgttggtagagatctgggtgcttatgcttattgcgcagcaaactaaaaaggacaccaaaaaaataatacaattttttataaatcaatatgaaatgcttatgaatagtccttggcccagtatggaggccctttttccctcaagcagtaaaagatatttaggcaactatgtagaccctaacgcgctcataaagtgggcacaactcaaattaaaaagaataccgcctttttatcctggaaagccggatgaagaatcatgttaagccgattaaaaaatcatgttaagctggttgaaaaatcatgttaagctggttgaaaaactcttggtgaaagcacggatgtaatattaacattggccgctcgcatttcgtgttgaaatacgatggaagagcgacggctatctaccatgccgatatcggcctggacatcacagttcatgcacttgtagatgggatgactcgcgttatagatggcaggctcgccacagtttctacagatgtaggagatgcagccatccgagtcgtcgtgcgatttttctatgatggtttgcatggcgccctgcgccgtaagcacccaatgctccatttctcccagacgaagacctccgtgcgatcgtttgccgtccaacggctggcctgtgagggcatccgtgggcccatagcttgcaacggcgtatcggtcatccagcacaaatttttgcaggcgctggtgataggtcggtcctatgaagatggccgcatcaaagtactcgccggtctggccgttgaacattttttggcatccattgaagcgtagaccttcttgcgccagtctttctgaaagaagctgcacattaataggcaggaatgcggtgccgtctgttaccaccccctgtagggcatttgctagaccaaccgtggtttctatcatttgaccgttggtcattcgggagggatgtgagtgggggtttacaatgaggtcgggctgcaatccgtcctctgtgaagggcatgtctgaagtgggcagggccagcgccgcaatgcccttgttcccgctgcgagaactcattttgtcgcctatattgagatttctttcatagcgcaggcgcatgaggccaaagatctcgtcattaggcccatggggacgcatcacagcatccacgacggccggctcatcgaagccgtacatgacagaccggtcgatgtatttgttgagttcgtctttttcgccccgtattttggccacttttcctataatgatgtcgccctttttgaccaccgttcctacgggcacgaatccatctacaagcttttcgtaattagcaccaggcttaagatttttggtgattaaagggtcgggcttcccaaacgactctatatcgctttctaattctactttttcttctcggtagaaggtgccggcaaagccgcccctgtcaataaaggactgcgacacgatcacagagtcctcctgattgtagccgccgtagatcatataagccacaatggtattaagcccgttgggtatgacatagttatgtgctatggtctttacaagcggcatttcattgtaaaactggaagaagcggttcatgtcgacacgatatggccagctaaagcaataccagccccccgtttgccggccttggtttgtttcataggtaacacgcgcaggttgggtacagtttgcgtagggggacactagggcggcaaggcccaaaatagcttggggcacgtccacgtgtgtgaaacgacgcgttacatcatgtttatgtttgcgtagctcgatgatggagaaggcaacaagacagttttccgcctcctcgggggtaatgaactcacagatgccctgtgctacgagatcttcaagtgtaagcgttccggctaaaatgtcttttgccatttgaggcgtaaatcgcgtattttgaatgaaagggattttatgtttttcccagtctttatcgcctttttttctggcctctgcggccttgtagcaggcttgattgtatttttcaatattattatctacaatgagtagggggcgggtcagcctaccgacgtccaaccaaaattctacttcgtctaccatgctatcccagtagatggtggtatggggatgcacaaccttgccctcacggcgaagcattctataccgctgagcaagctcaaaggcattggtgcagcagccgatccattctccgttgataaatacgcgcgctaggccctttcgtacaatgtccttgttggaaacatcggctaactgttgaatggccggatctgatagaaggcgttgttttaacgaaagtacttctccggcggtgcagacattggcagtgatggctaactgtttagacatgcctactttttcaccagtatcggctgactgggctacgcagatgtatccaggataggatgcgtgcacgcgacgcatcatgtcagccctttctgtttgtttggatgcgttggtggtgttatgagtatttaccgtacgcaatgctgaaatggtatttaataaattttttctttccaaactttgagtagatactctgtttacaatggggcgctgtcgcaccatgatggttttatttcctgaaatgatagactgttccatactgcgattaagatcggaggcggtattttttgataaagcggcagaaaatgcctcgataatgtttcgctgagtaagctcctcaaaggctgtttgtttaagaagttctttgaacccattgatgatgggtgctatcacggaagtattaaaaatagccttaaaggccttggcgagtgagacccctgagccgtgcacccgcttggtgcggtagctatcacggtccgtgggtggaaacacattcataatgacaagaagtattttatgaataagcaggcctaaaaagcgcagctttcgtacacgtgtatctgcggtttggcccatgtgtggcagcaatattttgtctaaaatagtaagttgtctttcatttaagtattgtaccgcattttcatcgcttttgtaagcagatgggtttgagacaaatttggaaaccttctcggataaaaactggataattttttctcggttcagctcgtgttggaccggttgaaatatggggtctaaaacatgaatggatttttccagaatttctatcatgaaggtattcacaagggagttggattctagatcaaataccacttgctcaatgatgctgtcatcgcctgtcattccaaacatgcgaaagatgagataccaaggtatgcgaagttttgagaacttggtgctattgatttcaatggtaatggcgccggtggtcatgtagcgtataataatttgagagctattttcgaaggcacctcccggttgggagataaactcgccgcgaatgatttcattattcccttgttgcatggtatggtaatggatgtgaagcgtgttaaagcggatgttttctaagaggtctacgacccattccccgcctcgggctataaagtagccgccgggttcattagggtcttctcctatttctttttttgcggtttttgataggtgatgagtgtggcagcggttgctgccccgcatgatgggaaatgtagatacctgaaaaggaggaatacttgctcgttttacctcctgccgaccattgctgtagtgcgccgttaaaataacctcggcggctagattaaccgggcccgaataggaaaggccacacaggcgtgccttattgggtagtaaatttatcttgtttccctgtgaatagtttcgatgttgcgggcgttcaatgttcacatctgtaaagttaaattggatctgaactgattcccgaagcttatctatttcagtatggtcgcgttggtctttataagtaatatccacgttaaacatttgttttacaatttgcggaattccattgtccataagatcgtcgaagcttttgatgttataccctatcaatcctgtagagtttactgcagcggagataaagctcagcatatcagcctctgtaagctcctcattatccacggtttcaatggggccgtaggttatttgcggccgcaagggttccatgattatgaagtactacattaatattcagttattctttaaaataaatctttatttataaatcttatttataatataagaatgccttatgcaagagacatcacaaagtttattacggcaacggaaccagaggtgggtcttcccctgttggcgctgcagcgctccaaatccatcataggggttattcttcttgtaataagtttgttatttattttcattggcattattatattatcagtgagtagtggtcataccacagcagcctctatatttatcgtattgagtcttatcctaggtggcggtggtttttttcttatttataaagataattcttaacccacataaaatttgaaaaaatatagagtaagaaaatgtccaattactattattactatggcggggggagatatgattggttaaaaacagtagaacccactaattttttaaaaatcgggttgccttaccaggcacacccattacatcttcaacatcaggcaactactcccccatctatcttagaaaaatttaaacgagcagacattcttcttaatgaggtgaaggccgaaatggacccactcatgttacaaccagaaaccgaaaaaaaactattccagatattgagtagtattgatatgttcaaaggtctgcgaaaaaaagtagaattcacgtacaatgctcaaattgttacgaatgcttggcttaaaatgtatgagctgctaaataccatgaattttaataatacatctcaggcattttgcaattgtgagcttccaggagggtttataagtgcaattaaccattttaattatacaatgatgcattaccctacttttaactgggtagcttcctccctttaccccagttcggaaacagatgccctggaagatcactatggtctttatcagtgcaatccggataactggttgatgcaatctcctttactgaaaaaaaatatagattataataacggggacgtaaccatcgctagcaatgtaaaaaacctagcgcttagagccacacaaaggctgacgcccatccatctatatacggctgatgggggtattaatgtaagacatgactacaataaacaaaaagaattaaatcttaagcttcactttggtcaagcccttacgggtttgttgagtcttagcaaaggcggaaacatgatactcaaacactataccttaaatcatgcatttactctttctttaatatgtgtattttctcacttttttgaggaactatacattaccaaacctacctcctctcggcccacaaactctgaaacctatattgtgggtaaaaacagattacgcttatttacccccaaggaagaacaagtccttctaaaacggctagaattttttaatgatacgcccctcgtagacctaagtctttaccaaaatttacttgaaagcgtttactttgccgtagaaacaatacatctaaaacaacaaatagaatttctaaacttcggaatgaaatgttatcgacatttttataacaagattaaactacttaacgattatttagctccgaaaaaaaagatttttcaggataggtggcgtgtgcttaataagctttatgttcttgaaaaaaagcataaacttaagctttgtgcctcctagggatctgttgcttaatttaacagatgcaatcttaacagatgtaaactaaaaagtgtgttcatacaaggattgtatttatgaatatttattaacatataaggttgtgatgtaacactgtataacctatataactacactatgaagcacggcgtataataatttatattgaacacgatgttgactcatttatttgcaaacaaatatttgtttgcaagacgtttgcatgcatttactaatatgttgttgactagtttatttgcaaactagatgtttgattgcaaactagatgtttgcacgtatttatttgaactaatatacactccttgttttatttgttatatacacagcatacataagtgtatattgtttacacttatgtttataactcgacgtaataacattttacacgctttttttttgcaaatcttaataatattgtatgataaatcaaacaatgtcttatatatgtggtttattattttaggcgccgcaagatgtactccattctcattgcatgcttggtgttattactctgtctagttatatatgtcggtcatcgtgccgatcatgcacgaaaatatttagaaggaatgtggcatggagatccggtttttctaaaacagtcggggctacaatccttttatctctacatacaacctgaccatacatgtttttttagcattgtgaataaaaatggtgaaaagctgatggaaaccaaaataccttgtacgataacaaataaaatatatatgttttttaaacctatttttgaatttcatgttgtgatggaagacatacatagctacttccctaagcagtttaactttctgttagatagtacagaaggtaaacttattttagaaaacaatcacgttatttatgctgtattgtataaggataatttcgccaccgcactaggaaaaacggttgaaaaatatataacacaaaattaatcatgttttctaacaaaaagtacatcggtcttatcaataagaaggagggtttgaaaaaaaaaatagatgattatagtatattaataattggaatattaattggaactaacatcttaagccttattataaatataataggagagattaataaaccaatatgttaccaaaatgatgataagatattttattgccctaaagattgggttggatataataatgtttgttattattttggcaatgaagaaaaaaattataataatgcaagtaattattgtaagcaattaaatagtacgcttactaataataatactattttagtaaatcttactaaaacattaaatcttactaaaacatataatcacgaatctaattattgggttaattattctttaattaaaaatgagtcagtactattacgtgatagtggatattacaaaaaacaaaaacatgtaagtttattatatatttgtagtaaataatatttttaattacttaaaatttttatatataagtttttgatactatattataaaacatatgttcataaaatgataatacttatttttttaatattttctaacatagttttaagtattgattattgggttagttttaataaaacaataattttagatagtaatattactaatgataataatgatataaatggagtatcatggaatttttttaataattcttttaatacactagctacatgtggaaaagcaggtaacttttgtgaatgttctaattatagtacatcaatatataatataacaaataattgtagcttaactatttttcctcataatgatgtatttgatacaacatatcaagtagtatggaatcaaataattaattatacaataaaattattaacacctgctactcccccaaatatcacatataattgtactaattttttaataacatgtaaaaaaaataatggaacaaacactaatatatatttaaatataaatgatacttttgttaaatatactaatgaaagtatacttgaatataactggaataatagtaacattaacaattttacagctacatgtataattaataatacaattagtacatctaatgaaacaacacttataaattgtacttatttaacattgtcatctaactatttttatactttttttaaattatattatattccattaagcatcataattgggataacaataagtattcttcttatatccatcataacttttttatctttacgaaaaagaaaaaaacatgttgaagaaatagaaagtccaccacctgaatctaatgaagaagaacaatgtcagcatgatgacaccacttccatacatgaaccatctcccagagaaccattacttcctaagccttacagtcgttatcagtataatacacctatttactacatgcgtccctcaacacaaccactcaacccatttcccttacctaaaccgtgtcctccacccaaaccatgtccgccacccaaaccatgtcctccacctaaaccatgtccttcagctgaatcctattctccacccaaaccactacctagtatcccgctactacccaatatcccgccattatctacccaaaatatttcgcttattcacgtagatagaattatttaatatgtactatatattaattatttaacctttcaagctggtcttcatttaaatttaaaatccactaataaaatgtattttctagtagcagatcatcgagaacatcatgtgattccttttcttaaaaccgatttccatcacatgcatcaaaatcctatacaaaaaaatcaagctctcctagaaatcaaacagctttttactggagattatctcatctgcaaaagcccttctaccattctggcctgtattgaacgaaaaacctacaaagactttgcggcttctttgaaagatggacgttataaaaatcgccaaaaaatgctgtcgctgcgagaacaaaccaactgtcaactttatttttttgtagaaggcccggcatttcctaaccctcaaaaaaaaattaatcacgttgcctatgcaagcattattactgctatgacgcatcttatggttagagatcatatttttgtcattcaaacgaaaaatgaggcccacagttcccaaaagcttgtgcagcttttttatgccttttctaaggaaatggtgtgcgtcgttcccacctccctcacccccacggatgaagagctatgcatcaagctatggtcttctctttctggtatttcaggcgtgataggtaaaatcttggcaaacacttgttccgtagctcatttggttcatggaaagctttcatcgcagaatattgatcagttaaaaactccctccaaccgaccattccccaaaaaagtaaaacgtatgcttataagcattagcaaaggaaataaggagttagaaataaaattgctctcgggggttcccaatatcgggaaaaaattagctgccgaaattttaaaagatcatgcgcttcttttttttctaaatcagcccgtagaatgcttggcaaatatacaaatcgttcaaaaaacccgtacgattaagttgggaatgaagcgagccgaagcgattcattattttttaaactggtgtggctctgcccatgtaaccgatgatagccaaaatatcacagaggcgtcgcggtccacaatgcaggtcgcgacgcagtccgccgcaatacagcccgctgcaacgcagccattgcacgaagtatcagatgatgcatcatcagatgcttcatcacccgtagggtatcaaacattatctaaagaaatgttattgaacacagcctgatgttaataattcactacatctaaagaaatgttaacctcgatactaaaaagtcattgaacacaactactggggcgctaagttgtccaacacatctaaagaaatgtcaacatcctcgatgctaaaagggtcatcgagccggtcaataatgtcttccccaaaaagtccgggagaactgtaggccgagatgtcgtccatggagctatcttccccagagcacacaaagtcctctccaaaaatcataaagttaaatgcaccgggcttacttaacagcttttcgctttgaataatagtgttgagttctgtcagcgcaaactctctcacaatattcacaacccaggagggctctttaatttcatacagcgttaagaaacttatacataaaaattctatagagtaaagcaaggcgctggcaggatctgttacccgtaggtgtttaaatgtagtgtgatattcattcacaacgttaggcagcaccttttccaaatcctccttttcctcgtacgacaggtgctttacaagcctttcaacatgtataggaggcttgttaaatgtactaacgtgccgcaaacagttataattatataagaaaatacgtacggcagagtcgaccgccatgagccttggatcatccattgaggtaggtggtggcggggcaccctggccttccctgatgtctgcgtaggagcgcccctccatggcccctatggcctctatcacagcaggactgatatccaaaatcttggccgtcttgattatttttccgtaatcgaaagtccatggctcctgtggaggcttgggttgtgtttcggtggagggcgtggtcatatctttctttatttgaatagaacggatcgacatcttttccttatcgtactggtctttataattattataatagtcatgaactaattcgggttgagaaagatgatcgtatataatataggtaaaaagtccgcacttgacacattttttatcctggaagtcgtgtaatcctcccttggggcagcgtgactcgtagaaggcataaaaggtgttaaattctaagctcgcctttagggctgtttggaccttttttatgtttaattgccccacctcatgttgtagcacgtggcatacagaacagcgtagatcggcaagtgcataatggttgtcaattttttttatgacgtctttgcgtgttacttcaatctcggcgggtttctgcgaactgtctacggccttgtaaacgtaaatggtccacttatgaggaagccccctttcatcgtatagggttgaaatgggaagccttttatactcaaacagccgagtccgttggtcggctcttcctgtgttaggatcaaatatgttataaaatccttgctgagcaagcagggccttttgctcgccataagcattttcgtacgttttgaattctgcaagttcggagttaaaattaggtgcattttgtaaatacttaagaaataattcataggctctaaggtaaatgagagttgaggttttttcctcatcccgtcctccccaccacacccgcaggctttcttcttgaaaatagatgtcattcagacgcgtcaactgcgtaaaatcaggccgatatttagaggtataaattttatcataaaattctttttgcgataatagctcggccggggtacgtcctatcacggttttaaactcatattcagcctccttgggagtccgtggtttgtgcatagggatgctgccgtcaatacgggccactgtggcagcataatcatacatggggtccagcagaatctctgtcaaaagtaccttggtgtcgtcctgcacgctaagcccttgtagcccattttggtggataatttttttgaaagcctcccgaaaattattagcaatccactgatccgtaatctcagatagctgatttattataccgctatattgctgcatcattttctccaaaagaaaggtcacgtatgcattcaaagagctatccgccttcattccatgaatggtaatcgtaagaaattctttatttttttgcgagctataaatgagattcaaaatataggcatagatgtagatcacagcatacagctgcgttaaaggatcgtaatcctcttcctttttaatattttcgatgctatacacgagcggcaggcagacatttacggctatattggcaaactgtttcacgtctacaagctttccaaagtggataaacgtgcaggccttcatggtttcctgccaaataaaaacacggagcttactattaagatcgccgatgatgcccacatctgccgtacgatcctcttgaataaaatgggccagctcttcgccacaaattttgcaaaagtaggagtaaataagcccctggttgttttctttctccttgtttattcctgaaaatttcattagcttggttcgcatggtgtcgtaggacgcttctgccgcttgaagctgtataagcatgtccacatggggacaaagcagcttaaacccgcaggctttgcatagattccaattggtggtattgtttttttccttgtagagtacacgaatactttctaatacttttaataactccgcgtattgaagacccgaacgcaactgttttaccagcttgagatgagcacatgcatttttttcttggagttcccactgttttttaatgtttaggtattctgttgtaataagttctgcctcctgtttcccacaggctttaatgacttcttgaaggatgctgttagggtcatccactttaccctccattgtaagaatttcacgtatagcatccgactgcaccctacctattttttcttccataattttaaaatactgtctcgcctgggtaatgacctctgtgagcttcatgtccacctgctgcagaatcatttgctccttttcacgctgttcagcatgttgtaaaaacttttgttctacagggttccaaagcacctccaaatagcctgctctatataggtcataaagcaagggcatgtatcccgatgtaaaaaccggggacaccgagtacatcgtagacaactcttttaaaaaaaatatcacgcgcttaatgttctcctccggttcaatctcctcggtttcaacgatattagatatatgactgccctgatcctcacggtctagctttcggtgtaccatctcctctgctagccgattaatgagccagctatgcccgccgctccgcaaaaacttataaagttcgatatactggtgcgtaaactggatgatgttttccttggtggttacgacaaccccttctccgttttttttccaggtttcttgatccacgcatttcataaatactcgaataaaattggtcaaattggctcctgaggcgacgtagcccaaggtttcaggcgagaaggagcctatctcagccatacgcataaaacactgcggggaaaaagtttttagccgcaacttaagtccatagatttcaatgggggcttctgcgggaacggccaggtgcgtcccattaattaaaaaaatttctttgcgtgtgctagggcgaacacgtaattccttttttttttcactcacgatggggaccacatcggggtctaccagcagttgacgtatgtaggcctctatgggcatggatagatcgggcagctttgactgctcggcgcgaacatggttcacaaaatcttttagagtgaaaagaaagtctattaaacgtatgttttttatatcattagaccctttaagggtagagtagatttcatccactagtgcctcgatttcctcattattgagcgataagatatctgtgccacggtggactatttgcgcgatcgtaattacttcctccattagatagaaactgaatattatatttaaaataaatacaaaatgtcaaatgaaagttttcccgaaacgttggaaaacttactttcaatgttacagaccaaacagcaaaacgcaattcagtcagaggtgattgaatggctgcacagcttttgtgaaacctttcacttaaaaatacactgccataaacagtttattcctagcggggaaaaaaaacgagctaaaatacccgctcaagaaacacagggaaacacgcagccctcccaccatgtgtaccgggttgttctctccagagcacagccagtcaaagcacaggaatctctgctaacaaccatgtgcaacggactggtgctagatgcaaacacatggacatgcctagccattcctccgcctgcgccctttcaacaggcgacccgccaggtccaacacttttaccgtaacaatttctacgaagtggttcccatccaggatggcacccttctcacaatctaccactgggatgaccctgaatatggcccctcctggtgcctagcaagtacccacggatatgatgtgagtaactactgttggataggcgacaaaaccttcgccgagcttgtatacgaattgctgcagcagcactctacctgcgacgtcaccctggaaaaaaataaaacgcggggaacgcgtcttttctttgataacttaaatcccgattactgctatacgattggaatccggcaccataatttacagccgctcatctatgaccctcaaaatatttgggcgattcaatctacaaacctaaaaacgcttaaaacggtatatccagaatactacggctatataggcattccaggaattcagagtcaagttcctgagcttccccagtatgatttaccttatctaatacgatcttataaaactgctatgaatcaagccaaaaatgctataaaaaatggcaaaaaagacaagggatactttaattatggctatttactcatttcgcgagcgcctgccattactaaaagtacttctaatgttttgttaaaatcgcctctgctggtatttttacaaaaaagtgtgtaccagaaaaaacacaatatctctaacagccagcgactagaatttattatactgcaaaactacttgatgcagcattttcgagatcatttcattgctctatttccgcagtacatatcctattatacgaaataccaaaacatgttgaatatgattatccatagtattgcaactaaagataaagatcatccctttgcaggagccgtggtaaaaaaagtgttggaagatattgaaaacgccgaaaacattattgatcatacaaccattcaaaactatgcccatcaaagcaagtacgccatgctttacttgtcaattatttcccatttttaatctaatacggccaaagccgcgggttttttaataaactaacatttaaaaaaactgttttattaaaaattataatacttttattatatatggaacatccatctacaaactatactcccgaacagcaacacgaaaaattaaaacattatgttttaatccctaaacacctttggtcttatattaaatacggaacgcatgtccggtactacaccacacaaaatgttttccgagtcggtggctttgtgcttcaaaatccctacgaagccgttataaaaaatgaggtaaaaacagcaataagactgcaaaatagttttaacacaaaagcgaaagggcatgtaacgtgggccgtcccatatgataatattagcaagctatatgccaaaccagatgcaattatgcttaccatacaagaaaatgttgaaaaagctcttcatgctttaaaccaaaacgtactgacgctcgcatcaaaaatacgttaaatataatttttgtagaggataaaaagctattttagctaaaaaataattcatatacgtttatgcagaggaagaacggtggctttcaaattcagattgcatccacgtagaccgtagcgttttttttgcttctggtttatatcgtaaaccgtaataaacatcatcatttgtatccgttggatctttttcccactccggataaaaaatcggttttctttttttttggtcgttttttgcagtaagctgtaaattaagggaatatagcttatcgaaaagttgttcctgatccatataaatagcagcatatattaaaaaaaaataaaaaaagacgcttcaacgagtcagtaccactgcttgccaacgatttacgttggttggtgcattatggtgatatagtaatgagtgcctgcacaagtgcttgcacaagtgcctgcacaagtgcttgcacaagtgcttgcacaagtgcttacacaagtgcttgcacaagtgcctgtacacattactgcatcgccaaagcacctgcaatgcctacttcctcaacagagtacgataactaaatgcttttaagcaccgcttgcgtcgatgtgtccttcggggcaatcgggttcaattggatccaatattattagtcataattacctaatacttattcaattttatcttttttaccttgtaagatttaaacagcgttttagcttgtttaaagcaacgtttaaaacaagctaaaatgctgtttaaaacaacgttttaaacaagttaaaacaaataagcttataaatataccatgacaaaattagcccaatggatgtttgagcagtatgtcaaagatttaaacctaaaaaatcgagggtccccctcgttccgcaaatggctcacattgcaaccctcactgctgcgctattcgggtgtgatgcgtgctaacgcctttgacatcctaaaatatggctatcctatgcagcagtcaggttatacggttgctacgcttgaaatccactttaaaaatattaggtcttcctttgccaacatttactggaaccgtgatagcgaggagcctgagtacgtctgctgttgtgccacctatcaatcgcacgatggcgaataccggtatcgatttgtttggtaccaacccttcatagaggcttataatgccatagaggcggccctggatcccctggaaaccattatcctgaacctcattgcggcacgagatctagacttcgttgttcacatatttccttataataagggccatgaagactatttggcctccacgcaacttattctcaaaatctttattgcgacgcttttaatggacattttaagaattaaagacaacacgttggacgttcacttaaattccgactatattattgtgatggagcggctttggcctcacataaaggatgccatagaacacttttttgaagcccataaggacttactagggtacttaattgcctttcgcaatggggggaactttgcaggaagtcttagaccctcctgtgggcaaaagattgttcccctaacgattcgagaggtcctacaaatgaatgatattaatttagccgtatggcgggaggtgtttattatgcaggaatgttccgacttagtcatcaatgggatagcgccctgtttccccatttttaacacgtggacgtatttgcaaggtattaaccagattttttttgaaaacacgtctttgcaggagaaatttaaaaaagattttattgcccgagagctttccaaagaaattatcaagggccaaaaaacgttgaatgacaaggagtttaaaaagttaagcctacatcaaatccagtacatggaatcctttctacttatgtcggatgttgccattatgattaccacagagtatgttggctatacccttcaatccctgccgggtattatttcgcgatccagctatttatcccccatcgtgaaaaacattttgatggacgaagactcttttatgtccctactatttgacctatgctatggcgcctacgtgttgcataaaaaagaaaatgtgattcacgcggatttgcacctgaataacatgacctactaccatttcaacccaaccagttttacagatcgcaacaaaccaggaaaatacaccttaaaggtcaagaatcctgtgattgcctttataaccgggcccaaagtcgaaaccgaaacgtacgtgttcaagcacatagatgggttcggctgcatcattgactttagcagagccattatggggccaaaccatgcaatcaagcttgagcggcagtacggcctcgcttttgtaaacaccttttaccgcaatcaaagtgagcatattttaaaggtattacggtactattttcctgaaatgctaaccaatcgcgaaaacgaaatacagggggtgattttatcaaactttaatttctttttcaatagcattactgccattgatttttacgccattgctagaaacctacgtagtatgctttctttggactatttacacacctctgaggtgaaacgaaacgtagaaatttcgcaaacatttttggatacatgtcaatttttggaggaaaaggccgtggaatttttgtttaaaaatcttcatactgtcttatctggcaagccggtcgaaaaaacggccggggatgtgcttttacccatcgtatttaaaaaatttttatacccaaatattcctaaaaatatattacggtcttttaccgtaatagatgtatacaattataataatataaagcgttattctgggaaagctatacaaacgtttccaccctgggctcaaaccaaagaaatcttgacgcacgccgagggtcgtacatttgaagatatttttcctagaggagaattagtttttaaaaaggcttacgcagaaaacaaccatttggacaaaattttacagcgtattcgtgagcagcttgctaatgaaaatttgtaaggcttgcagttcttgtatggtcagaacctatgtcgatggaaacattatttttcgctgcagctgcggcgaaagcgttcaaggggatagtcagaacttgctcgtctctagcaaggtgtaccacaccggggaaatggaagataagtacaagatttttattaaaaatgcaccctttgaccccacgaattgccaaataaaaaaggattgcccaaattgtcatttagactatttgacacaaatctgtattggaagccaaaaaatcattatattggtgtgccgctgtggctatatgagcaacagaggataaaccatatcatcccaccgaattatgacattcctttaaaaccgtccgcctaaatagttttcacacctttggtggcagactattttataaaaagtaatgttggttcatgaagataaagtgtgccaaagaaacttttataaacaaatgattaatgtaggtgctagtcgtgtgtacttaaacagggtattctatagccaagtattttctatagccaagtattttctatagccagtattagtcaagtatttagatgtcagggtatttttatagccagtatttttctatatgtacaaactattccagtaaacatatgtgtgttctttattgagcagcatcatggcattaacaagtttattaaactgctctaatgggcattaaatgacaactcggtgcttagcaaaagtgcctataccttttaacaattagggccgggaggcattcccagcttttttctataatcagccatacagtacccctgagcctcatacacgggaataaggtccttccattccttgttgggatcggcgggccagctctcaaatgaggtgtgaatgtaagggtcctgttctttttccttaatgaagcgtttaatctccatttgatgttgtttacttttttgtttgcggcggagcgtgttccgcaccaatacgtaaaaaataccaagaatcacacataaaagaattattaaaaaaaatatcatcatcgcggggtttaaaaaacgatcccatgcaacaggaatcgttcttaaaaccttgtctggcagggctgtaaacatgaagtctcctcctataatcggggtgggactgtagcctaacagttcaaggtcctgtcgttctagatacttattggcgaactgcccaccctttgcccccgtttttttattaatcaagcagcgctgcattttccaccattctaaatcttcaggagaaagctcaatgccatatatcaactttaacgttattgcatctttttcaatatccttatcaatttggctgagcttttgagctttaagcgggtctagtgtgtacttccatttaaacttagtgtcctgtagtttggctacatgaaatacggaacatttcggcggggcctttgtgacgcccttacactgcggaagtttatcattaggacaggcgcatagatgagactgcgccacagcatcgcgaactacatcgcagacggagtacattttcctcctatgttaaacaataaatttttttcatagctgaaatttgtgggcctatcttttcccttgcccggataataattataagggagtgttgaaacatctgggagagaattgcttaaaaaatgggtttttgggaggggtaactgcgactgttgtacgtcgttggccagggagattctatatgccgggctaaaggtgcaacgttcctgtgaacaacttagtacgcgcgttgttaatacaaatggactggtattagcaaacctcgtaaactcttccggacttgtttgtttttgtatgatgtttagcagggagtctgccttttcgagaatccaaagcgtcgcattgtagtaaaataaaaatagcgacttatcggcaggcgttgcaaaagcgccgtatagaaaataaagcagtaagtactggggagacaccacaataaggttatcttgaatgatagatatcgctagctctttaaacatagtgctaaaaaaatgtatgtcgttcgtcttgaatatagggggactatagtccatgtagggctcacatatctcagtcaggtgaaggcccatttcttttatgacttcttccgggttgtacgtcgctaacaccagcgcgggataggctttgggcatatccacggtaagtgttatgtttttatcattcttatggtaggagtaagatggttgtggaaattctgttttccactccgggactttgcaggtaattctcagctcatttagagtctggtacaggagggcgtatgccgcaaagccgtgtatggccacttgtttaaagggaattgaaaacgttttactttcgtatgtcgacttcacaggaacaacgggaatggggtaatatttttctatgaggttataccgctgcaaatcctttttaaacctgctaaaaacatcttcccttggtgggttatcaaaaggaaagcaaaatgctaggtgtagcccggcccgctggtaatcggggtgaatgattttaaggtttttatacgttaatgtgggtatggtgttaaagatattggggggcatatatgaaagatcagcaacccacacaaagtccgtgcgcacccgcatggtctgcacatggatggcgcgcaccgtgcccacctgcttgaagcccttttcatacaaaatgtcagcaagttcgtaggcgtcctcaacgtggttgggggaaaacatatcaaagtcgggtctttctccctcgggataaattgagctgcctttaagatgcagggcataatcaatggcaatccccccgtacaaaataagctttttctttatgataaattcgcggaccacctccaaagccgcctcaatctccacggcatttgcctcacgtttttgagcaatgagccggtacttagaaacattaaaatcagtctttagtaaagacgtcataaatagtgtttaatatatattaaaggtttgaataaaatactaaatagtaaaaatggatgccctattaaaggaaatagaaaagttatcgcagccatccttgcagaaagaaaacaatgatgtatgcgatctctgttttatgcaaatgaaaaaaatttctaactatcagcttttatgcgaagagtgcggtcagctgaaggactggtttgaacctgaatataatgaaaaattcacggtatattctcgtctaaagatcgtgggtgccaatagttcctatcaccagcgcgatttggacaaggccaactcaagtgactatagctccttgcaatttcatcacattttagaggagctcaaatccctaaatgttaagtatatggatgcggggcaaaagccctttcctattcaggtgttaaaagaaactgctcacagttataaccaagtacaacaacatcgggtcatacgcagcattacaaagcttcagatcttagccagtattctacgtagcatttgtttaaaattaaacattgcttgtacggtggcagacgccgcgaggtttactcaacttaataccaaagggatctcaaggggcatggatcttctgcgctccctatttgtagacaataaaattactttaaacgttgatttaaaccctatagacagctttattaatagtacctacagtgccttacaaattaaacaaatccaccaagaactgcaggaggaaaatgtttataatttaaaagaaattgttaagagctttatattatacgcggatgagaagaacatcggcgtcgatcttaacaggagaaccgttgtgattgctacgatgtataatgttttacgccgtgcctactaccccatagaaattgatacggtggtgtatcaatgtaaaatacgaaaaaatacaattacacgtgctcttaaaatgtatgaggattactactcccactttaagtctctttatgagcagtatcatttaaacgcggcaaaaaaattaatttaaactaaacgtttaaactaaatgtttaaactaaacgttaaaactaaacatttcgactaaagtttaaaacctagtctaacagcgggatgcccatttccctggggttccatatttcaacaattttttgaccttcgggtgttaccttgatgcagcgcatgacgagcagtggaattttcctattaaagagttcttgcttagctatatcaataggactgctatatttttttttaagcattgtagatccattaattgccaattgttgcgctctaacggcgaccaaccttgtggcctcaaaggtggttaaaacgttggaggtaatgcgctcgttatcgggtataatgaccaatgtttgcgacgaggcctgcacaaagccctcgcagatggacggagactccacgatctcgtccttgtcctcggactcctcctcactgtcgacgaggttctcctcttccgtttccacatattcctccacgaggtcatccatgataagatcctcgttgtcattatcagccatattacactgttatcaaatgtactgtttaatacgcaaatggatttactacgttttaattgtatgtcttcatgtgcaggctctagtggaaagtaattttctcacaatttttggcaccgttacacttgtgcccacaaaaacccgcgatttttttattttatattacttttggaagtacgagtttaaccagtcgctttcaaaccttatgcgtctatctcgccaaaaaacgctcacagcggtgttggatattacctttaaaaaaataacattaatttttaccacagagggcgtattgcgtatggattctacgaataagccaggcgtgccactcgatatagacccccagttcattgaccttgatagtattttaatggaactggatcattaggacctctcccgcccatttaaatttttagtttctacaataataaaatgcgcgaggaatcatgggaagaccacgataccattcagctcaccgctcagcgcaaatacctcgccgaggtgcaagctctagagacccttttgactcgagagctttcagtctttctcacagagccaggcagcaaaaaaacaaatattattaatagaatcacaggaaaaacctacgcacttcccagcacagagctactaagactctacgagcatctcgagcaatgtcgcaagcaaggcgccctcatgtattttttggaaagacaggggacctactcgggtctcatgttggactatgaccttaaactcaatacaaatgctgttcccccgctggaaccccccgcgctatcacggctttgccatcgaatatttgtgcatataaaaaacagcagtgtgctgcctgagggcagccataaaatccacttcttttttacattaaaacctgaagtggttcagggcaaatatgggttccatgtgctcattcctggtctcaagctggcggcttctaccaaaaaaagcattataggatccctacagcacgatgccaccgtacaaaaaattctacacgagcagggcgttacaaatcctgagtcctgtctggacccccactccgcctccgttccctcgctcctctacggctcctccaaactaaaccacaagccctaccaactgaaaaccggctttgagttagtctttgatagctctgatcccgactacattcccattcatcaaataaaaaatttagaatcttataatttagtttctgagttgagccttacgaatgaacagggaagccttgtaagacctgtctattgcgcggcagacattgccgctgagaaggaggaagagatcccgaccgaggatcactcgctctccatattaatgctacatgatcccgaagcccggtatttacataaaattttaaatctgcttcctccggagtattatgtagagtaccccctatggagcaacgtcgtattcgctttggccaatacatccgctaactatcggcccctcgccgaatggttttcgcaaaaatgccctgaaaaatggaatacgggaggaaaagagaaactagaaaaactttggaatgatgcctcgcaccacactgaaaagaaaatcaccaagcggtccattatgtactgggcccacaaacatgccccccagcaatacaaagaaattgtagaacaaggctacttttccattctcgctgaatatgtgtatagctataacggcatgcttgagcactacatgatcgccaaagtcatctatgctatgatgggcaacaagtttgtagtggacgtggattcaaacgggaagtacgtttggttcgaatttgtgctaccgggccagccaatgaatcagggagaaatatggaagtggcgcaaggaggtaaacccggatgagctgcacatctatatttccgaaaacttttcaagggtgatggaccgaatcacggagcacatcaaataccacctcagtcaaccccatgaaagcaatattttaaattattataaaaaactattaaaagcctttgaacgctctaaaagtaaaatctttaatgacagctttaaaaagggagttatcaggcaagctgagtttttatttcgccaaagaagctttattcaaactctggataccaatccccacctactgggggttggcaacggggttctctccattgagaccatcccggctaagctcattaatcattttcacgagcatcccattcatcagtacacacacatatgttatgtgccctttaatcccgaaaacccctggacaaaactattattgaatgcactccaagacatcatcccagaacttgatgctaggctgtggatcatgttctacctaagcacggccatatttcgcggcctgaaggaggctctgatgcttttgtggcttggaggcggctgcaatggaaaaacttttctaatgcgacttgtggccatggtattgggcgatcactatgcctccaagctcaacatcagccttcttacaagctgcagagaaaccgcggaaaaacccaacagtgcctttatgcggcttaaggggcggggatatgggtactttgaggaaaccaacaaaagcgaggttctaaatacgtcgcggctgaaggaaatggtaaatccgggcgatgtcaccgctcgagagcttaatcaaaaacaggaaagctttcagatgacggccaccatggtcgccgcgtccaactataacttcatcattgacacgacggaccacggcacatggagaagactgcggcattatcggtcaaaggtgaaattctgccataaccccgaccccagtaacccctacgagaaaaaggaagatcctcgctttattcacgagtacatcatggatccagactgccaaaacgcattcttcagcatactcgtctatttttgggagaagctacagaaggaatacaacgggcagattaaaaaagtgttttgtcccaccattgagagcgaaacggaggcgtacagaaagtcacaagatacgctacataggtttatcacagaaagagtcgtggagtcgccctccgcagaaactgtgtacaacctatccgaggtcgtgacggcctacgcggaatggtacaacaccaacattaacgtaaagcgccatattgccctcgagctatcccaggagttagaaaactctgtgctagaaaaataccttcagtggtctcccaacaaaacgcgaattctaaagggttgccgtattttgcataaatttgaaacgctgcagcccggcgaatcctacattggggtgtccacggccggcacactcctaaacacacccatatgcgagccaaaaaataaatggtgggaatggtcccctaatccctctgcccctcctgagaaagaagcgtctgcaccaactccttagggaatatccttagaagcatgtctttcggcagagccattaccggtagcaaaaaagcaacattgagtatattatatgccttagcctgctcataagcgtccttttttttcatggtattttatgtttttaaatatttttaattattttttaaatacgatgaacagttcgtgctccgaaggctgtttactaaaaatcggtgtgaatccgcattctttaaatatggtttcccattcggggatggtatggaaatccatgtctctacgaatagtatggtgcccaagtgcgtcctgcaggctgtgaagccagaaggcctcctgaccttgatgaaggtcgtacatgataagaaaaccatcaggtttcaacagatggtaaagcttgttaaaatcgtttatcgtaagatgatgcgccgccataggtaaccctatgagctccacagagttttcatgctggacatcgtccatatcggtataaaacgtttcacagtaaatgagacgcttaaacgagtatcgatgacaaacatttatttccaagtaggtttgcactacgtttttaggtatatcgggaatcatgttgattaaggttgtttcgggaaacttaatcatctgactaggcttcattttcaactctttaaaggatttcccggagaagtgaaaatgggtctttacgtatttatgtaaaaatacctgaatgggcagagggggctcctcctcttcgttctcgacgcctcccaaaatatttggaatttcctgacgtggcaaaagaaagtttatgtccacgtttacgaatccatcgaggacggacacaaagcttggctctaatctccattccatatactgtttagaaacgggagatagcataatcctaggcgtcacaatgcacgaagggtttttaatcaccgcatcgtggtaagaaaagtgtattccatttcttccagtataaagaagcctatgttcgtcgtagcagaaacaattaaggcggtatgcctcatacatacactgtttcaaagtacaaacacgttttaaaaaggtttctgcattggcggaggccaagcggttttgccattggtggaaggggttcaatcctacaatggccagctcgtttaaaatatcttcgcggcgcgctaaaatctgcaccatagaagaatactttagcatttttttttcgcaccattcgcgaagatgtttagctacattattaaccttattattgataaagtatacgatggcatgttggaagccttcaaaaataaagagcccctccaaaagatcatctgccaatagaagatggatgttggtgtaagcattgtcaatattttgtagaaacggcggaatgcctgccaaaaccgcttcagcaagcatagctccgttccgttgtttactgtccaatagattcgtaagttttttgtccgcaacagacacgacggctaggatggttgcaatgtcagaaatggcggcttgccagaaataacccgaaaagcacatgcgcgcttcttctatagataaaaacgaaaagcgagaggcaatgtctccgagctgcgtgagttgaagacctttttctcctctggttaaaaggcctgccacaatggcccgctcaatggctgatgccagcgcatccgtggggggaggatccagcatatcaatctcctctgccttaaacacgccttccttattttttttaatcgtttctacgacaatgctaagaaaaatggccccagggccttccgtaatgatttcaggatactgctgcactggtatttgctcaaagacgtgttttgtgtaaagcgggtaaaagtgcccaggaaatactctccctacacgcccctttctttgctcgatacggctttgagccgcggggcgcgtaataagccctcccgcccattcgggatagtaggtttcaatgcttctgttccacccgggatctatgacgtacttcagcgtttcaatggtaaggcccgtttccgcaacaaccgtggaaacaatgacccttcttaaaggtttttccactttagcggttaagggatttttcacccacagattcttaatttccgctttcaggccaaggtaggcctcattttcctgcgcaatcgcctcactatcgatcggcaaaatcaacattaacggcagcttttctttggcaaggtccatatttgcattattcagcaacatcgaaaggaagcgtatttcagccataccgggcatgaaaattaaaatatctgcttccgtgggacgatcatgaatgttttctttatgaatagtgagagccgtttcgcaggcggtcttaatgtagttgttggtgttatacagcggccagtgggtttccacaccgtactgtcgtccttccaccaaaataatgttttcttttccgataccaaaataggttgagtatttatgggtatcaatggtggcggaggttaaaattacaaagggaatacgcagcgcccctatgcttcctctttgcaacatgcgctgaagcatacttttaatatacatgagcataaggtcgatgcctagggctcgctcatgggcctcatctataatcataaaggcatagcgggaagctatctcatcatccgtcattgtatgtagctgcgccaacagaacccccgcggttgcataaataaggccccgattgggtttttccgtcagaggcttcgtttggtagcccactgtttggcctaatatcatgtcggggtagtgggttgaggcgccgatgtctttggcgagggtcaccgcggttaggactcttggctgggtacaaataaccgagcgtcccaagtatttttggaaagaatgcgtgttttcatttctcagaattctgaacacgtgtacgggtaaggccgtggattttccggaaccagtgcgtgactttataatgagcacccggtctgcgagggaggttggaatggcccctccaaactccgggagacgttgttttatccaagtgatgatgtaatgaataggaacatcattcttgtgctcagcgggcacgttatagagatgaccaggctccaataaagtcggttttcccatattctattgttttaaggattgattgttcataaatatttttatactctgaccaagaaattatttttttattaagccggttatttacgttgttatggaacgcgaaggtccagtactgaaagtcctccgagttgtttaatgtcaagggattttttgtaagatacgaaaaggcgtggtgctggcacctggtgcatggcagagactcgataaagttcagtatccattggatggcttcatatttttctttccagctaggagcgtctgaaaaaaagatagcatatagatgcaaggatcgccagtatttaggtccccaatgcaacatttataaccttttgaaaaatctcattccatatagaggtaaatattttttttccatggagaatttttttgcactcttgaagggattgcgccacatcgtcaaatgttttttgttttccatgtattttggcgtaattccagccagtatctgtgtcatggtccttaatgtcatccgctaactgaaaggcatgtccaaaacaatgggcagccctttcaatcatcccaatgtcttcaacggatccagttcctaaaacccagcccataataaacgcgatcttaaaaaagggaatggttttttctggagtgtctactaactgaccggaacccgcgctgtttagagagtggcttacaaaggtacacagcagcgctcccagttggttgggatccggaaaccttggacagtgttccttaatccagtcgatttgccggcaaatattttgaaatccttgcatggttagcgccagagcgctcatctgcgccttggctacgccaaagcgggcccacactgtatctttatttcgccgcttcacatcgttgtcaaaggagggcatatcatcgataatcaaagaagctacgtgaaagtactccgctgctagggcggcctctgccggataaataggcgccccaaaggaatgttgcaactgacaggcccgaacaatttccatcaggataatgggacggatatacttcccacctcttagagcgtaagagcaaggctctgttagttgtcccttaaagtccccatcttcaatagcattatttaagatggtctcaaactcttcactaaaggttttataatttttaggattcagtggatgtattccatgaaaaagcgcgacactacgcggtgctgtgattctaaaatacttaggtttgcgcgtataggatattaaaataataataagaactacaatgatggagatatagatgagatgcaacatgctgagttgtctccccgcagggaatggtccttttccgcgcttgttaacggtaccgaggaggcgttgaaatctttaggaaaggtgctgtctagtttggaatctccaattcctcccgtatatttaggtatataattattgtgtctagaaattgtttgctttgaggtatcaaaatattcagcctgaccgctatttcttttagaataattcggtatagggcttgagtagttggcaatactcttaaaccggggcaccaaggtaacaatattttccatataatgggtttgatacgctttgtttaaaaatgggcttaccggctttatgcttgttagttgtgcattgagtaccggtatgtcttctaggatttgtggctttatagaatgattagcaaacacagaatgtagtatattagatacttgtagcatatgtctatttgcggaaaattcctggtattctctgccgtgttgcgaatctttgggcggaaggggaccaagcatcggcacgtccgtgtaggtactggtggattttatgagttcctgctctatgttcggtttgacatgtggatttcctaaaggaatacctctacctgcaatccctttttctaccgacgcaggtagattgtgcgctaaacacaaaatattgtacacgtctttgtgcggaatatatccgttatagtgctggcccggcatctgatcgccaaggtgctgctcatgcttaatggtaccctttgttctgagtttaggaagatcctcgtacgaaaaaaattttgtgtgctcgctgaacctcgtagaaggaaccgaactattttttgggttttttaaggaaggcaatgaggaaggctgggtcagacaatttttctgtgtgccctttaagctagccacctgcggaaatgtttttttttccgtacgaacaacattgcgcctaattaggttttccgtatgggttgaaaaagcaggacgatgatttttaaaatgattaaaaagtttattttttggaatggagctgtacggctccagatcttgcgcatcgccgtaaccaatgtttttgtgctgagggttcagcataaaagaaaagttacgtagatcactgagttgcaatcccttttcagccttttcaggactattagtgtattcattgtatacaggcgcagctccatttttgttgccgcagtaccgggaatttagtatattatcagaataccggttatgacgcggcaaatcgctttcccaaagaggtggatctgacctataatcggctaacagctttgaagcataatcatgatacattgtatataaaagttaattattatattgagaaggcataattacttcttgtaggggtacaagaggctttgaatcaggcaaactgacgggttttgaatcggccggctttggaccggcaggtatctttttaggttgatcttcttctagctcattagacacggatgggggagaaataggaggaataatttcatctccgcccttatatttgtcatggatagaagaaacaattacatccatgtttgatttattataaatgtcgtttaactggtgatttaaaacataataatgcaaaaataatagggctacaatgcatatatatacgtaaatagccgtcttcgtttttcgttttttatccaccggcggattacaaattgcaaaaaatacaactaataccaccgctgtaatgattaaggccacaatgaaaggattttgaaaggatgttttgaacggttcgcacgtataaattttttctcctaaattattgatacccgcaataaaatctacattcattttatatatttataaattatgaaaaatttagagttacatctccgccggaccaatcattgctaaaatttgaagattcttcaaaaaggcccgactggttgaatgtcttctgctcaggtttccaaaaattttccaagaatggattttgaacaataggctcatcttgattttcttcttcaaggatattttctttgatatcaagaacagcttctttaaactcaggtgtatcttgattaaactcaggtttatcctgatcaatcgcaaaaatattatcttcttcagatatatcctgtttaatcgcaagaatagtttcttcctcaggtttatcctgatcaatcgcaagaatattttcttcttcaggtttatcctgaccaaactcaacaatatctttctcgctaaatccgtttttagtgtgaagctcttggttttgaagagaattatcaaaatctattttagttgttgtcctagaccgtggcacgggatagttatctaatggtttacttactatagtcctcgaatgtggcacgggataattgtttggtgacttgctggttagctcttggcttgttaatagttcttgttttctcaataattccatctctactacttctttttgatccgctggtgtctctttttggtattcttcattagaaaaatgttcagagggtaatgtttcaataaactttgtgagtggatagctgctctttgatgtagaagagcgttgaatttgctgataaaggagttgaacaagtcgccggtattcactctgtcttttttcatattttttacgtagcgtggagagatctgctaagagcgacttgttttcagatgttaattcttcaatttgatgaagaaggctgcgattgtatgaactaagtcttgcatacgtttcttctaattctgtctccggctccacataggcctgttttcgcagaaatttattgtatagttccattctttttttgagcagaaaggtaagactataatcttgcatttctttcgtaactttatggtagttttctttccggtttttgataataaagggcagcattttttctgttgtgataaaggtgcccagattgctaatgtagtcgcacagtagcaattccaagatagattctttcttttcaaggcttatagattggctgtattctttaggtatgaaagaatcaacaatcgttgttacgaagtttgaaaagtttaatgttttgctgttaatttgggtaatgttacaaaaatatttgtaaaaactatctagcattttttcataaagttttttattttgtttaacccctaaaatatagccctttacttgatactgatattccgtaacaatggaatgttttttgtatagtgcatttttgtataaaaagttataaaaaatgttgataaaatacgcaccaagggtttcaaaaatacttataacgtgggattcttcctgatccattatatcatatgtaatattattttaataaaaaattactgacgaataacatgcaaaaaaaatatgtttaaacttattttaagctagcacttatttaaaagtgttttaaacacgttttaaattgtatgttaatacacttaaaaattaagccgaaatttgctccaataaggattacttttatcaatgaccacctctttactataaacggctttacataattttaataatgctttagagccaaagctgaaggcagtgggaagcggcactgtactatggtaaaaatgttgccgatgttcatcctcgcggatgtacacaagtttcctatatcctttaaacacaatatggctaatttcttccacatactccttatcctgtttggaatagcggttgctttgacgggaaaaattcgacatacaaatagaggcatttgtaaaaatggaaacaaatgcgtttttacgaagattggcgggtaaatcggtatcatcttggcagcaaataatcatcgaaataaaacagtgacgattttggtaaaaaaactttttaaaaatttcttttgtaaataatgggtgcagttcggccgcgcagtcgtctaatattaaaagtaaacgaggattaagattgatatagtttaacgtaaacttttcatcctctgtaaggcataagtttttatacatatgaatgttctgtataataattttttttaaaagttgctgataaagcgatgtaatcttttcttcttttttttggtccgtttgttcagcctttaagcactccacttttgcaatatttttgttttccttttgctgtatatcgatcggaagtttatgatacaatgtttttagcatatcgatgttgtttactcgactgtagatggaggacatcatagtttgccgctgccagatggcctccaaaaagcgttcagcgcccttgttgtcattttttttttgcttatcggcgagccacaagcggtagtgtattagagttggatgtacaaaaccctcatatgaacgatttgagggttccgagggggcaaccactaaaatttgttcaatatggggttgcaggattttcataatatgtttaacgtacacggttttgcctgtttttgaggggccatatagcacagttgttttatctataaaatgatgtgctttgaactgtagttcaggaattagcttccctgaatgggtcgttagggccatctctatattattacaattctgcttttgtatataaaatttctttttcgagtttattattattgttgacccacatatctacccgtatcgtatcatcaggcacattgagcatttcaagcgcattatctaactgtttttttgtttttatcagctcgctttcttcatcgggggttaaattttctttactaagcagttgcttaattttttcttcgcagtcgtctataaaatcatactctcgagcttttttgatatttccagatgctttttctaggttttttagctccttaaaggaaagcagtcccttaatcccgctatccgtgtgaaaggttgaattatagatggagagccccggagcatccgggccagtttcttgtatattttttgcttttttgtggtaaatagtatttcgtaaaatctcttttcctatctttaggtcttcctcatgacggtccaaaatccgttttattatttcattattttgattaaaataattgtagcgctctctgttggccttaaagcttcccaggagtgtccagttgcctaattgaatggatgaaacctctgagaaaatctggtctttatatttataataaaattcatcaaccttttgttggttgctgctatccaccacatcataaataatgaaggcaaactctaggtcgggtttttctgggtagatgctttccgtagcggcccgcaactcttcgtaattatcctcaatgtaataattccacttataaaaagtatcctgaggtggaatatgctgcgaaagatatctagtaatttttgtgttaaagagaatgggtttaaacgccctcggattttcaagcatatgtttaatgctttggtgaagttctatattttgtaatatgtgggctgctgccctatagccctgtggggtttgggtgattgcatcaatatcggcctgaagctcattaggcacatttaatgttttttgcatgatgtgtaaagggatgcgctcaggatctgctaaatcggtgtattctgtgcttgtacaagtgcttgcacaggtatctacattggtatctgcacacatgcttgcacaggtgtctacattggtatctgcacacatgcttgcacaagtgtctacattggtatctgcacaagtatacgcactttgagcatgaagattaggatcaaacacaaaatgttctcgtaaaaagctatcgatcgttgttttagcttccttgcttttctgcgtctgggttttgcagctatctgctatagataaaattgtatttactaccgattcagagggaacatcattagtttcctgtttcaaagtatcaactaacgttattagctcactgagaagagttttggtcgtgtgggtaggttttgaataggaaggcatccattcctgcagagctttgaagacatatccaataaagctagtcattataagacgtcgaatatactgctcccgcaaatttgtaaaagagcaaaaggccaccctgctatcatttttgaactgtttgtaagggttcgtcctttggtaaagctgtttaagcgtttcttcggatatttcagtagagggatcctccaatacgtttttgagaagctcatcaatattaaattctgccatatcttagagtttattatatacatattaaagctttaatataaggggggtataacaatggacgaaatcatcaataaataccaagctgttgaaaaactttttaaggaaattcagcaaggattggccgcgtatgatcaatacaagaccttaattagtgaaatgatgcactataataatcatatcaagcaggagtattttaactttttaatgattatttcaccttatcttattagggcgcatagcggagaaacgctgcgaaacaaagtaaataatgaaattaaacgtcttattttggttgaaaatatcaataccaaaatatctaaaacgctggtaagtgttaattttttactacagaaaaaactttcaacggacggggtgaaaacgaaaaacatgtggtgcaccaataatcccatgctgcaggtaaaaacagcccacaacctttttaagcaactatgcgacacacagtccaaaactcaatgggtacaaactttaaaatataaggaatgcaagtattgtcataccgacatggtgtttaacaccacgcagtttgggctgcaatgtcctaactgcggttgtattcaagaattgatgggaaccatttttgatgaaacacatttttacaaccatgatgggcagaaagcaaagtcaggtatctttaaccctaaccgtcactatcggttttggatagaacatattcttggtagaaatccagaacaagagttggggaccaaacaagatccctgcggaaccaaggtgttgcaacaactaaaaaaaattattaagcgcgataataaatgcatcgcgcttttgacggtcgaaaatattcgaaaaatgttaaaagagataaaccgcacagacttaaataattgtgtttctcttatattgcgtaaacttaccggagtagggccgcctcaaatatcagagtcgattttactacgaggcgaatacatatttacagaggcaattaagatacgggaaaaagtgtgtaaaaaagggcgtattaataggaattattatccgtattatatatataaaatttttgacgccattttgcctccaaatgataccacgaatcgacgcattttacaatatattcatttgcaaggaaatgatacgctagctaataatgatagtgagtgggaatctatctgtatggagctccctgaaataaaatggaagcccacagatcgaacccattgtgttcattttttttaaagatgaagattttttagatgattttttttagttttttaaaagacgaaaaaattttttaaaagatgaatattcttaaaccccgcaaattacttttttttaggtactgtaacgcagcacagctgaaccgttctgaagaagaagaaagttaatagcagatgccgataccacaagatcagccgtagtgatagaccccacgtaatccgtgtcccaactaatataaaattctcttgctctggatacgttaatatgaccactgggttggtattcctcccgtggcttcaaagcaaaggtaatcatcatcgcacccggatcatcgggggttttaatcgcattgcctccgtagtggaagggtatgtaagagctgcagaactttgatggaaatttatcgataagattgataccatgagcagttacggaaatgtttttaataataggtaatgtgatcggatacgtaacggggctaatatcagatatagatgaacatgcgtctggaagagctgtatctctatcctgaaagcttatctctgcgtggtgagtgggctgcataatggcgttaacaacatgtccgaacttgtgccaatctcggtgttgatgaggattttgatcggagatgttccaggtaggttttaatcctataaacatatattcaatgggccatttaagagcagacattagtttttcatcgtggtggttattgttggtgtgggtcacctgcgttttatggacacgtatcagcgaaaagcgaacgcgttttacaaaaaggttgtgtatttcaggggttacaaacaggttattgatgtaaagttcattattcgtgagcgagatttcattaatgactcctgggataaaccatggtttaaagcgtatattgcgtctactggggcgtccagctataaaacgtgactggcgtacaaaaagtccaggaaattcattcaccaaatccttttgcgatgcaagctttatggtgataaagcgctcgccgaagggaatggatactgagggaatagcaaggttcacgttctcattaaaccaaaagcgcaacttaatccagagcgcaagagggggctgatagtatttaggggtttgaggtccattacagctgtaatgaacattacgtcttatgtccagatacgttgcgtccgtgataggagtaatatcttgtttacctgctgtttggatattgtgagagttctcgggaaaatgctgtgaaagaaatttcgggttggtatggctacacgttcgctgcgtatcattttcatcggtaagaataggtttgctttggtgcggcttgtgcaaatcatgaatgttgcataggagagggccactggttccctccaccgatacctcctggccaaccaagtgcttatatccagtcattttatcccctgggatgcaaaatttgcgcacaagcgttgtgacatccgaactatattcgtctagggaatttccatttacatcgaatcttacgttttcataaagtcgttctccggggtattcgcagtagtaaaccaagtttcggtacgcattctttgtgccgggtacaatgggtcttccaaaaggatctacaagcgtgtaaacggcgccctctaagggtgtttggttgtcccagtcatatccgttgcgaggaaacgtttgaagctgcccatgggcccccatctgggacgtgccctgaatcggagcatcctgccaggatgaatgacatgcacccaatatatgatggcccaccatatcatggaaaaagtctccgtactggggaataccaaaggtaagcttgtttcccaaggtgggggtacccgtatgcgggcgtactttattgtattcaaaccctactggaacataaggcttaaaatgcgcattaaaatgcaccaaatgtgtttcttcgatttgactcaaagtgggttcgggatcgggtttcccataacttttgttcacatttttaatgttagagatcctgctattcagcaagtcttgggccaatataatcttgtcggccttcccatcgttagcaataagacaaaaagctcctcctgatgccatatataatgttataaaaataatttattgtttttattaaatatggcggtttatgcgaaggatcttgataataacaaagagttaaaccaaaaattaattaacgatcagcttaaaattattgacacgctcttgctggcagaaaaaaaaaactttttggtgtatgaactacctgccccttttgacttttcctccggcgaccctttggccagtcagcgcgacatatactatgccatcataaaaagcctcgaggagcgcgggtttactgtcaaaatatgtatgaaaggggatcgtgccctccttttcatcacctggaaaaaaatacaatccattgagataaacaaaaaagaagaatatctgcgcatgcacttcatacaagacgaagagaaagcattttattgtaaatttttagagtctagatgagcttttacgcaatgttgtacagtgttgtatatatgtcttgtaagcatttgttgtagagtaataagtaaaagataaataaaaatgactattaaaataaagcccaaaccattaaaaatatttttatctgttagatttaatttaataaatggctcatggaatgtgtggtgcgccgctgcatgaggtgtggccgcatgggatgtggtcgcataagatgtagctacatgggatgtggcatttgcttgcatgtaaggatcatgatgtgttgggtcttcatcccagcaataatcgccatctttatctagctgaattgtataccccattatatatcacttattatttttttttaatgtttcatgaatttcattataggcggtgaaagggtcctcaggccccttctgtaaaagattatagagatcttcggacgctttatgtttcgtgcgaattaaggcgggatataacaaaagagagggccccagttccaaacaaattttacttagcgggctcatattttgcaccaagtttcccactacttgcgatgtttcataacgcattttaaagagctttatcataaaagtgttatgcaggccggtgtagtctggcctatagttaaggaaggggatttctctggtaccgtcaaacacgatctcaagtcctctagcaagcccgatcaaaatttcttcagcaatggatgagtatctaattcctacattacgaagcgtaagcatttctataacatcatctatttcctgcatagaggaatctattgtaggaattttaatatcatctgtgctgatttgttcattcccaagataggtaagcagcatattaattttttctagctttactagcttagtcttacgctcataatcatgatcttttttataaaaagagttgggatcaccgttggaccgtagatgattaataaggcggtctacttgctttgtactaggtttaatacttttttcactatactcgctttcagcatagtggtttttacgatctcttttagaaatagctgttttttgagatgcctcagactctgcatatttttttctatgcgtagaaagagaataaccgcggtcattacgtgaactactgttgcatgcaaggcctcggcgcgtcttaccgctgcgcacactgccattgcgtatactgccatcgcgcacactgccgctgcgtatactgccattgcgtatactgccgctgcgtatgctgccgctgcgtatgctgccgctacatacactatcactacatatgctgtcagtacatacgctatcgcggcgtatgccgccgtgtaccttatcgccgcccctacccgagggttttttagatataatactgtgtggggagtcaagcgaaaattcagggtcattaaagttaatgcccaatgactttgccaatccattaagctcttcatcaaaatgatcggtaggaaaactttgttgcttgcccatgacctgtttttcaagttcctccaaattggcttgctcatttatatggagattattcataagcgtcgtaattccagcaagatttgctccttctaaaaatgtggtgtcctccatcggatatactatactatttaaaagcttttaaataaaaatgtgtttggaagaaatgctctcttcaagcgtgtgtagctcagatataaatgcctcctcagaaagctttccaccatactcctttctcatcgtataggagggcgccggtttaatgtaggaaatccactgggaggtaaaaaaccggtacaacatatttagcagctcgcgggcctcccaccttttgggctccgtatagtgcacatcaacataagaggcggcgcatgaaaagctgcaaaagttgccgagaacgcccatctcaatctctcctcgctcattttcacgcatataggtgggcacgaattttgggacagtcttgaaatagagatgacatgtccagcatttaaagctagaatgggtaacccatttggaaacagtggtgaatacggagggtagctttttttcgacctcggcttcatcgtcattcgtatttaacgtatcggtggcagtttttttggattgcaagcattcttcaatggtaatcccggataagtataaaatattaggacaattagtttccataattttgatagttatttttatacaacatggatttaattaaagataaatggaggacgaaacggaactgtgttttcggtcaaacaaggtgacgaggcttgaaatgtttgtctgcacatacgggggaaaaattaccagccttgcatgttcgcatatggagttaattaaaatgttgcaaattgctgagccggtgaaggcattgaactgcaactttggccaccagtgcctaccgggctacgaatctttaataaagactccgaaaaaaactaaaaacatgttgcgccgtccgcgcaaaacagaaggcgatgggacttgcttcaatagtgccattgaagcctccattttgtttaaggacaagatgtataaattaaaatgttttcctagtaccggggaaattcaggtcccgggcgtcatttttccggattttgaagacggaaaaaacattatacagcagtgggtagacttcttgcaacatcaacccattgaaaaaaaaatccagattattgaatttaaaacgattatgattaattttaagtttcaaataaacccagtgtctccccgcgtcatcattcatttaaaaaaatttgcagctttgttggaacacatccctactccatatcccatacgtgaaataaagcctccattagaagactcaaaagtatccgcaaaatttatggtcagtccgggaaaaaaagtacgcattaatgtttttcttaaaggtaagataaatattttaggctgcaacacaaaggaatccgcggagaccatttatacgtttttgaaagatcttatcagcgtacattggcaagaaattttgtgcgtgttaccggtacccgattaaagaatgttttcattaataaggtaatcgactatgctaaaaagaataacaagaaaaataccttgaagaactataccaaagtaggtaggttttctgcatgtcacggcatggttaaaattgctaataatgtagtccacaaaagcattgctcaatacgactaaaaatagtaaaaaaaggataagtgctctttttatatccatatactttaaaacttattttttacactaataatttcctgcggccgcaatataaactgtaggtcatctataacgcccagacctgttaaaagtagagtactatgttttaagggatttaaaatatccgccgcaagaatgtgaatataattttcaaagtggtttacaggaatgcgtaagcgtttttttttgcactgcggttggtttagggtcgaatactggcaggaggtatatatattaataagaccgcggtcgatggtttcaatatcttcatagaattcaatgcgcggcgtcaaaagttttttaagatgttgacataactcatcatacgtgtaggactggaggggggaaagaagggtgtagtcaaagttaaaaatgtttttttgaagaacctttaaagcatgttccgcgtccgtggtttccaaaatatgttttatggtatgaatgtcatttaaatctacaaagtctgacagctttgtgtagaactcggtgacggaggttattttctggaaatcggttttttgaaaaagattttcaatgtgtttgcgggttgagttgctttgcagtccatacaagacatcaaaaaattcaatcagcaaaaacttatacaaatggttaatataaaaagctttgttggccttattctgctgaggatatggttcctctaggggatatagaatggcttggtctatatccctaggatcaatagtcaatgttgcgatgggaagcttttccagcgtagcgggaagagtttgggttggagcgtagtaaaagtatagcccggtttttccctctgaaagaaagcccacaaattctttttttatattttgcagcaccgctgagggtacgatttcgtactgtttatactgtttgttgaaaagggtaataaatttccaggtttcttcaaagcttgcaatctgggtgggccgcagatcaaagtcgatgggaatgtcgtcatgaatgtaggatgatagtcttataggaaaataaatagggcgatcggtgtctgaatcgataagtaaagcataacaaaagttatgcctgttgataagttttttaccaaccgtgtagccgggaatgtttttcacgtcatggatatcccaccagttatccttgcacataaactcgctcatagactggatgacctccatcacagggtcatcttcggtaaaaatatactgggcctcactgtttttcagaaatcttttttgctgggtgatggccattgggtagatcccttcgtccgtgtcaaagataatggctatcttcttcgatgggctaagaattttttgtattgtgctgggggacacctcaaacccgatgtcgccctgtttatctttaaaaaagacacagtgaaggtcgtagcatatggcaacaaggtccagaaagatgtcctgccatgtggtgtcccattgaagcagttggtttttttgttcaacaaaggtttgtaagataaggtttgccagctccgcgccgctggaaaacatgttgccggccccattccccaaaatatagtactgcggtgtgttggccgcctttgcaatttcaatggcaagggccttgggggcaagatccaaaattcgagcaagggaataaaaaagcccggcattgctaattccaagcatggtttgctccacccccacaatgcaaaaaatgtcgggctcttttatcgtatttaaaaacagttcatctgctatctggtggggtagaaaggcaatccggttcaccggtattttttttccataggacaaggtatgacgcgatgtttgtgtattaagatcctccaggtcttgttctacaaacgtgtgcttggtgaggcaggtattgttaatatagaaccgctttgtgcccagcagggccttcgtcttttggcagcacggcagacagtaatttagggggtggcggccttctagtaggcttagatgagggtagtcaggatgcgggcagctatagtaggcaggtaccccctccgtgaaattccaatactttactagctccttgcgcttggctggcggcatggacttcacctcggcctctgagtaaatgacgggtggccgtgggtgctggcataggacggagtaaaccgttgcctgcgtgtcgtacttgcgcaggtcatacaggtcggggtcctgttcttgaagcgcacgtagctgagaggctccctttccttgttgtttatcgtgcagttgagagagtttattaaccaaaattttgtcaggcccggtgatcaagttatctaaaaacacaaataggtaaacccaaagatagttaaactcttcctgggtaatgttaaacatttctattttgatatctgtaaccctatggtagatgcgaatgttgcggccgccgtagattgtttcccaccgggccgcaacatttgtgtcaaagaggtacgcatacgtgttttggagcaacgcaacattgatgtccattttgcgccccggaccggaggaaataatgatcatccgttcgatttcgtggggatcatacgaataaatcccctttttaaataaaaaattgtagaccccggtttgctggaggccccgcacggaaataatccctgcttgctcgtattcccgccaacgacttttgagctcggtaaatcccttgctagaaagcgtatagggccaaaaggtggacaccgacatggagctgatagaaatttggatgtcctcgttggagggaaggggcagactccctccacgaggaaacgcggcaggccccatatcattaattgtatgaataataggatttatgaaattatttagggtggacaccacggagttaaagtcgtggcgctcgttttctgaccaattgctttcgataaagtagtgcccattattttgtatggtaagaataaaggcctttttattgataaagcgtattaaaataatagtgggtacacggaatgttttattgctgaatttttcaggctccgtggaagttatgtggtgtttggaaaccacggtgggacctgttttactataaaagaacaccaccagctgaggaatatcgggagtagctggaaataggtcgaaaacattgcgcacattaatttgaatatttacgaggggtgaaattttaatcattgccgaggtgacggccaacgtgccgcgtgttagtctattcccctcgtacttggcaatgacttgttgtgctctggcatacgtaaagtttattagtttttgctctaggagaagcctctttttaagactggtcaaggatggagaaagagcaggatactgtttttccatttgtaagggagattgtaccaatagtttaaaggcatcgggggaaagaagaggccaatacttcataataaggccgtaatagagtaagtcaaattggtaattatcctctatggcaatggagatttggcgccgcatgggggccactagcgtgttgaggtctgctacaaagatgtgatgaatgttttttatgagctggaagctgtcgagcgcttccacatagagctcatctttttgactttccatagatgcgtcgatgttcaccccacccacctgttgaaactcctttttgtagtcgcgaatgtctaacgccaccccgctaccgcttaacaataggcgatacgttacctgaagcgcattgttttgaaaaaagaaaatgtgttgtctataaggggggatccctgtggcaacgtaaattttttctcgaatgtctttaaaagtgtcttcagggaaaatactatactcgctatacatcgtctcaatttctggcatcatcacgtttgtctcctcgccacgatcctccacaaaaagtttttcaaactcatctaaatcatcgctatctccacccaccacgtattgggaaagctttttctcccaatcctcgccgtaaaaattttgtaaaatttctttgtccttaggggttcgctgcaggtctttgcggcaggcctgtaacacgtttgcaggaacggatcccaaaaaaataaacgtcttcgtgtactcattttccacaggattataaagagtaactcgtagaggatttgttaaaaagtcattttggaaatccattatacccggtatagaaaataaaatttaaaataaaaaacggatgatatctatcatggaccgttctgagattgttgcacgggagaacccggtgattacccaacgagttacaaatctcctacaaaccaatgctcctctactattcatgcccattgatatccatgaagtacgatatggagcctacacacttttcatgtatggttccctcgaaaacggttacaaagcagaagtaaggattgaaaacatcccagttttctttgacgtacagattgagttcaatgatacaaaccagctttttttaaagtcgctactgacggctgaaaatattgtgtatgaacggctggagacgctcacccagcgtcctgtaatggggtaccgcgagaaggaaaaagagtttgcaccatacattcgaatattttttaaaagcctgtatgagcgacgaaaagccattacttacttaaataatatgggctacaacacggccgcggacgacacaacctgttattaccgaatggtttcccgagaattaaaactacctcttacaagttggatacagcttcagcactattcctacgagcctcgcggcttggtacacaggttttccgtaacccccgaggatcttgtttcctatcagaatgatggccccacagaccacagcatcgttatggcctacgatatagagacctatagccctgttaagggaaccgttccggacccaaatcaggcaaacgacgtggtgttcatgatatgcatgcgcattttttggattcactccacagagcctctagcgagcacgtgcatcaccatggcaccctgcaaaaagtcctcagagtggaccaccattctatgctcctctgaaaaaaatttgttgttaagctttgctgaacagtttagccgctgggctcctgatatatgcacagggttcaatgattctcggtacgactggccctttatcgttgaaaaatctatgcagcacggtattctagaagaaatctttaacaaaatgagccttttctggcaccaaaagctggataccattctaaaatgctattacgtaaaggaaaagagagtcaaaatctcggccgaaaaatcgatcatttcctcctttttgcatacccctggatgcctacccattgatgtccgcaacatgtgtatgcagctttaccctaaagccgaaaaaacaagcttgaaagcgtttttagaaaattgtgggttagattcgaaggtagacctgccgtaccatctcatgtggaagtattatgaaacacgagacagcgaaaaaatagccgacgtggcctattactgcattatagatgcccagcgctgtcaggaccttctggtgcgccacaatgttatccccgatcgcagagaggtaggaattctgtcatacacctcgctgtatgactgtatctactacgcgggaggacacaaggtatgcaatatgctcattgcctatgccatccatgatgaatacggccgtattgcttgcagtaccattgcccgaggtaagcgggaacacggaaaatatcccggcgcctttgtgatagaccccgttaaagggcttgaacaggataaacccaccacaggtctcgactttgcgtcgctgtacccctcactcatcatggcctacaacttttcgccagaaaaatttgtagcctctcgggatgaggcaaatagcctcatggccaagggtgaatctcttcactacgtctcctttcactttaacaatcgtctcgtggaaggatggtttgtgcggcataataacgttcctgataaaatgggattgtacccaaaagtactcatcgatctacttaacaaacggaccgcccttaaacaagagcttaaaaaactaggtgagaaaaaagaatgtatccatgaatcccatcctgggtttaaggaactacagtttcgccatgccatggtagacgcgaagcaaaaggcgttgaaaattttcatgaacacgttttacggcgaggcaggtaacaatttgtcgcccttctttctgcttcctctagccggaggagtcaccagttcgggtcaatataatcttaaacttgtctataactttgttatcaataaaggttacggcatcaagtacggtgacaccgactcattatacattacatgcccagatagtctttatacagaggtaacagacgcatatttaaacagccaaaaaacgataaaacattatgagcaactctgccacgaaaaagtgcttctgtctatgaaagccatgtctacactatgcgccgaggtgaatgaatacctgcgacaagataatggcaccagttacctacgtatggcctacgaggaagtactctttcctgtgtgctttacaggcaagaaaaagtattatggtattgctcatgtaaacacacccaattttaatacaaaagaattattcatccgcggaatagatatcattaagcagggtcaaacaaaactcaccaaaacgataggaacgcgaattatggaagaatccatgaaactacgccgccctgaggaccatcgcccccctcttattgaaatcgttaaaacggttttgaaggatgctgtggttaacatgaagcagtggaattttgaagacttcatccaaacagatgcgtggagaccggacaaagacaacaaagcagtccaaatctttatgtctcgcatgcacgctcggcgtgagcaactaaaaaaacacggcgctgcagcatcgcaatttgctgagcccgagccgggagaacgcttctcctacgttatcgtggaaaaacaggtacagtttgatatccagggccaccgcacagattcctccagaaagggggacaagatggaatacgtctctgaagcaaaggctaaaaatcttcctattgatatattgttttatatcaacaactatgttctaggcttgtgcgcgagattcattaatgaaaatgaagaatttcaaccccctgacaacgtcagcaataaggatgaatacgctcagcgccgagctaaatcctacctacaaaaattcgtgcaatccattcaccctaaagacaagtctgtcattaagcaaggcaatgttcatcgacagtgctacaaatacattcaccaagaaattaaaaaaaaaataggcatctttgccgacctttataaggaattttttaacaacaccacaaaccccatcgaaagctttattcaaagcactcagtttatgatacaatactttgatggagaacaaaaagtaaaccattctatgaaaaaaatggttgaacagcatgctacggctagtaatcgagctggtaagcccgctggtaatccagccggcaatgcgctgatgcgggctatatttacgcagctgattacggaagaaaaaaaaattgtacaagccttatacaataagggggatgcaatacacgatcttctcacctatatcattaacaatataaattacaaaattgccacgtttcagacgaaacagatgttgacgttcgagttttccagtactcatgtagaactgctattaaagctgaataaaacgtggcttattttggctggaattcatgtggcaaaaaaacatctgcaagcttttttggattcatataacaatgaatcgccgtctagaacattcattcagcaggctatagaggaagaatgtggcagtattaaaccatcttgctacgactttatttcctaatacttcttaagaaactctttaaacaaggacttcgcatggtcaaaggttctaaacccatggcccttatgattcgccaaaaaagcggtttcatcaagattttctaaccctttcacggatgaagaaataaggtgttcggcctcgtttgcccattttctatgattttttttcacctcgggttctagatctgttttctccatatactcattgtggtcatatttttttttgggaggaggcgtgggtggaggaatgggtggaggaagtacacccgactttcccgcttcaaccgttttataaaaaaatagaagcataatacaaagaataaggactatcgcaaatatgataaccagtgtcccagtcgagggcattttgttatataagtaacgtttttttttattttttataattcgaatgaagaaccatgttgaatagtcttctactcaaagacattttgttatacggtaaatgagaatttataaaatccgaatatcactatcatactgtttatctgagaaggtctcactgggtcctgtgatggagaacccatactctgtaatgctggggtttataatgtggtcaggactgacaagcacatttctgaactgcgagagttctaggtttagacgcagtcgtaatagtcgctgtatatttgtaataaatattagattgcgtatgaggcgagtgtcaaagcgatcctttccaatttgtactaaggtgggcttttgtattccaactcccacttgtttaacgatggaccagggtccttcttcccgattttgttccgtgatataggtcagcacactattttctgtatatgaggtatgatgtcgcatattaatacctggtgccattccaactggcggttgtgcaattcgggctgtaccgggacccaaccatcgtggagttttataaacatatcgttctagcgtatttaaaaattccttaaggttatttacgagtagcatgaagggtgctattaaaacaggtggatggtttataaccattgtcataaaccattgcattgcttcaatatcattttgtaatgcttgacggggaggcggggcaggtaatccacgtatgttgaataaagcggttaattgtgcaccggctgtttggggcgtaatattttgtattaaatttatcatcgaattggcttgcccggcatttcctataagatcgattaaattggttatttgacctcgatattgttgtacccagttttgaatggcagcgatgatctcaggggttggattgttttgaatttcaggtgtttgtattagattattcacttctcttcgtgtatcttcaagctgagtcctaaatgcatttaactcgcctataatttggtttctatcaataacatttcttaaacctcgaactgtttcagccaatcgtatagtacgcacaatttcatgtaaggcctggtttatgtatattgacatgggatggccccaccgctcacgtccacgttgaatacctgcggccaaactaggacctgcctcgtcataatcaaattgtgtaggataaaggcttccaaatagcactttattgaaaatttggtcagaaagaaatttagggcggcccatatttagcgcgttgtcccctctaaagatgcgtgacatgtatccggcgttgcctttggatagtaactcattcccatattgagtaatagagaccgagacataggggtttataagaagttttagcataaattctcgagtatttatggggggacgattcggaatgtttaatacctctgcaacatctggttgaggagccgtggtgtccagagatcgtactttttcagccgaaatgccgtacataagacaagcaatttcttcaaaactatagtcatagttgtaaatattggcaagtggtatagatcgcatcagcgcatttacattgataggtataatattcatatcaaacaagttaaatatgcgctcgcgctctctattagagccaagagtgcgtgtttgacctttcggcgacactattttgtgaatatgattgatttgctcctcttggtaagagctttccacgaaggaaattacgtcttgcaatgttttacgaagcgaatacactgcattcatccctattcccgctgttataatgggtttatcgtctctgttctcgctaataagattaactccaccaaaagtattttcattgtacatcatcactgttttaaaactacggatatttatgataaatcggagagcctgaatggcgtgggtataaaagtgttcaaatcgcgtgggagtaatttgttcgcgagcaactaccgtttcattatagtttttcatgataagctgtactccgggcatatctgagagctgtaccggatcatttcccagtaattttcttgtgccgtatagtagtttaaactcgggggagccgctttcaaggttcgggtaaagaagaggatcatatacctcattattttctattcttaggtcatgtaaataatagagcgaaagtgaaaatggcataagaggctccttattgtaccgggacatatagttttgaatgaagtgttcttctgtttcaagatagatgggatgatcggtaagctcgtgcaggacctccatggcagaatctgccagagtgtgagagcctctaatgatcccgtcgatcactgcgaccagtcgctttcgcacaacatcgctcgtattattttgtgcgtctcctaggggcataagcgtaacattgggacgaaatacgccgccaattccccgcagggccgcctgaccgacggatagtcctgtcgcaggaacattgttattattataataaataacggaatcattattggctcccaagagtgccgtcagattagggcgagctagttggacatttgtgtattgtataaattgttttagaagctctccctggctaataagaatattaaacattttgttaaatagtggaagattggctctataattttctttaaggtaaatgggaatttctgttaaagtagaaataagatgctgactcaggccctggcgattggtatccttaataagccgctgaagtataagtcccaaagacagaagaagcaccgactgctctgtggggtcgcctctatgaccaaagacgttgttattgcgtgctaagtcagggtgagcatatcccatctccatcactgcttggctaaagttcccattagcgaatgcattaataagatttagatatatttttccgctgggagcatcataaaatcgggtaatatatgaagctatgagctggttaaacaccatcatcatactacgattattttgaataccatagtctgatccgtataggcgataacgtcgaaggttgtttgcggcatcattgacattggcataggttctgagcgctatgttgtcccagtagctaagagtattttcctcctgggcgttgttggtacgaataagattggagagtctaaagtctcctagtgccacctgctctacacgaagtccagagttattctccaaagcatcgtaaaatacgagtctactgaatactcttccgtattgttcaaagcgttcagaggattggggattgttatttatttgaatattagccgcgtcccttctttgcgccccacctcgaagttgcagtacattataaggctttgtaagcaaggtgtaggttttattaatgatttggttaaccccctccaggcccaattcaccgccaggaagcggccttcctccggcatcggtaggtggtttaataagtttgtcaattaaatgttcttccaaccagtaaaatgagccaggattagatctattttcatagtattgaataatgtttttatcaatatgcgggcgtagaagatcaagaaaatacttcgtgtcggccatcaaagaatcaattaaggaaataagacctgtaaaatctaaatgcacttgagcggtgctggtttcagggaagcgaacttgaaccattttgttaaaactggaggtcatttcgaagatattggtcaacaggagctgcatgattcgctgattatctactaaataccttgcggccaactcttgctccggacgaactcctccaccagcaggaatacccacatatggtacaatccaagcaaaaagagtttctgtggttaaatttcggtcttgggctgctgcagccgcttcggtagtgggatcagggtacaccatagaaagccgcatattgatttctttaatgactaatcctggatttctaatctcagagatggccccgtgttttcttccgagccagtcaataagattggcgcggttcacgttggcagcttgtgtctctcgtaaccattcgataatgcttttttgaatcgtatctaggtctaaacctttaatgttattacgaaagttattaagaagtacgtaaatagcactcaataagttaagacctgtaataacggtttcatgaaacagaaatattttgttaacatctgtatctgccagtgactcagagccttgaataagttttgaaacgatttgaattttatcggtatgctcctttttgagttcattgatagcctggcgaatgagttcttggtaggaaattttgcccaattcttgttgcagactgggatcttcaaacatctcactaagctgtttcctaaatttttgtaccaaatcccactgggagttgggctgcagcattcctgtttggacatccacagagtctatattgtatagtgccgggcgccacttgggggtaggctgggttgaaggactaataaacctatcggagggaagtaattgtgaggattgtgtatagccatcctcatcaggaagaatggagtagttggtttgattcatcattccaaaatcattcatagttcgcgcttcctgaacaatgcgttgaaatttttcccattcggtgcgtgtaatgacaccgaatctgcggtttatttcatttacaaaatggataagcgcttttttggttgcttcttgttcaccatactctaagttaaagtgttggtaaatgacgtttatttctttgataagctgacgaatttcggtttctgagtagtcaccaatgttaataagctcaataggacgcataaagataatgcgaataagtcctgagaagattccttccagctcaggaagcatcgagatctgtacattttcatctctaaaggaaaacaacttttgataaaattcggcgaggcggggaaggcggaagtaaagctctgctgcctcgggaattacctcgggctctagctcatcggcaccccccaatatcatacgcgtgggtataagtttgtacacgggctcaggccgttcaaacatgtcgtaaatccctaatacaataaaaatcttggcggccatacttttcagcatgaaggtgaagaagacgtcctcggtttcccagcgggttgatagggcgtcgttaactctcacagtagagaggtagacccgctgagccgcttcctcggcagtctgtgcaagcgccatcctttgtcctccaatttctgattgatttagatttttaagtcccacggaaagcgcagaatgttgaagatattcaagcaaggttttatagatttgcaggggcgacatgggcaccatttgccgcagctcctctcccccaagcatgtccccaatccgggcaaaggcattgatgatatttttaagcgcctgaaagttagaaagagagcgcccgataaggtcgcgaatgtttttagcctggcttgctctgacgggacggagggtaccaacgcttcggccttgttggatttcagccgcaactttttcgtagtagtggcccgcaggagcattatccgtaaagacgttggagtcgttgcctgtggaggtgggaaaactttcaaagacttgtgcaagcgtgtcccctgttgtctcggtgaaccatcgtcctataatgcgcacgccatccagcatctgttggactgtttgaatagaatctatgttgtttacaaacgttttggtaatgtttttaagataaagatctagcccttccagagctcgatagaatcggcgttttacatcatactccagctcgatggcgcttacggttgccttccagtctacttcctgggcacctccaggatttgggcccacgtgtcctctggcaagatctacagccggagaattaatgcgcgcatttttttccgtatccaactgcatgaggcgtcccgcaatagcatctccgagaatagtggcatagttttcctcgtaggattgaaactcctgtttgttatgcgttaaattggagtaaatctgggccacataatagtaatacataaaggtgttaattgcctggttgaggtcaacctgcgatcgcgcggccttgctgagcccaagctcttcaactgttagggcagcaccgcctacccttgtacactcgcagtcctcctcgcctccatactttttttgcacaatatcggtataaaaatcaataatctgtagcaagcgagagcaggagtcataaagatttttaaaattagggtcggttttagatatctcctccaaaacatttttaacaagcgtaagctgtgttaagaaggtttcgcgttcttctcgtgcggccgcattggtgtaaaagccgataagacttagatcaagtgcgatggtgcccatatcattaatgcgcgaaagagcatctcgaagcctcgttatgttcggcgtcaaggcaatttctttaacaagtttgatgcctatttttttcacattttccaaaaagtcgttataggcttgtgtgcttttattcaaaaattccatgaggatgtgctttctatccagtctttgcgcttcaatcctcctatctagtggcgttttctcctcatcgcccccctttttggcacaactgttctcaaggattttgtggcgttcattaaaggtctgtcgcaacaggttcacggctttttcaaactcagcaatgttttctgcggagacaagaccactaaaccttttgaggtcaagctccttgtcaaactccgcccagtttttgctttgaaggtactgttcaaccttgagtcctactttctggagagccttattaattttattcgcaacagacgcagcaatacctagattacaaagtgtgtacgaaagtacttttccaaaatttttggttcccaagacactatttgtatcatttaaaagtttaataatatccacctcatccgtctgcagtttatcaagttccttttgggtgggagttaaaatattgtcaataaaattcgttaaaatgttgatttgcaggttttgttcatttaaaagtcgacgatatactgcttcaatcatggtgactgcattaatgacttcctcattgggggctgctttggttacctccgtcaccatgcgctcgtgaagttgcttaatggcgtcgtttaacagcttgatattttcaagtgtattttctatactgccgtgtacatcaagatactctgcgcgcagtccatgagttagggagttaatgtacagaactatttgtcgacatatactggcggccccttcggtggtatctataagcttatcctgacctaaatcaataaattcctggttaatggcgtctgcaatcattttacagacggtctcctgtttttccgcattttttacaaaggtggaaccggctcgaggatcgggcagttgttttttgatatctttaagaatatcttcgatgggctgctttgtgtctactttgaaccctattttggcaatcgccctgataattccttctataatccgcagctttgctttactcgatacggagtctatgtgataatctttaatgtgttgtacaggatttttgtcccccccgccattaaaatatcctccccctgaaaaaggacgagtttgtctttgtatatgatcctgtaacttcgcatatatatttgcttctgatgaaggcagtggtctactagaggttgaagatccacggttacccattataataaaaaaaaataaagatttaaaactacaaatattttgctgtttataaacccaatcatataagactaactaaaacattaaatgtaggtgagataaaagcttattttttttttaaaagtttaataaccatgagtcttaccacctctttttcttcttcctttagaggggttccataaatggtttgaataaaattatgtgctctaataaccttgttaaaatcaggtgcctttccatattgttcaatatgttgcacagtcttttgtgcaagcatatacagcttggagtctttaggtacctccgatgagggctcttgctcaaacaacgtttcaaaggaggatgtgcattcattggtttcattatcatttttttcatgaatgttctccgaagatgctgaggattccgtctcctcttcaaacagcacatgcagaatcatattccattcttcttgagcctgatgttcagtatacccttgccctgcatatatacgagcagatttcacaatatcatacttaacagtactaagcaatgtttttatagcggtcgtaacaattctaccgctattgataatctcaacagaaaaccaattatacaggctacccgcatgaaacacaacttgtgaagatgatcttaaatccgttttgaagatgacctccattttcatggatatatttaaaataaaatccattcaattttaaaattataaaataataagaagatgccctctaatatgaaacagttttgcaagatttctgtatggctacagcagcacgatccagatttattagaaattatcaacaacttatgtatgcttggcaatttatccgcggcaaagtacaaacacggagttaccttcatttaccccaaacaggcaaagatccgcgatgaaataaaaaaacatgcctactccaatgacccttcacaagccataaagaccttagaatcactcatccttccattttacattcccactccagcggagttcaccggggaaatcggctcctacaccggagtgaaattagaggttgaaaaaacggaggcgaataaagttattttaaaaaatggagaagcggtcctagtaccggcggccgattttaagccctttcctgatcgccgactagcggtctggatcatggagtcaggctctatgcccctggagggtcccccctataagcggaaaaaggagggtggggggaatgacccgccggttcctaagcatatctcgccgtatactccgcgcacgcgtattgccattgaggtggaaaaggcctttgatgactgtatgcgtcaaaactggtgtagtgtcaataatccctatcttgccaagtcggtctccttgctgtctttcttgtcgctcaaccatcccaccgagtttattaaggtactgccgcttatagactttgaccccttggtgaccttttatctacttcttgagccctataaaacgcatggggatgactttttaattccggaaaccattttattcggccctaccggatggaatggtacagatctgtatcaaagtgccatgctggagtttaaaaagttttttacccagattactcgccaaacctttatggacatagccgattcggctactaaggaggtagatgttcccatatgttactcggatcccgaaaccgtacattcctatgccaatcacgtgcgtactgaaattttgcatcacaatgccgtcaataaggttacaacacctaacctcgtcgtgcaggcctataatgagctcgagcaaaccaataccatacgacattacggccctattttcccggaaagtaccatcaacgcactgcgtttttggaaaaagctgtggcaggatgaacagcgatttgttatccacggcctgcaccgcacgttgatggatcaacccacctatgaaacctctgagtttgcagagatcgttagaaatttacggttttcgcgtcccggcaataactatataaacgagcttaatattacaagtcccgctatgtacggcgacaagcataccaccggagatattgcgcccaatgatagatttgccatgttggtggcctttatcaacagtactgactttttatacaccgcgattcccgaggaaaaggtaggggggaatgaaacccaaaccagtagccttacagacctagttccaacacggctacactcttttttaaatcataatctaagcaaacttaaaatcttaaaccgcgcgcagcaaacggttagaaatattctttcaaatgattgtcttaatcaactgaaacattatgttaaacacacgggaaaaaatgaaatactaaagttacttcaagaataagtatgttgatacctgtggtgtgttttacctgtgggtttcctattggaacctacgcggcaatttttgacaaggctcgtaccgagtatattaaaaccaaaatgggcggaacattgccgcaaaatatcccattagatgcttctctccagattgagttaaaagacctcattacagctctgggaatcccaatgcgggtgtgttgtcgcactcatttaattactacgttggattatcgtaaatattattaatatctaaaattgaaaaaatatttttaatgttactagtaaaaatgactacacacatctttcacgcagatgatctcctacaagcattgcaacaagcaaaagcagaaaaaaatttttcatctgtattttctttagattgggataaattacgcacagcgaagcgtaatacaacggttaaatatgttacggtcaatgtcatagtaaaaggcaaaaaagctccgctaatgtttaactttcaaaatgaaaaacatgtaggaaccattcctcccagtaccgatgaagaggttatacggatgaatgctgaaaatccaaagtttttggtgaaaaaacgtgacagggatccctgtttgcagttcaacaaatacaaaatctcgccgccattggaagatgatggtctcactgttaaaaagaatgagcagggtgaagaaatataccccggcgacgaagaaaaatctaagttgtttcaaattattgaactgttagaagaagcctttgaagacgctgtgcaaaaaggtcctgaagccatgaaaacgaaacatgttataaaattaattcaaagaaaaatttctaatagcgcggttaaaaacgcagacaaacctttgccgaatcctatcgcacgcattcgtattaaaatcaatcccgctacaagtatactaacaccaatattgcttgataaaaataagcccattactttacagaatggtaaaacaagctttgaagagttaaaagatgaagacggcgttaaggccaatccggataatattcataagcttatagaatcgcattctatacatgatggcatcattaatgctagatctatttgcatcagcaatatgggcatttcatttccgctttgcttggaaatgggagttgtaaaagtttttgaaaaaaataatgggattgatgtgaactccatttatggctcagacgatatttcaactcttgttaatcagattgctattgcttaaacaatttgctcaaaacaagcttataaacgtttcttaggtatgcgatacgtaaatcctaattctttaataagttctttttcagtagtgatttttagaggtactaaagtttgatttttaaataatccatactgatttagcttataattctttttttttaacgcagctcgaattcttattaaataagaaacgggacccgtaaaatgaagtactgcgtatggcttttcctcggctaaggccgtaaaaagatcaagttgatatgtgttttttttccattcaataaaaagtacacactttcgttctccgcagacttttacagaaaaagaaagatcctttatgcgaatgttgggcaggacgtgttttaaaagttttttttctggaacaataataagaagatccacgtcattaagcattttctcttcgcgtcttaagctaccaacagcaacgatgttttttgataaaatttttataagttgtccattatattcaaacgcaagtcgggagcgtaagtcatttacaattttttttccttgaataagcgttaacattttatatttaatattaaaatcttttcattttatatattatatacgcaaaatggcacttgatggttcaagtggtggaggctctaatgtagaaacattacttatagtagcaatcattgtggttattatggcaatcatgctttactatttttggtggatgccccgccagcaaaaaaaatgtagcaaggctgaagaatgcacatgtaataacggaagctgttccctaaaaacaagttaaaacatgcaattatatgcatgcatataaacgcatgcatataaacgcatacatataaaatgcgtaaatactatataaaaaactataacatatcaatcaaggaatcaacacttttataattttccgtaatatatttttcatccataatgatgtcagagtacatggtccctatgcgaggaacagagcccataagggtaggcgcggcaataccgtaaatgggattcacggcggagtcaaccgcagcatctgtcaagacctggactggagacgacaaggccattcgcaacaacacgttggaaggctctcttgcattaagccctgccttttctagagaggtaacctgtcccgttcttgtcatgagatctgcgtacatgagtaaatgacgatggttgggacccttgtcccccataaccgttctaatttcactaataattttttgccgtgccgcttctatgccgtaaagctccatggtgtctcctatagaggacgatacgatggtgtatgggtcgatgttatcatcaagcattgcgccaaaaatattagtcccgtttgttttgatggcgtagatattgtctagtcttaccagtttcccctgggcatccacacggtggcgcataagcttaacaacattcgcatttttgatgcctggtattcctctaatcgtgctatttaatagtttatccaccacatttacggcaattttttcatccgtagccattcgggtattggtactgcgtctaaaggcgctttcccgtaggtatatgcgaataatgatgggaatccctgaggccgtgttttccacagaatgcatgatgtaggtgttggggtgtttagctcttagactattaataatactttctagactaatgctttttaatatcatggttgttttgtttaattccaagcggatacaccagtttgcaatatcctctgggggctgtagtagaggatggttttccagaaaatccgtcatccattccacatcacttgcaaaatcggggtacatcacatttttttttgtgcttgaatacgtttcgtacaataggtgccactgcaatatcaaccgttcgaacgttataagctctatgctgttagcaatttcttgcgcatatgttttatttgtttccacttccgggttctttagacgtaaaagcatttcagaggattgttcagcctctacgggcttcgcgctaaagatctcctggggccgcacaattcccgacttgttggttcccccggccacggaccggtggtgggagtccagcatatattgtgtcaagggctctgatacggactgcgccgccaggattcccactgcctcaccgtagttaataagactttgagtatattgtagccttatgaggtccaggatggcactcatctgctcgcaggtaatgtttaatgttttaacggttgccagttcgatgcgaataagcatgcgcatcagagaggcagcccgtttaagataaacgggtatgggcgtttgtagtcgttcctgaatgttgttaataaacacgtatggaagatttttgcaaaacgttttgaccatcgcgtatttttgtagaatacttttttcgtcgaagggaagcacgccactggtggagctcagtagaatgttttttacgatgctggccacgtttaccggcacctgtctaacatctgtaagcagctgactgaaattaaaattttcgacgtttaggaagatctgtcgatatttatctctatcctttttaaggcgtgaaaattcttcttcaaacaagggcgattgtatcccggtgtacttgaatttgtcttcaagttcctggtccgacagcatgatggtttcaaaccgtacggtttcaagctggcgcgcatcaaggccgtcctctccgtacaactgctgcacaagacgcgtatcgatggaaacccgtcggtaataatccacaatacaggattgaaggccaaagatggctttacggttggcatagcctgtggatgatgtcgataatgctttgttgatcaagtcgaatcttccattcatttccccaaagataaattcaggggaggtaaggcccgcaatatagctgttgcagatgaacccgtaggcctgcgcctccagggcaaacctggggtagtacaccagggtcctaccgaaggaaaactggggttgaatgcgttgtgtattaatttcaatttggccgatgcccgccatgatgtgaatcatattggggtttgagcccttggcgccagtggccaccatctgaaaaagcccattggtttccggattaatggaattcataatcggctttaaaattctatcgggaaatttaagcgcattcagctgcaatttttcgtagaagtcatgcgttgtcaggcctataggcggcatgatgtctccatgaagcagccggttgtttatttcctccgactcaagcagcagttcattgataatttcttggacctcctgatgtgcctccggggttaggagcatgtcggccgtggacactgtgaatccggcgttgcgcacgtagtttagggcgagctgctgggtcgcaaatatcattttcaaggcctgctgcggcccatacctacgcgaaataaggtgatagattccaccggaggaacccgctccgacggcctttttgtcaaggacgccttcaatgagttcgccgttgcgtatttgtgtagagatgtcctgcttgttataatgcatgtagggtgcatacacttctgagtaccatgtgggggctcgttgataattgatgggggtctgcctcagtagcatagatacaaccgatttgccatccagcaggtcagttggggagtagttggcaaaacaaggtgggtcggtttgggttgtttgaaacaaccccatggcgtgcagcttgttcatcacatttttccccatgggggtgttcgtgcgtgtaagcaaaaagcttcccaccgtggagtcctgcacctgcccattaacgggacccgagctctttgtggaaatgaaccagtttcgcacagaacaaagtagttcggcctcaacgcggctcatgacgctccagggaacccagagattcatctgatccccgtcaaagtccgcattataccaggcacatgcgctgacattcatttgaaacgtagaaatttttgggttttcaagaacgacaatccggtgaacccctatgctgcttcgttcgagagaaggctggcgattaaaaaacgcgacgtcgccagtgacgacgtcacggtaaaggatgtctcctacctccagcctaaagtcttgtttgagaccctcaatgtcgtgaacggattgtgttatttgcttatacactcttgaacaaccagggtactggcgctttccatttaaaaaatagggcattaatctattaatattataatgttgcactgtttccgcaacttgcagcgttcgtgcaaaggaaatgggatagccaacctcgtccaggtgaaggtctgagttcccgcagatggtggaccggctgatcgaccatacctggctgcccagtagggatttacgaattcttccctccttgcgaggaagtcttcgcatgatggagggagcagggcgtgcccccatgacgatcccacgctttcccgtgcctccctgggttgcggtggtggaaacggaatccaacaaaaagttatagtaaagttgctgtatggtttgcaaattgcggtcaatatttaaaggtattttttggccgcgcacgatttgtaggtccttcgggatcagcagattctttcgaaccagatactgaatcacgttgttaatgtcgtgaaagctttgggggcctgacccgattcccaatctgatgccaggtcgtatgctgatgggggggatctgaatggccttaagcacaagtttttcgggatgggagtttttacttcgccccagttttacaacggtgtcgtaggttacgcgcgaaaaaatctctctgatgatctgcgggtacagtttgtcaatcttgccctgctgatccgcccaaaaggtaaaataatcttccgagtccttaacaattttggggtgtactgccttacagacgtagcactgctttccttcggtttggcttgaagccgcttcaataagacgcttaggcctaataaggtgctcgtacctctttaggtcaacgatgggagccccgcagttgagacatataacccttaaccatcgtcgtatttcggcgatgaagagcggctgaagcaccggagcatgcatctgcagtatcccagggtgtcccatacattgcttgcgctggtgtgagcaagtgatgcatttataatggtgatcggtggttcccattcgcgcatcatagatacccccttcggcgggaagggtgccctcaaataaattagaaatggtaacctccataacgccttgcctcttatgatcattgtcaccggcaatattgaactgaacggcggctatttcggcatatccagcctccatatttttgctaaatacataataaaacttcaaatgttaaaaaaaaataacatcggttggcatatttttttgttaaaaccaagtgttaaatgatttctaaaacacttatcggttcacgaaaacctaccgcacgggcctgaagaggaatgccagttttgggggaaagctcggcatattccacggtaagctcttttccataaagatgttttttaaataaggcgggcgtgagtttttgaaaaagagcataacgatccgcgtacgtcaaatgcttaggagtgactacaaaccgctttttgtttggcaattcgcaaacccataaaatggcgcctaagtcctttcccttttttccctgagtatagtccactaaaataaattcagcgtctagcagcggtttcagcttggcaagatgcgctgagtggtagttgttgtatcccggctcatagggcccattggcattgcgtacgatggctccctcgtagccctccttaataaactgcgccttaagcctaagggcctcatccacattcttcacgctaaaattttcaacttggtggataaaggtaagatcttccttctgtttaaaaatatttgttaatagctgttgtctcttgttggaaggcatttgaagctgatcactccaaaaacagtcaaacacgtaaaagtgcagctcggaggaatctgtcttcgcattcgcctgccccgcgatccattgcagaggtttgcggtgtaaataaagctcaccatccaaatatactctcacgtctataaataaataaagctgtttgagctcttttttaatattgtcaagacctaaaaattcctttttcgtgcgcgaatacaagagaatgctaccatcgccctgctggcaggccacagctcgaacgccattacgcttgcgctgcacgatgggatctgtttcttcttcaaaaaatgtcttaggaattatattaaaatattttaccagcataggggggataattcctctatttgtgtgggctccccgcttttgtctggcatggcgattatatttactaagggcgtccttgaatgcctgatggactaccgttgtggcattttttttacccaagttttttccctcggtaacacgtgtcatttttgatatccgcaccgccccttcttccacaaaaaattttgtgaaaatttcagcaacggcgtcttttacatctgtggaaaacatctcatctgtgatgggaatgatcgtgttgtgctgcaccacttgcacacaaataatccatgaggccttttttccgcttttcgtttcagactcaatcggaggaaaacaaaaaatgttgtttgaatattgcccaggaaattgatttagcatggttttaacaataaaataagcctatcaatttttttataatttgaatagttattccaaattcaatatggcttctttagataatttagtggcacgatatcagaggtgctttaatgaccagtctcttaaaaatagtactattgaacttgaaatacgttttcaacagataaattttttattattcaaaaccgtatatgaggcacttgtggcacaagagatccctagcaccatctcccacagcatccgctgcatcaaaaaagttcaccatgaaaaccactgccgggaaaaaattttgccgtcggaaaatctttacttcaaaaaacagcctctcatgttttttaagttttcagagcctgcatctctgggctgtaaggtctcgctggccatcgagcagcccattcgtaaatttatcttggactcctccattctcgttcggctcaaaaatcgtacgacctttcgggtatctgaactttggaaaatagagcttaccattgtaaagcagctgatgggaagcgaggtctctgcaaaacttgccgctttcaaaacgcttctgtttgacaccccagagcaacaaacgacaaaaaatatgatgacgttaataaacccagatgacgaatatctttacgaaatagaaatagagtatacaggaaagcccgaatccctaacggcggcagatgttataaaaattaaaaacacggtgttgacacttatttctccaaaccatttaatgctaacagcctaccaccaggccattgaattcattgcctcccatatactgtcctcagaaatccttcttgctcgtattaagagcgggaagtgggggcttaaacgcctcctcccccaggtgaaatccatgaccaaagcggattacatgaaattttatccgcccgttggctactatgtaacggacaaagcagatggaattagaggcatcgccgtcattcaggacacgcaaatttatgtggttgcagaccagttatacagcctaggtaccaccggcattgaaccccttaaaccaaccattttggacggtgaatttatgcctgaaaaaaaagaattttatgggtttgacgtcatcatgtatgagggcaatctattgacgcaacaggggtttgaaacaagaattgagtctttaagcaagggcattaaagtcttacaagcgtttaacataaaagcagaaatgaagccctttatttcgctaacaagtgcagatcccaacgtgctcctcaaaaactttgaaagcatttttaagaaaaaaactcgcccatattctattgatggcatcattttagtagaacctggcaattcttatctaaatacaaacacctttaagtggaagcccacctgggataacacattagactttttggtgcgaaaatgtccggagagtttaaacgtaccagagtacgcgcccaaaaaagggttttccctgcatctactatttgtaggcatctccggagagctttttaaaaaattagcgctaaattggtgtccaggatatacgaaactattccccgttacacagcgcaaccaaaactactttccagtacagttccagccatcggattttccattggcatttctttattaccacccagatacctcgtcattttctaatatagatggaaaggtccttgaaatgcgttgtcttaagagagaaatcaatcacgtcagctgggaaattgtaaaaatccgggaggataggcagcaggatcttaaaaccggcgggtattttggcaatgatttcaaaacagccgaactcacatggcttaactatatggatcccttttcctttgaggagctggcaaagggcccttctggaatgtacttcgccggtgccaaaaccggcatataccgcgctcaaacagcacttatttcctttattaaacaagaaatcatccaaaaaataagtcaccaatcctgggttatcgatcttggaataggaaaagggcaggacctaggacgttacctggacgcagggataaggcatcttgttgggatcgataaggatcaaaccgcgcttgcggagcttgtttatcgaaaattttcgcatgctacgacccgacagcacaagcacgctaccaacatttacgtgttgcatcaagacctcgcagagcctgcgaaagaaatcagcgaaaaggtacaccaaatttacgggtttcccaaggagggagcttcttccattgttagcaacctgtttattcactatcttatgaaaaacacgcagcaggtggaaaacctggccgttctgtgccataagcttcttcagccggggggaatggtgtggtttaccaccatgttgggagaacaggtcttagaattacttcatgaaaatagaatagagctcaatgaagtatgggaggctcgtgaaaacgaagtggtcaaatttgctattaaacgtctctttaaagaggatatattacaggaaactgggcaagaaattggagtcctgttacccttcagcaatggcgacttctacaatgaatatcttgtgaacacagcgtttttaattaaaatatttaaacatcacggcttttccctagttcaaaagcagtcctttaaggactggattccagaatttcaaaactttagtaaaagtttgtataaaattcttacagaagccgataaaacttggacaagcctttttgggtttatttgtctgcgcaaaaattaaatattttttcataagaagtactacccaggttttaaagaaatagctaaaaatatcatatggatactgccatgcagcttaaaacgtctattggtttaattacatgtcgtatgaacacccaaaataaccaaatagaaactattctggttcaaaaacgttacagccttgctttttcagaatttattcattgtcattactctataaatgctaatcaaggtcatctgattaaaatgtttaataacatgacaattaatgaacgactgcttgtcaaaacactggattttgaccgcatgtggtatcatatttggattgaaactccagtctacgaactataccacaaaaaataccaaaaatttaggaaaaattggcttctcccggataatgggaaaaagcttatttcattaatcaaccaagcaaagggctcaggaacacttctatgggaaatccctaagggtaagccgaaggaagacgagtcggaccttacctgtgccatacgggagtttgaagaagaaaccgggattacccgcgaatattaccagattctcccagagtttaaaaaatctatgtcatactttgacggtaaaacagaatataagcatatctacttccttgcaatgttatgtaagtcgttggaggaacccaatatgaatctttctttacaatacgaaaaccgaattgccgaaatttctaaaatttcttggcaaaatatggaggctgtacgttttattagcaaacgccagtcattaaacctggagcctatcatcgggcctgcatttaattttattaaaaactatttacgatacaagcactaggatgccgcattaaaatgccacataaggtaatacactaggaatgtcgcacacgcacaagaatacaacgtcgccggagatttattatctagtacacgttttatgtatgtacaatccgccttcatttaatatattgagcggatgtactatgtatttattttaacaaaaaacattatttttttttaatcttcatcatctgtttttataaactcagtaatatcaaaagtagcttgtggggtttcagagggttcaccttggttatcctccgtgaggataacatgttcttcaggttcgtcgtcactggagaacccatcatttaattcctcttcactcaacatctgtaaaaaatcttccaagctttcgctatcgttaaaatcctcatcatccataagaataatggtaccttcctcatcgtttcctccttgtttcgtgtctaaataggcctgcatggcatttgcaaaagtatcaaaataggctgagtcagattgctgttccaaaatatggccttgcgtattaaatgtggttgcatcgttgttaaatgcttgcaaatacagtaagggatttatatccattattattaagcaaaaaaaatttaaattatttttcgaccgatgttaggtaaaattaaacaattgctataggtgttaagcaatgtttattgattttaagtactcaacaaccatgatgtaaatactatacagcacttttggatttttaatcaaatccagattaatactaacttcttttgtgatacagttcgtaataatagtatcctgctcatcgttttgtaagatttcttttaatatatttttttttaccgggatactaagcaattgattattttcttttaaaaactccttttgatattcaatcgtcttattcattgaatatttgtatataactataattacaaatgttcaatgaattgttattcatgtcgggagatggctatttaaaaatcatgtcctatttttctttgctcaataagcatccaaatattttcatggcgttttattaattgttcattattgaacgtatcacaaagatcatttataaattgcagatagtttattatttctttcaagagagtaacaaacattacttcagcagaacatataataggtaattcagtggcgttaaaagaattttgatcttgttgatacgccaatggcgaggacttaaggagatttgggggtcttgcccaaaaccctaggctgctgttcttgttttttagggcgtcataaagaaatgaaagcacattgcaaggcttaagccgcgacatctccttccccttgggccctttccatatttttagatctaagatctcatccgagcttatagagtaggtatagtaaagtttttcaaaaaagcatatctgcttgaagtcttttttagaacgactttcaagaagcatttctataatgttaacaagttttgttaggtttaaggcctgttcctgtgtaagctcctcttgcacgtgatagactgaaaaagtgtgcttaggaatgaaaatactccccgtggcactggcctgttgtctgccaggtatatagtacacgctgctgttagcaagctgtaccggcacaatttgccccacttctgcaacattattttgcgattcggacgagggtatgacaatagttacgggttcagtcaataggctttcgccgagaataatattactgtcatttttaataattttaacggccgctattaaatcaaaggcatttaagtaagaaacaacagcagaaaatcttacatgcatatatcctcttccgctattattcgtacgcataataaaacaaggggagcgttgtataacgccagtaatattaagaataaaactgtttttgaaacacttacccacataaatgttttcaagctccttcaaaagatgagcctccacatttgtacaaaaattggtaggatcatcaatattcaacgttgtctcaaaaattttttggtcgatcatatctataatatattctgtctatttcaatttaaataatatacgaataaataacgagattattttattaaataagcaatggtgtatacactttgtatttactttgagatatactttgtgtatcacaacgtgccctaagatgtgtgcacaagtgacggcattttgtcgttaaaaaggtaaaaccagcggattccatcctgcattccatttggttgattacgagcctccatttctttttgcaaaaggttattgcgaatgagtaagcagagcttgatggcactaatctttgtaaggtttaaacttatgcccaattggtcagcaattttttgttgctcctcccgtccgcgtgtttcgcatacggctccccggtttagcatgcgaatatcagtaatctcattcttttttaaaacctggataggtgggcggattttaaatttaagggcctttcccttgctttccatatagcctatgacgatgtcgttttcttttcgtttaacattaatattaagcatataaagcggaatttcatgccaggttttatcttctcgcgaggtaataagtcgcacggagtcctccgtggcatagcccactagagtgttgtcatccccaggcacgtggcttataattttaaaaatgtccggaaatggctgaatatctttttttgaaaaagcgatgaaaaactttttataaacctcgacaagggcccccatacctgcaagattatctataataagtgcttctagcatcgtatagtgaaatgaagcggggtagtggatgagtacctgctccattggctcatcctgaaaatccttctgaaacttttcatacaatacttgaaagggttctttggtctgcgagtgttcgaggtatttggtaatacggatgctgtgcatcgcgggaggctgaaaatcccgaatatatgtttcaatatctaataccggttcctttttatggttaagcaccgcagcgacgtacaaatgctcaggctttgccggcacatgcataatggtgcaaagacgattctgtatccataattccttgcactggttttttgagtagcatagagaaatgagcgccagcgcgaagttgtcctctgagaagagtttattatcgatggtaattccctgtatgagcttgggagtggaaacagccttccatagctcggagtacgtccacacggggcgtgccataaacaaagatataataatattagaaattgtttttacctcttgctccccgtatccataggcctcaaaggtattgaggacggtggctccgacgtttgccggcgtgatggatggactaaggggcagactttccaacataggcttatcaatcttaatctggttggtgaacccatcaatggcgtgctttcgcagcgccttatccccctcctgtattaaaatgtattcttttaatttttgtgcgtacttagcgagctctggccctccatcgggtgttgtcgatacgtacaaataaattgtcacgttgcgctcactgggggggagctccatgtgtgaattttttcgcaccaccctcccaaatacctgaataagccggggaatatcaaggggcaatgacataatcatctcgtaccgcacggcctgaaagttcaaaccctccacaatcaccttggacccgatgagaatacgcagctggtggccttccaggttggacgaggcgttaaaaagagccaggcttcgttcgcgtacagcgggctctatttcgctgtgcagaatggtgaaccgtactggaataaactgatggtcgctatgtgtgtgctcatcgcgaatcgcggcgcagatggagcagcgggtcgttcccacaggggacgaaacttcatttaaaatgccattactttgtaaaatttcttgcaagataagaacccccgacatgcggacccgattgtggtaaattaaaattttcccccggccttgccgaataatggaaagaatgtctttcatcatttgagtgtattttccgctataaaaggccaatcccgagatgtgcgttggtggctgcagcgacaaaaagctgccactcacattaaagggggctctacgcgaaggctcaataatctgtaccccgttttccagaagccagtctgtgcttgccatagaaagggcggtgggggtttccgtcgagttaaacaggccgtaagccttgggttccgtttgttttgaaaattttgggttgggaaacaccatgtcataaatgctgtacgcattactcgagattttagggtcagggcccagctgtttaagcgtttcaagctgatactcagacatggggcattcgatgaaatgtaagtacggcaatgtttcgtctttataggacaacatctttccggcaaatattctttcggggtaaaaattggtgttggtatccaacaaaaaagatacccttccggtgctcagtctttccacaagagctagggcgtcctttttccatttaacggaatgcccactgctgtcaaacagttgctggcgctggaggggctggccgttgggcagctcatgccgcggaaccaaaaggtttaacaggtcgacgtattccatgacactcccggttacgggcgttgccgacatgaagacggccctgggggcctggtgaggtggaaaggcatccaggacatactgtaaagcgatgccataattatttcgttcctggatattgtacacgttgtgtatttcatccgcaatgagcagtcctcccctaagttgctccatgattttttgattcacccggatgaggccgtttgtctcggcctcgctaattttttgcacgaactgagatatatcgttctcattcaatgtatcttctgcttcgtcagaacgatgaaacagagaaagcacatcaaagtttttctcttcacccttactcgtaatattgaaaagcttggatgcaaattccttatagccgtaaaactgaaaaaagcctccgcggtttctatcggttaaacggcgctttaacgtactaacgaacccatttagatgccgtgattcgaccgacgtggtgctgccagactgctttgcaatgtgaagaagccggtgtagctcagcgacctccttgtaagaaacaaatcccagctcaggacgtcttagcatttctgtttgaatgatggcgcgtgtaaagcctaccacaaaaatccagggcgcattttcaataaaattcatgtagtggttcataaattgacgcgcgatggcaatcgcggcaatgctttttcccgtcccggtctgccagtttaataaaagacgcgagtagggcgtgttgggattttgaaagttttggacgaaaagctgggcattatgcaattggagacccttgatggaaggaaagggcgacgcgtaggggtcacacggaaaaaacgctcgcccccccttctcgcagccaggcccaccgatctggacaaaatgagcccgcagatcacgaatgagctctttttggtcgacaggaggggaaatcaacgatttaaactcctttcttcgcgccaactgctgcaaaaagtctgcggcatccaattcgggatacgccatattatcataaaaaaaataaacctttttatgaaaacttttatgtgattctgtattgcaattgttttttatgaatactgtaaataagcgtatcaacttgtttttctaacgaagaggcgttattctttttttctggatataaaataataataagtataataattaagactaaacagcaggcaatcactatcaaactcatattatacttacttttttataaaaagtattatatcttatgaatgcgcaagttcagctaattgttcgtcgcttggaatgtgggactgcagggaggtggagtttttcctttttctaaagaataccgggaaatggtggtgaggctcaggttgttgtacatagtagctaggaggaggtttaggtatgctcgacttgcagtcaatagtccggttatagtaaacgatggcaacgatgataagaataataatgagcaaaatcaaaatgcccaggagaatcgcagttgttccgggatatttggcgattgtatgggctaaaaggccttgggtgctttgtttaattccctcgcgggttgacaggttatgagaaagcagtggagacgtttcagtgtccatttattacaattgaacagttatattaatctcaaataaaatataacacaaaattaattatggccatgcaaaagttatttacgtatatttacgagtttattgaatatcgtaagatggtgctgttggaagaaaaggtaccatatgataagtttgttcaaatggtacttaatacaggattttttcgtattaacgcggagacgctgaatcacggaatcgtatccgtgtttatctttggagcaaatggcaagtacgttcaccacggaggcgacatgagaacgcttttaacgaatacgcttaatgaaaaaaaacattatgaagaattaattttaatcgttgataagcccgttttaagcaaaaaaaatattttagatataatcgtcgagcagcgcgctgcaaatcccacgattgtaataaacatatatccctaccacctgttctgcattaacattcccaaggtgagtgccattcctaaacataaactaattactcaggaggaggcgcaggagtttttaggtcgcgaatatctgcaaccgcaggacctcatgcaaattagcgcgtcagaccccccggtggtctggctgggaggaagaccgggagactttgtgcaaattgagcggccctcagagacagctatgcacgctgttgttatccgctttatcaccaagtccaaaatttgagtcccgtgtttaaagatgacagacagctaagtaagcatatctgtaaaattgtcgatgtcctctgtggatagagcgctttcctctgagcagcaaattttttcatacatctccatgggggatggcgaggctttaatagtatgtaggtcacgtaagaactgttgtatgatgggatatttgtcttttaaaaactggggatgtttcataactggaattatttgaaagataaagaccttccatccaaagtagccaaccacatttggcatttcgggacacgcggtttcataaggcatagaatagtgaatagtgtactgatctttttgatacagcgtttcaagtagttggcgaaatgtttccgcgtcgagcgtgccaaaatcttgaggagcctcggtgtgctcctgtgtagagcagatcgtgatgattccccaggcaagcgggagcatggactctggagggtggatatccgtattggtctcattattcgatcccagctgatgaatgccgcacacgcgaaacatggcctcgacgtagatgcccatagagataggcggcgaaagggcaagaccggattgtatttgcggcatatagtaggagggcaccgagttttttatttttcggttgaatggggactttatttctaccagcacggggatgcgtttcgtggcctcatagcgtacgttgttaaaaattgttttgatttcccaggactgttgagtgtatcccagcgttaggtgacaaaacccatcggggctattactatgtccggggtatcccaaataggtcccatcaatatgaatattgtcacctatgacggtggtttggcagaacaactcaagcagatctttactaacacgctcaaaaagggttccccagctacaagcagcgcggttcaaattcttcttaaaaagatttgctttttccgccaaggttatataatagcttttgtaagggtttaaacctaaaacgctggcaaggtcagagccacccacctgagtgcgacgaatagcatgccaggcatcggagcgctgctgaggagagtctttaaacaggcgtacaaaggtttccattatacttgttttaacaggaattcaatataaaaagtcaacacagtttgcaatttttccaatctcaagatatagccatacatttttttttccaattggcgaatatgtttaagctcatgtgtttcaatattagcatccggaaatttaaatgcataaagatgttcaaaggcctgatttatacacgtatcaaaggatctgtggtatgttattagcttcagcatgtgtgccagatcttcaagatggtctaaatttatacggttttccacgtggtggatcatgtctgccacatcttgagcccccatccaggggatcacaaggtactcccccttaaagatgattcgtcgtttttttaaaaaatcatgaaaacgttttaaagcttcaagaaaggggcagttgggctttgaccccaaaatgctgacgacgatatcctcgggcatgatgtattcgcagtgaggatagtagtttacggactctaattcagcggcccgccgttttatttcgtatcttgcccagttattcagagagtactccacgcctccgaccacaacagacatcctatctattaaaaaataacaataaaaaccttatgaaatctatgtatagtggccgctaaaatgtctatattagaaaaaattacgtcaagtccctctgaatgcgcagagcatcttacaaacaaagatagctgtttaagtaaaaaaatacaaaaagagctcacctcttttttggaaaaaaaagagacactcggttgcgattcggagtcctgcgtaattacccaccccgccgtgaaggcctatgcgcaacaaaagggactggacctctccaaagaactggagactcggtttaaagcgccaggacccagaaacaacacgggtcttcttacaaacttcaatattgatgaaacgctgcagaggtgggccataaaatacaccaagtttttcaactgtcctttttccatgatggactttgagagggtccattataaatttaatcaagtggatatggtaaaggtatataagggagaagagctacaatatgtagaaggcaaagtggtcaagcgtccttgtaacaccttcggatgcgttttaaacacggacttttcaacgggcactggaaaacactgggtagccatctttgtggatatgcggggcgactgctggagcatcgaatattttaattcgacgggaaattctcctccaggtcccgttattcgttggatggaacgggtcaaacagcagctattaaaaatacaccacaccgtgaaaacgcttgcagttaccaacattcgtcaccaacggtcgcagaccgagtgcggcccctacagcctgttttacatcagggcacgcctcgacaacgtgtcatacgcccattttatatccgctaggattaccgacgaagacatgtataagtttagaacccatctgtttcgcatcgcataaactaataaagtttgaattctttataggaataaaaatggaagcgtttgaaatcagcgatttcaaagagcatgcgaagaaaaaaagcatgtgggctggcgccctcaacaaagtcactatttcgggtcttatgggggtctttaccgaagatgaggaccttatggcgttacccattcacagagaccactgccccgctttgttaaaaatttttgacgagatcatcgtaaatgccacggatcatgaaagagcttgccataacaaaacaaaaaaggtaacttacattaaaatttcgtttgataaaggtgtgttttcttgcgaaaacgatggcccgggaatccccattgcaaagcatgagcaagccagtcttatcgccaagcgcgatgtgtatgttcccgaggtggcttcatgtcactttttagccggaacgaacatcaataaggccaaggactgtatcaaggggggaaccaacggcgtcgggctgaagctcgccatggtgcattcgcagtgggccattcttaccaccgccgacggcgcgcaaaagtatgttcaacatatcaaccaacgcctagatatcattgagcctcctaccattacaccctccagggaaatgtttacacgtatcgagctcatgcccgtataccaggaactagggtacgcggagcctctgtctgaaacagagcaggcggatctttccgcctggatttaccttcgcgcctgccaatgcgcggcctacgtgggaaaaggcaccaccatttattacaatgataagccttgccgcacgggctctgtgatggcgctagccaaaatgtacaccctgttgagcgcgcctaatagcacgatacatacggcgaccattaaggccgacgcaaagccctatagcctgcaccccctgcaggttgcggcggtcgtgtcccccaagtttaaaaaatttgaacacgtgtccgttatcaacggggtaaattgcgtaaaaggagaacatgtcacctttttgaaaaagactattaatgaaatggtcgttaaaaaatttcaacaaacgattaaagataaaaaccgcaaaacaacattacgagacagctgttcaaacatctttatcgttatagtgggttccattccaggaatagaatggaccggccagcggaaggatgaacttagcatcgcggaaaatgtttttaaaacgcattactccattccttctagttttttaacaagtatgacaaagtctatcgtggatattcttctgcaatccatttctaaaaaagataaccataaacaggtcgacgtagacaaatatacgcgtgcccgcaatgcgggaggaaaaagggcgcaggactgcatgctactcgcggcggaaggggatagcgcactttccctgctgcgcacgggactaaccctgggaaagtccaacccaagcgggccctcctttgacttctgcggcatgatctccctgggaggagtcatcatgaatgcctgcaaaaaggtgacaaacattacaacggactctggagaaaccattatggtgcgcaacgaacagcttaccaataataaagtgttgcagggaatcgtgcaggtattgggtctagacttcaactgccattacaaaacacaggaagagcgagcaaagctgagatacggctgcattgttgcgtgcgttgatcaagatctggatgggtgtggaaaaatccttggactgctgctggcctactttcacctgttttggcctcagcttattatccatggtttcgtaaaacgactgcttaccccgctgatacgtgtgtatgaaaagggtaagaccatgcccgtggaattttactatgaacaagagtttgatgcctgggcaaaaaagcagaccagcttagccaaccataccgtaaaatattacaagggattggcggcgcatgacacccatgaagtaaaaagcatgttcaaacattttgacaacatggtgtacacgtttaccctggatgactcagcaaaggagttgtttcatatttattttggcggggagtcggagttgcgaaaaagagagctttgcaccggcgtggtgccgctcaccgaaacccagacgcagtccattcatagtgtccgacgaattccttgcagcctgcatctgcaagtagataccaaggcttacaagctggatgccatcgagcggcagattcccaacttcttagacgggatgacgcgggcgcggcgcaaaattttagccgggggggtgaaatgcttcgcctccaacaaccgtgaacgaaaggtttttcagttcgggggctacgttgcagatcacatgttttatcaccatggcgacatgtcgttaaacacaagtattataaaagccgcccagtattacccaggctcctcccacctctatccggtattcataggcataggaagttttggctccaggcacctgggaggaaaggatgcaggatccccaagatacatcagtgtgcagcttgcgtctgaatttattaaaacaatgttccccgcggaggactcatggcttctcccctacgtctttgaggacggccagcgggcggaaccagagtactacgtgcctgtgttgccgcttgctattatggagtacggcgccaacccatcggagggctggaagtacaccacttgggcccggcaactggaagacattttggccttggtgagggcctacgtcgacaaagacaacccaaaacacgagctactgcactatgcaataaaacataagattactatactcccgctgcggccctccaattacaatttcaagggccatttgaagcggtttggccaatactactacagctacggcacgtacgtcatctcagagcagcgaaatataattactattacggagcttcctctgcgtgttcctacggttgcatacatcgaaagtataaaaaaatcgagtaaccgcatgacatttattgaagaaatcatcgactacagtagttcagaaactattgaaattctggtgaaattaaagccaaatagtcttaaccgtatcgtggaagaatttaaggagactgaagagcaagattccatagaaaattttctgcgcctgcgcaattgtttacattcacatctaaactttgtaaaacctaaaggtggcattatcgagtttaacacgtattatgaaattttgtatgcgtggctaccttacaggcgtgagctttaccaaaagcgtcttatgcgtgagcacgcggtgcttaagctgcgcattatcatggaaactgctattgtacgctacatcaatgagtctgcagagctaaatctttcccattatgaggatgaaaaggaggcaagccgcattctaagcgagcatggatttcccccgctgaaccacacgctgatcatttcccctgagtttgcctctatagaggaactcaatcaaaaagcactgcagggctgttatacctatatactatctttgcaggctcgagaattgcttatcgcagccaaaactcgtcgggtggaaaaaataaaaaaaatgcaagctcgtcttgataaggttgagcagcttttgcaagagtctccctttcccggcgccagcgtatggctggaggaaattgatgcggtggaaaaggctattataaaaggaagaaatactcagtggaaatttcattaaacgctaccggttttatgatgtccaataggtgttaagcaatcagttcatcaacatttttttcaagaatttgaaaagtttggataatgttctgaatacttttttctaaaagagttatcaaatcttcttgtgaggccttatgaataattgttaataccatttcttgcttatggggaacacactgataccccacaaagctaatatcaggaatcatttcataaatatatgtttttagcagatttccgatggtatgggtttcatcttttatcgtgataatggcctttgttttttcctcatccatggaaaacagcacaagttccggctgcggctcttcaaagttttcataaattttttgaatgctttggattcggccaataatgatccggcaggcgttttttaaatacgtgcgaacggcctggttgatatgtggcagcggcaccgctggaaagcaaagccccaggcggtggtgacgcgggtctgaggtcatagagctttgcttgtaaccgctaagcgccatatattcttttttatccgttgggtactgttcaatgtcaaggtgggaaaaatgtgttttaacggcaagattaaaggcggcatgctttcgtcctatgccctttttaatatagatatcctctataatcaacgattttccgggttgtaggaagccaatctcaaaggtaggattaaaaatcgggtatttaagcttagggcctgccacctggatgagatcgcggctatagatggttttaacctcacagctattgtttaaactccgcagagcaaataccagtgtctcgtttttcgcataaatcggaatgaaattaatgcggtttctaataaattgttccgtcataaacaggtccgtggaatcctcgatcttatacccaccgggcttaatatctagcatataattgggaatttcatcttgcaagacccgcgacaggccgtggaccgcggctctgctaatgcccttaaagtccataacaacattgaccgggacgaggggcaactgctcctcgagctgaaatagttttttggccgcatttttaataaagaggttggaaaagtctatcaaaaacggtttgatttccacgttttggaaaattttttccatttgtattataaatatatctatatatattcaaattatggtagtttatgacttgctcgtttctttaagtaaggaatccatagatgtgctacggtttgtagaggcaaaccttgcggcgtttaaccagcagtatatttttttcaatatccaaagaaaaaactcgatcacgacaccccttctcattacgccgcagcaggaaaaaatttcgcaaattgttgagtttttaatggatgaatataataagaacaatagaaggccctccgggccgccgcgtgagcagcccatgcacccattattgccgtatcaacaatcctcggacgaacagcccatgatgccgtatcaacagcccccggggaatgatgatcagccatatgagcaaatataccataaaaaacacgcgtcgcagcaagtaaatactgaactgaacgattattatcaacatattcttgcattaggcgatgaagacaaaggtatggacagcatgttaaaacttccagaaaaggcaaaaagggatagcgatgatgaggacgacatgttttctataaaaaactaacgacgtaacaattaaacaaaaaataaaaatcattataaaatgaatcttgaatacgtccaagttgttcaaaaatttaatcaagtactcctagaacttaccaaaaaagtatgtaccgttgtgggcgggagcaaacccacctattggtatcaccacattagaagggtttgctcagaatgtccatccatgccgatgagtatgataggtccgtatctgaatgtctataaagcccaaattctaacaagggacaagaatttttttatgaatttcgatcccgcgcataatgagtacacctttatcattcaaaaactaaaagaagcagcccgaaatatgccggaagacgaattagaacagtactgggtaaaacttttatttttacttaaaagctacataaaatgtaagccctttattaattaaagaattgatgcataactaataaatggccggtcgtgttaaaataaaacagaaagagctcatagactctactgtaaaaaacaaaaatgtgatgaatctgttccatgaaattataggctcaaaaggcaatattaattttagcgttgtctggcccaagtttaaaaaaatcaaacagagcgtttatgactacatttccactctttctgtgctggaaaaagcaaacgttatgcaaaactttgaagctgataagaaactgttggaactttttgtacaaaagctgtgggctgcctatgaaggctatttcaaatatcccgagattgaaaaatatgaggtggaaggccaggtaaatttcaatctcgtacctcagtgcgtcctcgaaaagtttagccagttgtataggataagaatcaattcagagcttgtcacactcatcctaaacagctgtgcctttatgagtaaatataacgattatattctcaaaaaagatccctacatactaaccataacccccggcctatgcttttcccccattcccaacttcgaggacctaaattttaaacatctttacaacagtgataaaaattctcagcatgacaaagagtttatcatgtttatattatataagctttatacggctgccctaggagtgtacaatgccatctcgattccagacatcgacgtagaagaccttgaaaatatcatcctatcctcggtgagccagattaaaaaacaaattccgcgctgcaaagacgccttcaacaaaattgaatcttcggtacacctgttgcgcaaaaattttaacacatattacagtgactatgtgggctcaggctacaacccaaccatcattatggaacagtacattaaagacatatcacaggattccaagaacatatcaccacgcatttcctaccagtttagaaccatcatcaagtattaccgcgacatgattgccaccaggcatcaaacgatggacccccaggtattaaacctcgtaaagcacgtcgaaaagaaattagatatgcttgatagagaaaaaaattagtatatatagttatggtgaatctttttcctgtttttaccttaattgtgattattacaattttaattacgactcgagaactatccaccacgatgcttattgtttctcttgtaacagattatattattattaatacacagtatacggaacagcagcatgaaaacaatacatttttcatgccgcaaaaaaattcttttaacgaatcttataataaagacaaaaaatctaatatacatattccctaccagtggctggcgcctgaactgaaggaagctgagagcaagtactggtggggcaattatgatcctcatagcgagcccgttctcgctggcgcatcttgaatatcttcatacgtggcacgtcaccatcaaaaacattgcccaacagcacgggcttgatataaaggtggccattgtggtctcaacatcgcatttaaataattttttgccaatttccggggcgcttaacatcgaatgtataaccttccccagttgcggcatcaaggagatagacctcctatgggcgcgcattaaactatttcaacattactgcgccatcggtgcccgtcttttatggctggtaagtgctgacatcaggccccctgtttcagcgtggccagccatcgccgacagtctaaaaaagggagcagatgcggtcgttattccctacccctcccgatggaacaatcttatacctaccgtcatcaaagaaatagttgtccaccaaaaaaaatgccttgtggcggtggatgcacgccaccttgatacagatacccagattgtaggggccgggatgggctgcatcgtcctaaccctaaaggcccttatggtgcgcctaagtattggcaaacagcccgttaagatactgtggcccgaccttcacggcactgccgagggcattcctctggagggggtggaggttggctggtttttaaacgcttatgcgcataaattaaatatacgctgcctaggggctgatcatattgcgcagcacttaacttaattctttatttaaaaagtccacgcatccagtggcggcctacattaagggcctacgcacataaatatacactggctagaagtacgccttcatttaaaccattgaattatttatataatggctgcaaacattattgcaacaagagccgtgccaaagatggccagcaaaaaagagcatcaatactgtctgctagactcccaggaaaagcgtcatgggcattatcccttttcatttgaattaaagccttatgggcaaacaggcgcaaatatcataggagtacagggctcacttacccatgttatcaaaatgacagtatttccatttatgattccttttcctttacaaaaaactcatatagatgattttattggtggacgcatttatttattttttaaggaactggacatgcaagcagtttctgatgtaaatggaatgcaataccacttcgagttcaaggttgttcctgtaagccccaaccaagtagagcttcttcctgtgaataataaatataaatttacatatgctataccggtagtgcaataccttaccccaatcttttatgatctttcgggaccgctagatttcccattagatactctttcggtccatgtggatatcctctccaatcatatacagcttcctatccaaaaccataacctaacaacgggtgatcgtgtttttatttctggatataaacacctgcaaacgattgaattatgtaaaaataacaagatttttatcaaaaatataccgccgctttcatccgaaaaaataaaactatatatactaaaaaatcgaatcagaattccgctatactttaaatctttaaaaacgtctaagtaataacatttttatagtctactcctagttccgaaataggctgaatttcttttttaagtcctttaaaccaaggatgtgatacaagactcttaaaggaaagccgcttattttcattaattgttaaacattccgtgataaactgttttcccgtctctgaaatgttctcgggaatataattttcccgtttcaggatatcatttaaataaaaattttctgcacgaaatctaaaaagattaaccgcgaccatacctatcgtccacacggttaaaggaagctggtagtaataaccataataataaaattctggacacacgtattcccatgttccaaacatattatattggggacgggtttcgtctaatctaacagcgcttccaaagtcaatgaccttaatgatcttttgatttatgtctataataaggttctcatccttaatatccccatggataaagcccttctcataaatgttttgtataataagaataagctggaatattatttttttggcttcggtttcctcaagttttttaaagtaatgataatgaagtagatcaacactatttggaatatattctatgattagtatatgatacatagcattttcggtatattcgataagcttaataacaccgggagtatcttgcagggctttcaacacgatgacttcatttcctggaatttcttttttagaaacgtacttaaatataatgggttgccctacttgatgacccaaaaagacgttatttctgccaccctcaaacatgggtctcgtcgcaatgaaatacatgtgctgcgttgtggagatcctttccacctttgctgtaggataaaacgcatattgtgcctggggattttttaacatttttttaagctgttgttccggcctggacatgttttattagctttatatataaagggttagaaggtttaatttcaatatatgccttaatgatgggattatattcgtaaaaggtatagcctaatcctacgtctttgtttttttggtaaaaaaactgtttgccctcgtaggatatgctataggcttttacttcggcttttacaagcggttggcagggattgggcaaacgtaaatcgcgttcaaagttttcatgaaaaagcaaagcatttgtgggctgacacatcagacagccgctttcgccattgaaggcacattcaatggccgccctttttagtaaatcgcggaaagcagaattaagatggctcttttcaagccccctttcgtgaaaacgctcatcaatcgttttttgttcctgactgccttcgggaatactataaaacattttttgattagccaccgcgatgtacaaaaaaggctgtacggttttctcctcgggcggtagcgcatcgtggctaccaatgcgtataatgcgcgccttcacttgatcctctcgggccttatcccagtacggctctaggatatgaacctgccgcccgtatttgagatccaatccctcagctcctgttttagagacgagtaaaattttaataacctctccgtgtatattcagcggcgaattccaaagctgctggatcatgtcgcgctctttagataaaattttccctgtaataagcgtaaatcgtgttattttggaggacaggactaacgtatgggtcggcccatcttccgcaaagtttttcaccataagatctttcccatccttatgaaggaggatggtgttgtgcccttcttccaatacttttaggggctgaaggcactggtagccctctatttctaaaaagcgggccacgacgtgaaggcccaattccacaaactgtgagtaaatgagcacagggcccggagacgttttaatattttttagcatgcgtactattttgggactagaattttctgtgaaggcctctttgggcagctgctgaacagcctctgataatttttcatcctcctttactgttagcatttcggacgcgaagatgctgatcatacgggaacgcacatagtaggaggagcctgactcttgctccgatcctggcaggcagagggcggcggcatttattttttcatacattcctgagctggcgtgcttttccgcgttttcaacgtctcgggccagcagatattgcctatactgctcgggtgacatttcaaccttttctataataagaggaagctctgtggggaatagcttgttgagctcattctggtttccagcgtagcttatcatacccactaggcggtttagtagtttgtccgcgtttaaagggctattcgttgttttattgacataagcggtgtagaatctttcatagtgaagaggtaataagattcgcccgcttagcatattaaaacagggcaccatttcaaaggggtccttcgaacacggggtgcctgttaaaaacagaatacgaatatttttagcttgcataatattattgtacagctggcgggcatttgttttatcattggcgctattgataattcctctaaagaggttgtgtgcctcgtcaacgatgagcaggcatccatttagggaccctcccgcctttatgatctgctgccccatgttgtaagcgtctagggacacaaacctgaagcgccgcgagattttttgtagctctttggagtgatccgtcgtttccggatataaaagtttaataagctttaacaaagactgttggaagtttgagtgcaacgacttgggtgcgatcagaatcgggttgtaaatatgtgaaagtgagatggcaagcgacaggctcaaaatggttttccccatgcccatctggtgatagatgaggaggccccgtgtgttttccccctggcctatcccaaatttaggatccgaaaaggcggtgtaaattaaaaactggtagtatttcagggctcgtgcaaagcgggcagtgagtgaggtgtctttgctttcctgaagctctttatatttttcatatacctcttttaggtatgcttctatttggacggggaaggaggtgttgttgtgcacgcaagacatgactcgttataaggatcccatattaaaacttcattagaagaatagggctgctgatagctagcgctgcacttaaaaatggggtagccctttttcttgtaaatccggtgcctgtcgtagacctggctagaaagcgggcttagtgtatctttaatgtccacaacgatgcgtacctttttttcatccgatccctgccgggtaatacgtcccaagatttgctccatgttgtttctgcggggcgttgccatgatgatcgatgtcatatgcttgaaggaaatgcctctacgcccgtagccataggtcagcaagataatggaagcgctgtgtgcctgagaaagagcggtatttgaaaccccgccgcataggagcgccacctccggaacgataatttgaacatctttgaattctttggaaagcgcctgataaaaaatttctaaaagtttgcgaaattccacgaaaatgatgatgccatacggctcatcggtcccccatttgtgaggctcagcggtatgcagggagtaaagccgctttgcctcatttacgacaagttgtatacgcgaaggatcttgaagtagtttatcaatggtggcaatggccgataccttttcattaatatacacagggctaacgaagtcaggatgtccctgatattcgatttccctcacgtacccggaaaaggttgtggtgggacttacagtcctctggggctgtcctagatggtgaataataatcttgtccataccatcgggccggtccaggggtgtagcggacagtcctaatatccgactaagttgtattttccaaaaaattttgtaattctccggcgagtgtaattcatgtgcctcatctaacacgactagaccaaagggctcaaagaactgctcaggcttcttgcgcagggtattaatgattcccacgatgacgtcgtactctttgctcgtcatgtcctttttcttgcacgctgcattattgtaagcagctacacgtaggtggggcaggagcaatgttagctcgtcgatccactgtatttgaatcgccttggtgggcacgatgaccagggtagggtacaaaagtttttgaataatgctgatcgcaatacgcgttttccccaaaccggtatttagatgtaggtaaaagcgcccatagggggacaggagctttttatgaatcttatcgaccatttcttgctggtagttaaatagtggaaattctgtttcaacgcatgggagggcccgcagcgacacggggcgcgtcgtgtaaaccatgttaaacatttcaaactgcttttgcagcaatatgggaaaataaatgtattccccctgcagcgtgaaggcagtttcctgtcttatggctatgtgctttggctgcccgggtaatgcccgcgccgtaacggtgagcgccttaagaacgcgcccgaaatcatgttgtaatttactttgtagcttcttataatttattcctattccagcaaaggatataatggcctccattctcacgctggacgggttatatgcagaggttccaaaattcttaccagaggcgttacgagagggctgtgctggcaagaatcctctaagcttttatattcaacaaattttaaatttaatgggatgtgacggtaacgagtaccatgttctttttaccagcagctccgaggaagcaaatactcatatgatcatggccgccgtgcgtcgccatttgctgcggacgcagcaaaggcctcatgtcattatcggagcagccgagccccctagcgtcaccgaatgtgtgaaggcattggcgcaggaaaaacgctgcgtatacaccatcatccccctaaaaaattttgaaatagatcctgttgcggtatacgatgccatacaaagcaatacctgcttagcgtgcatttcaggcactaatgctgttgtcaaaacgttcaacaaactccaggacatcagcaacgtgttaaaaggtattcccctgcactcagaagtgagtgatcttgtttatcaaggatgtattcaacaaaatccgcccgctgatagtttttcaataaatagtctctacggcttcctgggagtcggtgttttgggaatgaagaaaaaggtcatgcaaggattggggccgctcatttttggaggagggctgagaggcggaagccctaatatacccggaattcatgccatgtataaaacgctaacccagcaaaggccttctatgaaaaaaataaatacaatacatacgctgttcatgaaaactttaaaaaaacatcagcatgtatatctacccatagggggcgtgtctgcagaggacacgtctgcagaaaacatatctacaaaagacatgcctgttgaaggcccgaagggactcccgggctatattttatttagcgttggccgtcgcgccgaggagctacaaaaaaaaattttcactaaatttaatataaaggttggccgtgttgttgacttacaagagatactgtttcgtatcaaaataccccaaaaatactgggagacattattgttcatccaattaagagataatttgaccaaagaggacataaaaagagttatggttgttttgatgcatttagataccatcactcctcgtggctctcttcctcctccgagccactcttcttctttttcttaatcgtttttgtttgttctataataagggaaaagaactccgtgggatcttgttccccgtacaggttatctgcgaccataaggatgcttagaatggtaaacaggtgagaatacataagggtttgcgttttaagaaaaccctgacgttgaatcataattgaaaacaccttgcaaagccgactcatcagttgttctgtaatggcgttaagcattttctggaatttttcttggttttcgggtgtgattttatattcatgtagaaagtgtttcacacctgaggagaagaatctttcctccttcgagagcccatctttgatgatgggaagttccttgatcagggcaaaccattcctcctcttgggcttgcggattctgaagatactgatggcagatatggtttagaatggtgcacacgtagctaataagctctgagctgattctttggttggttttcaaatgttggcgaaagtagtttttcaccgaagtgcatgtaataaacgtcttcattttcttataatatacaacagtatgttgagtctttaatttaaaattacaaggagttttctaggtctttatgcgtataggtgtttctttgtcgtaaattttcaatagccgacattgtttgtgaagcagtgttctgagtagtgactgtcgtgtaaggctcagccggatgagcaggagcactcgcggccgcaggtgcggccgccggcccgccagttgccatgactagtctgtccgtaactgggttgtccgtaactggtttgtttgttgctggtctgtttgttgccggtctgcccgtgactggcttgcctacacttgctgtagtcgctccagctggtttagaggtacctggttgtggagtgacttctacccactgctgatcttgataaggatttataaactgtatatcttcctcctcaatagcagcagcttttttctttcttgaagagaatagatagattagaacgatgataatgatgactaagaccacgatagcaatgagaatagtatacatatgtgtggagaagaagcttggtgtagtgactggtgacaaacactcaccataatgccgcggataaaccggttgaaaaaattcagaatccatttaagatactattataaataatatataaaaatgttgtggcgcaatgaaattacagaatttatggaccaactttccaagtattctcaagaaatcttaaaaacgtttaagcaattgcgtcctagtgaatataaacaatacaatgaatttttaacacaagttacaccgttgctgcaaaaaacccctgaaaaaattccagagttggttgaccatatattcaattacctagacaacgttgaaaaaatttgtgagctcctcgtgaatgctagctcaattattattagttcaaaaatacgagaacaagtaaaacacggaatgagcttcagctataaagccgacctcgactccttggcggacattctctctcaaaaacagtacgtgcttatgcatctttcaaaaaatattgcggccgagtattttaatacgtgtttaaaccaagggaaatccaagttagatctcaaagctgcctctgtattttatagtagtcgttcccgaacggcaagctcagcagaactctatagaaaaatgctatacgcctatggttcaccgcaggaaattaattattatactgaaaaagcccgaaataagacgttggatgtggaggagagcgacagcatggccatcatcgaacgaacggcccgacacaacctttcccttatgcacccgctagaagccatggggcttacctttggggcaaccaacacggacgccgacccggaggatctgaaggacaaaacggtgataaatttaacgctcccgcaggcaacagaaagcatcacctaccatcttaaatccctaatgcagctaaaaaaagtaagtacggcttcaggactaaatacaaacattttgaaagcatttgataatattatttccacccctgtgaaaaaaaataaaatggcctccaagttggcgcccgggatggatgtcgtgttcactagcgataacggaaaaacattttttactaaaaacattttaagcaaaaacatgctagcggggcccaaagagcgggtgtttgcatataataatctcattagtaatttaaataactcctgtttcatacaaaatcacaacgattttttaagacagcaggactcttggcccttctatgacgcgcacaattttaccaacaagtttttaatgcagcctattttttcggggcagacccgtcctcggcttcagggagccatggaggcggcgcatgtggaaacgcatctcacggcatttttacaaagtattcagccctctaggccacaagatccctctgttttggcttcccccaagttatctgctctaatcttgaactaaaaacagcctttcttggacttaaatgatggtctaccagtttttgaaataacttagagaactatgaagattttcatgaaatttaaattagagatttgcaaaggttacttgcggtcattttctgttgaattaaataattattcgaatagtataatgtctgaagatattcgtcgtggtcctggcagaccgccaaagaaaagggttgttcccaactttgagcgcaagggcattctggaaaaaccagttcggccacaaagccgtctcgagttttcctatgataacccgctgatatttaaaaatctttttatttactttaaaaaccttaaaagtaaaaatattttggtgcgatgtacccccaccgagattacctttttttcacgtgaccagtcgcaggcaagctttgttattgccaccatcgacggaaaaaacgtgaaccattattacgccagtgatgtcttttggctaggcatcaacagagagctcgttgaaaaaatgtttaacagcattgatcgctcttttttaaaaattaccatcgttcaccgctatgacaagcctgaaaccctgttttttatctttacggattttgacattgacaaggagtgcacgtatcagattacggtctcggagcccgagctcgatatggaccttatcgaaatggaaaaaagcatcagtgaagaaagactcaagaactatcctctgcgctgggagtttacctccaagcagctcaagaaaacatttagcgacttatcaaactacaccgagctcgtgaccattgaaaaactcggcggcgatacgccgctgcacctgtatttccaaaagtttaactccatctcataccacgagatgtataaatcttccaacaagatcaacctgacctcgaccattcctaagtcgcaggtgttccagataaatgttaaaattgctcacatcaagtcgctggcctcggctatggtcaccgacaagatccgcattctgtgcgaagaaaatgggaacctaatctttcaatcggaaatggatgcccttatgttaaatacgattaccttgaacaccacgatatagttcggtaacattagatgttctaatatttagcatctaaataatacgctgtagtccggtcagggttgcgtcacagttttcccatttttttgcctcgtcggcggtggccaccgttgccctatcatttacgcccggtaagacaaagctaaaggcgttcagcggggcttggcaatgcccgcccagcgtgaaggagctcggaggattttgcgcatcccgaaatcccttagccatgttgtttaacacttcggttacgtcaatcgagtgaagggatcccttgggatccgtgaatgtaaagacgcagtttctaaagcgcatgtatgcgatggacgattcatcgggggttttgaaggtaacagtgttccccttgctgtacttaaagggggaccatccggtaaaattataccaaatgaaagcaataataattaaaataaccaacacaatagttatagacaacacaaagtctgtagtgccgcccattattaaataaaaatattttagaccgccggcttaaaatttacttattgctcatagcttaagtctattttattcatagcttaagtttattgctcatggcttaagtctattgcttatagcttaagtctattttattcatagcttaagtctattgttcatggcttaagtttgttgctcatagcttaactccattactgatagcttactgatcatgacttaaataaaaatattttgcccgcttaaaaattgtttaggtttgaaaaaataagagatggagggggcaacttatcgtcattgtgtttacccccactggaagacatcaaacggtaaataattataagaatcaaaatgattaatataagggttaaaaaaggatgattcatcacattaattaaaaacgtatttataacgctgttgcagttgaaattttggtataggtcggaaatattgcccgagcctccgtattctgcaatgttctgacatatggtgagtccggaggggcactgcttgttggtcaaaatatttctttgctccgttgttttataggcatttttatttccattacacggagcaaacgcacattcagcccatagggtgccggagttcacacaggcacaatactggctatacgcatactcatcctttgagcacaatccctgtttatcgcatatgctcccaataatattgtcatcctccgccgtttgttgatttgtatgcgagcgtaaaatagcggcccaggccttgggctcctttttttgcagctcggaaatcgaagggcctgtacagctaaagtcgacccaaatatcattgcatttcgtggaaactggcatgcaagacataattgaaataattaataagtatatatcatggcaacaaatttttttattcaacctatcaccgaagaagctgaagcatactacccaccttccgtgataacgaataaacggaaggacctgggggtagacgtatactgttgctccgacctagtgcttcaacctggactaaatattgttcgcctgcatattaaagtagcatgcgaacacatgggcaaaaaatgcggttttaaaatcatggcgagaagcagtatgtgcacccatgaacggctgctcatccttgcaaacggaattggtttaatagacccgggttatgtgggcgagctcatgctcaagatcattaatcttggcgacaccccggtccaaatatgggccaaagaatgtttggtgcagttggtggcccaaggtgaccatgtgcctgaccatatcaacatcctaaaaagaaaccaaatatttccgctgtttgcgcctaccccaagaggcgagggtagatttgggagcacgggcgaggccgggattatgagaacttaattttattttttttcttaacataatgggaggctctacaagcaaaaattcctttaaaaatacgaccaacattatcagcaattccattttcaatcagatgcaaagttgtatttccatgttggatggcaaaaattacataggcgtattcggtgatggaaatattttaaaccacgttttccaggatttaaacttatcattaaacacaagttgcgtgcaaaagcacgtaaacgaggaaaatttcattacaaatctttcgaaccaaattactcaaaatttaaaagaccaagaagttgcgttaacccaatggatggacgcaggaactcacgatcagaaaacggatatagaagaaaatataaaggtaaacttaacaaccacacttattcaaaactgcgtttcatccctgtcgggtatgaacgtgctggtggtgaaggggaatggcaacattgttgaaaacgcaactcagaagcagtcgcagcaaatcatctctaactgcttgcaggggagcaagcaggccatagacaccacaaccggcatcactaacacggtaaatcagtactcacactacacctcaaaaaacttttttgacttcattgcagacgcaatttcggctgtttttaaaaacatcatggtcgcggctgtagttatcgttctaatcatcgtagggtttatagccgtcttttactttttgcattcacggcaccgccatgaggaggaagaagaagctgaaccactcataagcaacaaggtattaaaaaatgctgccgtttcgtaataatttaattaaaagtaaaaaaaaaaggtattgttatagtgatggcagattttaattctccaatccagtatttgaaagaagattcgagggaccggacctctataggttctctagaatacgatgaaaatgccgacacgatgataccgagcttcgcagcaggcttggaagagtttgaacccattcccgactatgaccctaccacatcaacttccctgtattcacaattgacccacaacatggaaaaaatcgcagaggaagaggatagtaattttctacacgatactagggagtttacttcactggtccccgatgaggcagacaataaaccggaagatgacgaagaaagcggtgcaaaacctaaaaagaaaaaacatttgtttccaaaattaagctcgcataaatcgaagtaaaaattgaagcgaaaaaaagtagaaaaaaaatgtttggagcttttgtaagccaccgtttgtggtcagatagtggttgtacgaccacctgcatcacaaacagcattgctaattatgtagccttcggcgaacaaattggatttccctttaaatcagctcaggtatttattgccggccctagaaaggctgtgataaatattcaggaagatgataaagttgagcttttaaagatgattgttaagcacaatctttgggttgttgctcatggaacctacttagatgtgccctggtcccgtaagagtgcgtttgttacacattttatacaacaagaactacttatatgcaaggaagtcggtattaaagggttagttttacacctaggcgctgtggagcctgaacttattatggaaggactaaaaaaaattaagccggttgagggggttgtcatttacctggaaaccccgcataacaaacatcatacatataaatacagtacaattgagcagatcaaagaattgtttttacggatacgaaataccaggttgaaacagattggtttatgcattgatacggctcacatctggtcttccggtgtcaacatctccagctataatgacgcggggcaatggctgcgctcgctggaaaacattcattccgtgatcccaccaagccacattatgttccacctaaatgatgccgccacagaatgcggaagcggtatagaccgacatgcaagtctttttgaaggaatgatttggaaatcatatagccataaaataaagcaaagcggtttatattgttttgttgaatacgttacgcgacaccagtgtccggctatattggagagaaacctcgggtcttccatgcaattacaaaccgctttaaccgcagaatttactacattaaaatcgttattaaaataaggatgagttttagcgaatgtcccttagttattagtgcatgcaaaaaatttctacaaaagcgtattacaatagagaatgaagcacttataaatgccttaataaccgctttagcgcagaccagcacgttgaatgatctttgtttattacctattcaaacctatttgcttagttataaaaatgcttttgagtggatacacttcgtatgtattgcaatcaccactattttggataataagtataactggaaggactgtacggtagatattaattatatttttctccatgtaacctatatttacaatattaaaaccaaggaatacctagactactgttcttaaactttattttttctatatttacgccaaagagaatatttaaagttttttttgaaaaaaaataatatatgtagataaaattcagttacatgatatatgtgtaaacatgtgtggtaaacaacatatggttatgctttataagataaatgcgcataatatatgtaaacaaaatatggttatgtgttaaatgcatataaatgtattttaacgtatatcttgtgataatggatatatgcatttattaaaagaggctgtatttattataaatcttgctaaggatgccattgtcaacatatatcccatgttggacaaattgcgttgcgatccagttcttttttttttgattttgtttaatgctatcctttttgaagggatggttgtccaccatatttattcgatgttcaatgaataggtctgctttttcgtaaggcagtgaaggtcgttccaagactccttgaacgaaggacgtgttttcttggatccacttaaaaagcacgtggcattcaaaaacaggacagtgattggatccttggatatgctttggacagccaatgcttgaagagatgtagtcccttttctttaggacaagcttctccacgctggggcaacagagatcgttcaagttctggacggtcgcatttggaatgttgaaacttcgtatccattcaccctcgggtcctcccttatgaagaaggagtatttgctcatggtccttagtaatcttaaccaaatgttggaagatcatttttttacctgctttaaaggcctgaagggtgtcagttggcaaagctattgaattcgggagtgggctttcatcaagcgtgaaatggtgaatgtgacgcgactggaaagaaaacgaccgttgatttattttttcaaagattgggtcgattccgccatgaaagaacagctgcaagattttagaaggcgtatttttttcccaataaaaaatgaccacttctcgtgggattaaaatcgtctgtgtcccattttcattatataattggcccataaagccatcaacgtcaatcaacaccaaaagcatggtatagagagcttttagaaccggagttcgttaaaaaaatacaaagttcgtttaaaacgtgtaatgttactaaaaaaatgtaatgtttaaatgataatgataccacatgcattaatgaaaaaaacttttaaatttttgttttaatatttgcatgaaaatggaaacatttttagtctgtttatttcacaatgcagatggtttacatcaacagattcaggaaattttgtatttattgcggatgcatatttacgaaacaaatctttacttaaagcaggaactatcacggcttatatatccaaataggcaactttcttttgtgttacttatgcccctttcccttctaagaaactgggatgacattgaatatttaacggacgttgtagatgataagcagactctacattacgcggcaaatttgctgacaaactacgttctacatctatccatgtttcaaaagctgacaaaaccatacttccttttagcggtcaagcgggtcagcgaaaaactcaacaaaaagcagcgacattcattttacgaggtattggtaacctccgaaaccttgaataattatgaaaacctatctaaaaacattttaaatacgttgatgtttgccgtgcgctacgtatttaaacctacgccgaactattcagaaattctcgcagagttggaaaaaaaaaataaaattcaccatattatttttaatatggtaattacggattttgcgcaaatccgtgaacaacaaatggataaacatctgtgtgaaacaaataatgagcttcgtcaggaatgtaaagaaactatttttgatttaaaggtggtaggaaatgtttagccaataaactcatgcccgcattttttacaggtacaaaatatcgtggatggctcatcgagggcgcgtgtttgtacttctctgtaggtacacatacgctgcttgcagttgggacacttataaagttgtgacgtcttttcggcgaccttttgctgcgaacgtagagtaatttctgtcttctcctttaaggcggcagaggggcaaagctcggcgaacgtcatgctaccaattgcctccggttttagctcgccagaaattagcttattaagggcatcgttatcctgttgttggtgactttttttttcgcagttaataatatgattgatcgtcccacaacgggttgaatattcttctaaaaaggttttttcttgttgctggtacgtataatgataacacgaggcctcgattttttgcgcgtattcggtgcataaatcagtatgttccttaaaaaacatatgtttttgaagcgttctaaaaaacatcatttggatgatatcacgcatttccaaaataatatagggttctagtcttttggaatctttcataactagatcggtggtaatattcttagtcatacaatttattaaaaatggtttaatatattgtaaatattttttaggcgtgtcagcctgtaaaaaacattcttgttcaatcttatttgtaaggatagtattttgcaaatacttatttagcaaaaatacgatagaatcgcgggctatatgcattttcatataattttttttttaaaatttaatacaaaaaaaagaagtatagactcttcttctagtccggttagttcgttggttgcctcaacatggagactcagaagttgatttccatggttaaggaagccttagaaaaatatcaataccctcttactgctaaaaatattaaagtagtgatacaaaaagagcacaatgtcgtcttacctacaggatctataaatagcatactgtacagtaactcagaactttttgagaagattgataagacaaataccatttatcccccgctttggatacggaaaaactaattgtaaccagtagtacatttaaggatagtttaagcagtaaatgtagaataacacagttaagcaataaataacaagtatataggaatatataggaatatatagaaatatatagaaatagctaagcttaatactaattcagctttttttttaactaaaacctgaatagatgcgaagtagcggacatatacatactaaaataagccatacatttactttcttcttgaacatgaaacctttttttcttctgttgttggtatataaacaataggactgtttgctgaggttgtatgatcttctacaactgctgtctcaggatgacgatgtttttttaaactaaaagtgtaggatggaatgagtggaatatagttatggctcgacttatcctgtttcgtacaggaatattttttacaaatagaacgcaacaagcatatgaataaaaacagaaatgatatacaggagcataaaatagatatgaacactaaggggtagcagcttttataacgttccgtatttttcttagctatcaattgatttaccgtaatatttatctcgggaaactttgttctacaatattttgtttggtattccagaaactcatgtcctggcttattcccgcagcttaaaaaatgatacaaaaatgtgttattgttactaaaattaattcttcttaagaaaaactgcggaagacgctttaggtacgtctgttcctgttttagtaggaagtagtataagggacaatttctttttccacacattagattattgtaatataggtaggttggggtgttggagcgaataagttttctgagtatgttataatctatgacttgtaaatcgttataccttaggtccaaaaacttgagttctttaccaaagccacctgcaatttcagaaatatttttcatcccgcagcggataatacggatgtcctgaaacgtctttaaaatacttgtattgtagtgaatacttatgttatttttttgtaaataatctatgtcatgacaagtgcatgaaatgccagcagcattgcttggtatagtattatatgcaggaagaactatactactattgagaatagtcacattgtacttataccatgtattattttctgatataaagtatttgcaggtgacctgtggtttaatcctacctgttaagccacttcctaaaaaaacaaaaaatatgaaaacccttagcatcctgtatatactattaaaaatttataaaattttctgtttaaatttcatttagacaaaaaaaataatatatatacatcagcaagaaattatatacagattatataattttctgatttttttttgccacaataagcatcattatatgcattaaaatctcaatactaaacactaaaatctaaattctaagcattaaattctaagcattaaattctatgcactaaactgtaagcactaaaatctaagtaactaaaatcaacactaaatgtatgcaacctaaaatgtaaagcattactcatcatcctcctcttcttcatcctcatcatcataggttaagatatatgtgtcatcctccatttcttcacattcatcttcataagcatcactgggtattggtggaacattggatgcagcatttttaaaatattctatgtcttctggtgaacactcatctaatgattttttgacagtccttttaacttccatgggatatgattccaaatcctctttatataagagtttacggtagcttttagctgcatccacatttgctggagaatctggatttggctcattgagcagtgaaattacactaagaagaatggtatcaatcttttgagccggagaccaagtcattccctgttcttcagcattgtctccgtgtaagatagagatacatagttttccatcagagtaaatattaggatgccacatttcagaggtgaatgttaatctgggtggtgcatatgggtattctggaggaaaggcgatttttgccttgaataagcctccctcataaaaagtgtcaggtgggccccttaagatcacatcccattcagtcatatccttctcattcaccgaaattttgaaattctcagagggattctctatcaggtgtctgtactctgctattaaaaacctggaaaccatggttatttaatattaattaaattccctggtttattcctccttaaaagtagatgaacctcttttgttttttattgggttcatttttactaaatttatgaactggaaaaaactttaacggcataattatcaaatgcgaagggggatccgtataaaatcctagcttgccggtaatggctattaagttaaatttggtaccagtaacactaatatttaaaaagccctgatcattaactttccacattaaaagattattatattcgaatgtttgtccaatatggacaactttgtcaccagatgttacatttgatttggttgttagtggctgaagcttggcacaatcaaaaataagcccattaacactaagatatagaggagtgggttgatctattttctcatagtttaatattccatctttccacgtaatagcttgataattatccgcagcaatgagttgaaattttataaatagtacaggggttttagttgtcgttatacatttaaagggtgttttataaaaataaaaaataataattgttaaaagtatgataataatcgccaaaataatttcatacattttttataagaattatacatagtatggtatttaaaatattagctaaatttaaaaaaacttcatgatttttaaaacagggaaaaaggggattaggttgaataaaaaaggtaagcacttgtctatatattttttttacaatgttgccttgagtcgcatttttaactggctggggagtatcagagtggaatatcactgtagtaggtctataaggtcttgttaaaatatgatcggtcattgttttcgtactagtgtcatttagggtcgacctgatagctcgatataaagttataggggataacctatcaaatacagtcttatctgtgctgaaatgtatatcgtcttctttatcactaataatattaggaatggctgtcattaaataattactacttgttgttgtgggtgaaatagttgtactggtattattggaaatggctgtcattaaataattactacttgttgttgtgggtgaaatagttgtactagtattattagaaatggctgtcgttaaataattactacctattacaagtaaactaatgctaactacatttttaacctcaataaacctaaaaagccatactaaatacctaaacaacatcctgttataatatgagcagaaaaaaaaaataagtataattagggaattattcttattcgcttactattaagaataattcagaatcttatttagttagaaactatcataaagtgaataggactcatcgtcggatgaagattccgtttcagagatagtttctttttcttcctcagaataatctgttcctacaatagaatcggtgtcatcctcagaaagagaagtatttaaatatggactatctatagcaatatcctcttctatctcgcaatcctcctcctccatttccatagtgtgtaggagaatatttttatcatcatgctcacttctttttttgttgaaagatgaaccgtcctcaatacggttcatgttaagttccttcatcttatgtataatttccgtaatccgtgatgtttttgacatgtaagatggttttaaggttatatccacaataacaggagaatctctatcattttcatttgataaactttgatctttgatttcttcgtctaaaattcttgtctttttttgggtactagatgaaatagaggaattcatattctgaaacgatatatcaaggggagctggacgcttttttccaattaaaccgtttttcgagatactatgattagatgaatgatctttagccaagctgtccttggatatactatagttagatattttacctttaaataatattcttctatacaagttattcttaggtaaagaattagtatggattcctatatttttatctgaaggagtgtccatatcggagaacgtcctcttacgaatattttgaccacgagccatttcatccactataggcagtattttggctggctatggttctttgttgtgacaattctatgagatttgattgcaaatcaatttttagttttaaatatattggtacctaggacaaagaaagtatatatagccaataattattccactaaattgatttccagactgatgggtatggagccatgttgtctctgcagacgatcgcaaaaatggccgtagcaacaaacacctactccaagtatcactatccaatactgaaggtctttgggctgtggtggaaaaacaatacgctaaatggccctattaaaatatgtaaccattgcaacaacataatggtaggagaatatcctatgtgttacaatcatggaatgagtctggatatagctttgattcgggcagtaaaggagcgtaatatatccttagtccagcttttcaccgaatgggggggaaatattgactatggggcactttgtgctaacactccatctatgcaaagattatgtaaaagtttgggagccaaaccaccaaagggccgaatgtatatggatgctcttatacatctttcagataccttgaatgataatgatctgattagggggtatgagatttttgatgataatagcgtgttggattgtgtcaatctcatacgactcaaaataatgcttaccttgaaggcccgtatacctctcatggaacaactagaccaaattgccttaaaacaacttctgcagcgatactggtatgccatggctgtacaacacaacttaacaatcgctatccactattttgataatcatattcctaatataaagccatttagtctgcgctgtgctttgtattttaatgatccctttaaaatccatgatgcttgcagaactgtaaatatggatcctaatgagatgatgaacattgcttgtcaacaggatttaaactttcaaagcatttactattgttatcttttaggggctgatattaatcaggctatgctaatgtctttaaagtatggtcatctttctaatatgtggttttgcatagatttgggggcggatgcctttaaagaggcaggggcgcttgctgagaaaaaaaataaaagagtgttacaacacatattaggtcttaatatctttaagcgagagttgattcccccctgtaaagatcctgatccttatcaaatccaaattctgttaaaaaactacattctaaaaaatgtctcaactgtttttacatattattgccagtagccattgtttatatcagaaaataacccatttgtttatctttttttgtggggcaaccattaagacccgacgcaaaaaaagattaatcttttatcagatacctaaaacgttctataagggagtctatgagatggatcatattttgatggtcatagtaagaagcaagctttttggcgaaaacaacggagttaaagaatttaacccgctcatgtttggataggacttttaacagcgagccaaaacagtatttaaaaatttggcaatagtttttttgggatgcaataaacaaacacttgatcagtgcccgcttcactttctgatcagacatgtttgccgcataacaggcctttttaaacttagtaatataattatgttccgcaagcaccattaacaagggaacgatgggaagctgcttttcttggtgaaatttacgtaaatattcgatggtcaccgcttggacgactgtgtaatttactaagttagaaatgatagctttcatggttgtaaaaatatacataggattttctttttctgtatacagtttgaaaagcttatgattacgtgaaatgatggccatttttaatacaagatggtatagtgtatctttaggtaaaaatgccttgcaagccgcgatgatgtcgatgttgtctccatgaacagcgatagaaactaatgtttccaatctaaatgtttttatctgcattaatagaagaatgcagtcaatgttattatacttaataatactgtaatacaccgaatcaatgaccgtcatctgagaatcaagctgacttattagtaaatttaacgtttttttggaggcatgacctttgatcgcggcactaagtgcacacagtatagcaaaattgttaaatacattttgatttaggagaaggagtaatattttccttcggttatagtacgcagcatctgtgatgattattggccgataaatgttaaaatgtgttaacagctttttaaaaaaacggaagtaatttttttggatcgctgtttgcatcatcgaaataatgagataatcagggtatataatgggtaggtcacatgctacctctaacaaagaatagtcgcccaatctaaaggctgtgttgaaaagcgtactatcatcatacgtatcgagtacccctgctgttacaaaccaagcgataagatgaatgtgccgttccttgcaagctatcgcaaatagggagtttcctatggaatgtcgaataatgtactccctatttttttccaaaatgtttggaaaattgtatagcgttgcggcatacagtagacactccattctggcgttataatttttacttttacatatgaataggtggaagaactcgaataattcttgagaacttgttaaatgcataatatggtgatattttggtgtcgttaaatggtatgagaaaatgcattctaatacatcttttcggttatgctttagcgcctgagctaaggcatattcaggctcgacccataggactagtgtttctataattgagatattcgcctgctttgccagggcatactttaagacgctccggttagaaaaaatgttgttatgaagatggataaccgtatccatttttacgatgggaccattccagtatagtcctaaatgctgtagcagatcttttgttagttgtgaagcgttctcgggtgttatataaatatgttgcagggcttttttctgtaaggagaacatttcgtcgtaatcgtacaaaaaaaaattaaaatttgggcatggatgattcaaacataacaaaatcaagattttataacagtttgcattaacctatacatatatgcaagtaaatgagatattatctatcataacgaatcaagggatatttgtatatatcaggagtttctgaaataaagatatgaagattatcatagtagtatccatcaatcacaatgcaacttcctttaaggcataatttagtaaacttagcactcccattttctggatgctttacaactaacattaaaaactcctcagtcatattatctgtaataaaataagatcctcctggagccatttgtagcatgtctcttattcttacaaaatcttttttgggatggtaaaaactcagcagtttcaaactcttttttagttttttttcctggtatttaagccatttgttataaaacagttttcttatgaaaatgcatttgaaaatattgggaatgtttaaccatgcttcttccgagcacatctccagatacttactttctttgtttcccatgtctaatttattgctcactaagttagtaatgaatctattttaataatctactttactaatctatcttaataacctatcttataatctatcttaataacctaattataacctatttataattggctaatgttgccggcatttcatgcctatctaaacaactcctactaagcaatctactattacatatatagattcactttttatatttgtaaatcatgagaattataaaatcattactcatttttattgtaaattagtgggtatttgtaaaaatcttcaaacgttttaagatagttttctagagagaagtaatctttgccatcaatatataatgcttttcctttaaactccagttttgctatgtttagtgagccgtttctagatctttttgggcaataaatagattttcattggttgtatcgtccgtaagcagaaaggtaccactaggcacgttaaaaaacatacgttctatttcatggtcggatttttgagaatagaaaaaatctaattttttaatccgcgttaactcttttttatcaatctttccagactgttttatatatactttattgcaaatcttacaatcctctatggcttcattatacttattttgcttatcctctattgacatgtccgtatttgataggtaacttccgttaaggcggttccccatggttttagatagatttttaattcagttgtatacttttattatgaggctaaaatatagaagtttgatcctaaaaaaataaaaagattttgtacatttatttatggtttatagcggtatagaggccgataaaaggtatccgggtagtctcctatgatatcgtcaattttggtataataacagttgttatggtagtattgtccaaaccgagtatgtatgcgccggtgaagcgtctgcccgctaatggtacagttccaggttaagacaatcatatcacacccaaaaagagaggaaacagcataggtgcccaaaggtttattatataacatacgccgcatatattttagttttttttctccatggtaataatcacaggttttcatgtcctgcttaataggatgattccccatgtatgataatatataataaatttagtttttagctttttcaaaaaattgggcgctcgaaactaaatttttcttatcacagcgtttggagaaagcgtatttaaagatatatcttcttctaacaagactgcaaaaaaaatcttaccccttatttttataatgttcatcatagcgtttgaagatatcagaaggtgccaggttttataaaaatatcctttaggatttataacgatacaagggtctataaaatatatgcgggtataatcttataaaatcatcgattttttcataatattctccgtttatacaataaagatcataacagatattgatgcgtagatgcattattcgcgtgttcgttgggcagctaaaggatatcacaacgtagttttttttaagaaaagacgaaactacataagtccctaagggttcattgaatagtaaacgccatatttgttttaaattttgttgttcaccatagtagtattcgcactttttcaagtcttttttaataagcctattccccatgtatgcttataaataaaaatttagaaatgtgctatattatttgttgatgaatcatgaacacgtcttatatgttgatatgttactttaaaaacatttgtattttcaacagacgcgttctattcttattaagaatgatgccgtctttattttaaaccttggtttaaaatttaaagaagtatttataaactataatcatgggaactttttcagtaactgcctctgcaaaaagtgacgatgctgtttgtaagtatttagaagaaccaatagatgaaaattacagaaacatattaagaaatgagcatgttaaaaaaaatttaaatgaggctctgaatcgacatattactacctataatccagtagttgattggtgtaataactattcaacattttcatctcaggatttcgatgaatataaaatttatatacatagcgatcttatggatggacgacctcgtccaaaaaaaacatggtgtgtcatcatgtaatgtttgttagttttatataaacgcaaaaatattcttctaggagatgttgatatactacctattgaattcaatatattaaagtacatttctggctattcccattacggtattattattactatttttaagagctagatgtggatttaagtaataataacattctcccgttcctcctagagacacctcatcaaattcccatcctatgcaacctttatgttgtaaacataatgattgacagcattcatcttcttttgaccaagtcgtccaaatcctaccaagatctatacgtgtttttccaaatggagattgaagatcagcagtagtggcattaaacctataaaaaccaggtgcataatcacatgaacggatcgtaggatctaatttaatatcttttatatcttgttttactgcttctagacaacttttatcagtacatgttccacgtacacagtggtgtcctttatccttacaatccgtatctgtcttacatttttttttcggcggtttatgtttcagatggtaaaaacccagtattaaaataatcacaagaataattcctataagtacttgaacaacaggataaaacattttaatattaaatatattttttaattaaatgaatagatttaatccaagtagtattaaaattttttagaaatagtgttctacaaataatgaaatgaatggtccaaaaaaaataaggtgtacaataatgtaatatattgttaggctaagtaaatttaatattttaaagtatttggaaaaatattttttaacatatgatgtctaggaatattttttagacatttaaaaccatatagttactttatttattacactgaacttgaaaagacttattacctaaaatattaatagatgaagtaatattgtgtaattgagtccataacatgggtgggaaacaaaaatctcgtaatatgaaaaataaacatcctaaaaagagtgcaattgttataagtttatgtaactttattttaaagtaagaatataaaaatatgagtacaagaggaataggggccattactaacattggctccaacatcctgttgtctacaaaaaaaaatattttttttagcaaaaaaaaatccatggaaggatattaatacacataattatttgacatcacattagtgtacttaccaaatagtaatatacaaccatcctaatattcacctttatgaaatgatcccaacctatacggtaaaatagtataggttttaataaagaaaaaagatattctgtggtttttatttttgtatagtgtgtgaatacaaaataaaatcccaaattttaaccttttctttttttttctatacaggatgttagaaatagtattggcaacgctgctaggcgacctgcagcggctccgggttcttacccctcagcagcgggcagttgccttctttcgagccaatactaaggagctagaggacttcttatgctcagatgggcagtctgaggaggtactgtctggcccccttcttaaccgtctactagaaccctcaggccctcttgatattttaaccggatatcacctatttcgtcagaatcccaaggcaggtcagttgcgcggccttgaggtcaagatgcttgaacggttatacgatgctaatatttacaatatactgtctcggctgcggcctgaaaaagttcgcaacaaggctattgagctatactgggttttccgagctatccatatttgtcatgctcctttagttttagatattgtacgatatgaggaaccggactttgctgaactggcctttatttgtgctgcttactttggtgaacctcaggtaatgtatttgctctacaaatatatgcctctgacccgcgcagttcttacggatgccatccggataagtcttgagagcaacaaccaggtagggatttgctatgcttacttgatgggaggcagcctcaagggactagtctccgccccactgcgtaaacgtctgcgcgccaaactacgctcgcagcgcaaaaagaaggacgttctttcaccccacgacttcttactgctgctccagtagctttttttgccgcaggagcaccgcggataggagctcctccacgctcgcgatccggcgctggaagcggaaccgatcgaccgccacctgctcccagggacccttgcgctcgatgtcgtcggcttcccacacctcgacggctgtggcaaaatggacatgcttcgcgtcgttcgtccgttttttgcgccgcctccccattattcttcctgtaagattagtgtttaatacctataataacataattttaagatttaatataccaaaacttaaactatttttgtatagtaactattagcatgtctacacatgattgttctctaaaagagaaaccggttgatatgaacgatatatctgagaaatcagttgtcgtggataatgcacccgagaaaccagctggagcgaatcatatacctgagaagtcggcccgcgaaatgacatcatcagaatggattgctgaatattggaaaggtataaaacgtggaaatgacgtgccatgttgttgtccaagaaaaatgaccagtgcagacaaaaagttttcagtatttggtaagggatccctaatgcgctccatccagaagaataattaaaaaaaatattttttttagcaagtttttaaactatttaaataaatgtggtaaaaaaattcacataataattaaagtgaacgtgttagaattaatatttttttataatcggatataatatccattaaatcaataaatgatagtgttgctaccacactaaacaataacaaacagaaacgcacgatacctttcctcatgatttataatagcgtgttatctaaagatttttttgaaaaaaatattaaattttagttgattatttttttcagttacaacattgctttagaaaaaatacctaattactacatagcaaataaagcgagcgcattgttacaaacaacatttttttgcgcctggatactcctatatatgagaactataatacggtatattaatcctattaccaacattgtcaataatagtatgtaggcaatgacatactttaaataccaaatatccatggttatttctaaaaatcttgaaaaaacgttaaattttagatcggtcacctacgacagtaatactaattttaataattgatgactgaaatcataatataatgccgtgcgaaaaataattatttttcggttaaagataccattacataaaaaatatgccatctactctacaagtgcttgctaaaaaggtattggccttaggggagcataaagaaaatgaacatatatctagagaatattattatcatatattaaagtgttgcggtttatggtggcatgaagctccgattatactttgttatgatgggagtgagcaaatgatgataaagactccaatctttgaagaaggcatattacttaatactgcattaatgaaagctgtacaggagaataattatgaattaataaagttgtttactgaatggggagcaaacatcaattatggattaatttccattaataccgagcatgcccgggatctatgtcgaaaattaggagctaaagaaatgcttgaaggaaatgaatttatacaaattatattcaaaacattagatgataccaccagtagtaatataattttatgtcatgaattattcaccaacaatcctcttttagagaatgtaaatatgggggaaatgaggatgataatttattggaggatgaaaaatttaacgaacctattattaaataatgactctattagtgaaatattaactaaattctggtatggtatagcagtaaaatataatcttaaggatgcgatccaatatttttaccagagattcatggacttcaacgagtggcgagtaacatgtgctctttcttttaataatgtgaatgatcttcataagatgtatataacagagaaggttcatatgaataatgacgaaatgatgaatctagcctgcagcattcaagacagaaatttatcaaccatttactattgttttctattggggggctaacatcaatcaagcaatgttaacctcagtattaaattataatatttttaacttattcttttgtatagacttaggggctgatgcctttgaagagggtaagaccctggcgaaacaaaaggggtataatgaaatagtggaaatcttatcattagatatcatttatagtccaaatactgacttctcatcaaaaatagaacctgaacatattagttctttgttaaaaaacttttatccaaaaaatctgttcgcttttgatcgttgcaaccccggtttatattattcttagaggaccgctacaaaaattatttttttttcttgatcaaagctccaaaataattattagattaaagtcgcctatagcagcagcccactccaaaaaaagtattttatagtacaaaaaacacgaaaaatagtttgcggccggcggcaaactatttgttgttgtctaaaacttaatgtttttttaatatttttaaatgcaaccatggattgttggactatcagggagaagaactatagctacatcatattgtcaatactggtaatactattaatatggtatcttatacttaactattgtcgatcgaaaaaaaatgcagttacaaacaacatgccgccaccatacacggtgtcaagtagctgttctcaataatagggttgattgacgctcttcgtaataatatgttgattgacgcatcataaaatgctgtggttgattaatatgttgattgtcgcctactttattatataagtaatgatttttgtataaaatacgggtttgtgagggctttattttttcttattagaacaaagcatgcaatttaaggcctacagcaagagtaatttaacacctacaacagtaattttaaggtcagtaataatgtttaattaaggcctgaccactaaaacttaaacgattttgtaaaaaaaaatgtctactccactttctctacagactcttgttaaaaaagtgctggccacacagcacatatctaaagaacactactttattttgaaatattgtggtttatggtggcatgaagcgccgattacgatttgcattgatgaggatagccaaatattgataaaatcggcaagcttcaaagaaggcttatctttagatatcgcattaatgaaagtcgtgcaagaaaataaccatgatttaatagagttgtttaccaagtggggtgcagatatcaactctagcttagttactgttaatacggagtatacccggaacctttgtcagaaattaggcgcaaaggaagctttgaatgaaagggatattttacaaatattttataaaacacgtcatcttaaaactagcagtaatattattttatataatgaattgttttctaataatctccttttccaaaatatagagagattgagtttaatagtttataggggcttgaaaaacttatcaatcaactttatattggatgatatttcatttagcgaaatgttaactagatactggtatagtatggcgatattatataaccttactgaagccatccaatatttttatcaacgatataggcattttaaagattggcggcttatatgtgggctttcttttaacaatttgtctgaccttcatgaagtatataacttagagaagacggatatagacattgatgaaatgatgaagttgacctgtagtacgtatgatggtaattattcgactatttattattgttttatgttgggggctgacatcaatcgggcaatgttaacctcggtaataaactttcatattggtaacttgttcctttgtatagatttaggagctgatgctttcgaagacagcatggaactagcaaaacaaaagaataataatatattagtagaaatattatcatttaaaaattattatagttcaaatacctctcttttatcaataaaaacgacagatccggaaaaaattaatgccttattagatgaagaaaagtatgagtcaaaaaatatgttaatgtatgaagaattatctcattgatacaaaattattttttataacagaactctctgatggtgacaaatctccgataggaatatatgacgtaacataattatttttttcgcccagaaaaaaattataaatgttattattgccagcacttttatcaactatacgtacaaaaaggtgttgaccaaaaaaataattttttttcttgatcaaagtatgtaaacgcccgcttacagcaaggatcttaagtgagagccattaaattttattgatagctgcttgccaccagtagaatacggccaaaccacctaacaggaaatacaaggcggcccttcggccaataaggtggataaaaatcacgcataagacggttgtaacatagcactttagtgcgaatatcaggaatgccaatagcatgtagataaggcaccaaacatcgcagctatacatggctaaagatcaaccagaaaaggtttaaattttaacgccggcccaaaacttaaactttttttgatatttttaagtgcagccatggattggtccggccataggatgacctatgcctacgtggcattctcattgatggcaatagcaataatatggtatattctacttatctattgccgatcgaaaaaaaatgttgttacaagcggtaatacgctcgctttagcgccaatatcgcatatgtgaaaaatgttcgccgaaaaaaacattaaaatttagaaccgccgcggcatctcaggggcggcaacatttttttttatatggatattgtcacacaccacctcatctatgacgcaatatattactgctaatatcaggttccccaatagtatgtagagaaaccacacaagatagatattcatggcgatttttgacgaaaaaacattaagttttagcttctttgacgcctgtgtactaataatgtttaacgcctgtagtataataattgatacctacagcagtaattgatacctacggcgataatgtctctctggccgccccaaaaaaaagtatttacggtagggtttattaccggcggcgtaacaccagttatggtcaattttgtctggcccgccgcccagccgcaaaaaaaaatcaattacaaccgcaaaaaaaaatatttccggccgcggcgtttcaaaaaataatctttgcgaaataattccgcatcttgtgaaatgaacgcctacagtaataattttaatctttgacacctacagcagtagtaataattttaatctttaacgcctgcagcagtactaatatttttaatgtttaacgcctgcagcagtagtaataattttaatgtttaacgcctacagcagtagtaataattttaatctttgacgcctacagcagtagtaataattttaatgtttaacgcctacagcagtacaataattttaatgtttaacgcctgcagcagtactaatatttttaatctttaacgcctgcagcagtactaatatttttaatctttaacgcctacagcagtagtaataattttaatgtttaacgcctacagcagtagtaataattttaatctttgacgcctacagcagt